European Patent Application EP 4 400 593 A1, published July 17, 2024. Title: Method for RNA production. Applicant: SenseUp GmbH. The sequence listing filed with the application follows.

SEQUENCE LISTING (69 sequences)

SEQ ID NO: 1 - DNA, 719 bp, synthetic construct
  source 1..719: mol_type = other DNA
atggtgagcaagggcgaggagctgttcaccggggtggtgcccatcctggtcgagctggacggcgacgtaaacggccacaagttcagcgtgtccggcgagggcgagggcgatgccacctacggcaagctgaccctgaagttcatctgcaccaccggcaagctgcccgtgccctggcccaccctcgtgaccaccctgacctacggcgtgcagtgcttcagccgctaccccgaccacatgaagcagcacgacttcttcaagtccgccatgcccgaaggctacgtccaggagcgcaccatcttcttcaaggacgacggcaactacaagacccgcgccgaggtgaagttcgagggcgacaccctggtaaccgcatcgagctgaagggcatcgacttcaaggaggacggcaacatcctggggcacaagctggagtacaactacaacagccacaacgtctatatcatggccgacaagcagaagaacggcatcaaggtgaacttcaagatccgccacaacatcgaggacggcagcgtgcagctcgccgaccactaccagcagaacacccccatcggcgacggccccgtgctgctgcccgacaaccactacctgagcacccagtccgccctgagcaaagaccccaacgagaagcgcgatcacatggtcctgctggagttcgtgaccgccgccgggatcactctcggcatggacgagctgtacaagtaa

SEQ ID NO: 2 - DNA, 720 bp, synthetic construct
  source 1..720: mol_type = other DNA
atggtcagcaagggtgaggagctattcaccggagtagttcccatccttgttgagctggacggggacgtgaacgggcacaagttctccgtgagtggggagggcgagggtgacgccacgtacgggaagcttaccctgaagttcatctgtactacagggaagcttcccgtaccgtggcccaccctcgtcactaccctcacttacggagtgcagtgcttttcacgttaccccgaccacatgaagcagcatgacttcttcaagtcggccatgcctgaaggatacgtccaggagcggacgatattcttcaaagacgatgggaattataagacccgtgccgaggttaagttcgagggtgataccctcgtcaatagaatcgagctgaagggcatcgattttaaggaggacggtaacatcctcggacataagctcgagtacaattataattcccataacgtctacataatggccgacaagcagaagaatggtatcaaggtgaacttcaagatccggcacaacatcgaagatgggagtgttcagcttgctgatcactatcagcaaaacactcccatcggcgatgggccggtcttgttacctgataaccattacttgtccacccagagtgccctgtcgaaggatccgaacgaaaagcgggaccacatggtcctgcttgagttcgtgaccgcggcagggatcactctgggtatggacgagttatataagtaa

SEQ ID NO: 3 - DNA, 936 bp, synthetic construct
  source 1..936: mol_type = other DNA
atggcttccaaggtgtacgaccccgagcaacgcaaacgcatgatcactgggcctcagtggtgggctcgctgcaagcaaatgaacgtgctggactccttcatcaactactatgattccgagaagcacgccgagaacgccgtgatttttctgcatggtaacgctgcctccagctacctgtggaggcacgtcgtgcctcacatcgagcccgtggctagatgcatcatccctgatctgatcggaatgggtaagtccggcaagagcgggaatggctcatatcgcctcctggatcactacaagtacctcaccgcttggttcgagctgctgaaccttccaaagaaaatcatctttgtgggccacgactggggggcttgtctggcctttcactactcctacgagcaccaagacaagatcaaggccatcgtccatgctgagagtgtcgtggacgtgatcgagtcctgggacgagtggcctgacatcgaggaggatatcgccctgatcaagagcgaagagggcgagaaaatggtgcttgagaataacttcttcgtcgagaccatgctcccaagcaagatcatgcggaaactggagcctgaggagttcgctgcctacctggagccattcaaggagaagggcgaggttagacggcctaccctctcctggcctcgcgagatccctctcgttaagggaggcaagcccgacgtcgtccagattgtccgcaactacaacgcctaccttcgggccagcgacgatctgcctaagatgttcatcgagtccgaccctgggttcttttccaacgctattgtcgagggagctaagaagttccctaacaccgagttcgtgaaggtgaagggcctccacttcagccaggaggacgctccagatgaaatgggtaagtacatcaagagcttcgtggagcgcgtgctgaagaacgagcagtaa

SEQ ID NO: 4 - DNA, 936 bp, synthetic construct
  source 1..936: mol_type = other DNA
atggcgtccaaggtttacgaccctgagcagcggaagcgcatgatcacgggcccacagtggtgggcccgttgcaagcagatgaacgttctcgacagcttcatcaactattacgatagtgagaagcatgcagagaacgccgtcatcttcttgcacgggaatgcagcgagcagctatctatggcggcacgttgtgccgcacatagagcctgttgctcgctgcataatcccggaccttatagggatggggaagagcggtaagagcggcaacggctcttaccgccttctcgatcactataagtacttgacagcatggttcgagctcctcaatctgcccaagaagatcatcttcgttgggcacgattggggagcttgtctcgccttccattactcttacgagcaccaggacaagatcaaggccatcgtccacgcggagagcgtggtcgatgtgatcgagtcctgggatgagtggcccgatatcgaggaggatatcgcactcatcaagagtgaggaaggcgagaagatggtcctggagaataatttcttcgtggagaccatgctgccaagtaagatcatgcgcaagctcgagccggaggagtttgcggcgtacctcgagcccttcaaggagaagggcgaggtacgccgcccgactctctcctggcctcgagagatcccgctggtcaagggtggtaagccggacgtcgtgcagatagtgcgtaactacaacgcctatctgcgggcaagtgacgacttgcccaagatgttcattgagagcgaccccggcttcttctcgaacgccattgttgagggagctaagaagttccccaacacggagttcgtgaaggtgaaggggttgcatttcagtcaggaggacgcgcccgacgaaatgggcaagtacatcaagtccttcgtcgagcgcgtcctcaagaatgagcagtaa

SEQ ID NO: 5 - DNA, 961 bp, synthetic construct
  source 1..961: mol_type = other DNA
taatacgactcactatagggtaccacgtagaccgtacggcagtaataaccagctgaccgcatacccgagtaatggtgagcaagggcgaggagctgttcaccggggtggtgcccatcctggtcgagctggacggcgacgtaaacggccacaagttcagcgtgtccggcgagggcgagggcgatgccacctacggcaagctgaccctgaagttcatctgcaccaccggcaagctgcccgtgccctggcccaccctcgtgaccaccctgacctacggcgtgcagtgcttcagccgctaccccgaccacatgaagcagcacgacttcttcaagtccgccatgcccgaaggctacgtccaggagcgcaccatcttcttcaaggacgacggcaactacaagacccgcgccgaggtgaagttcgagggcgacaccctggtgaaccgcatcgagctgaagggcatcgacttcaaggaggacggcaacatcctggggcacaagctggagtacaactacaacagccacaacgtctatatcatggccgacaagcagaagaacggcatcaaggtgaacttcaagatccgccacaacatcgaggacggcagcgtgcagctcgccgaccactaccagcagaacacccccatcggcgacggccccgtgctgctgcccgacaaccactacctgagcacccagtccgccctgagcaaagaccccaacgagaagcgcgatcacatggtcctgctggagttcgtgaccgccgccgggatcactctcggcatggacgagctgtacaagtaatacgtattgccatgtgtatgtgggagacggtcgggtccagatattcgtatctgtcgagtagagtgtgggctcccacatactctgatgatccttcgggatcattcatggcaactcgagatagcataaaataacgccccaccttcttaacgggaggtggggcgttattttta

SEQ ID NO: 6 - RNA, 961 nt, synthetic construct
  source 1..961: mol_type = other RNA
taatacgactcactatagggtaccacgtagaccgtacggcagtaataaccagctgaccgcatacccgagtaatggtcagcaagggtgaggagctattcaccggagtagttcccatccttgttgagctggacggggacgtgaacgggcacaagttctccgtgagtggggagggcgagggtgacgccacgtacgggaagcttaccctgaagttcatctgtactacagggaagcttcccgtaccgtggcccaccctcgtcactaccctcacttacggagtgcagtgcttttcacgttaccccgaccacatgaagcagcatgacttcttcaagtcggccatgcctgaaggatacgtccaggagcggacgatattcttcaaagacgatgggaattataagacccgtgccgaggttaagttcgagggtgataccctcgtcaatagaatcgagctgaagggcatcgattttaaggaggacggtaacatcctcggacataagctcgagtacaattataattcccataacgtctacataatggccgacaagcagaagaatggtatcaaggtgaacttcaagatccggcacaacatcgaagatgggagtgttcagcttgctgatcactatcagcaaaacactcccatcggcgatgggccggtcttgttacctgataaccattacttgtccacccagagtgccctgtcgaaggatccgaacgaaaagcgggaccacatggtcctgcttgagttcgtgaccgcggcagggatcactctgggtatggacgagttatataagtaatacgtattgccatgtgtatgtgggagacggtcgggtccagatattcgtatctgtcgagtagagtgtgggctcccacatactctgatgatccttcgggatcattcatggcaactcgagatagcataaaataacgccccaccttcttaacgggaggtggggcgttattttta

SEQ ID NO: 7 - DNA, 1177 bp, synthetic construct
  source 1..1177: mol_type = other DNA
taatacgactcactatagggtaccacgtagaccgtacggcagtaataaccagctgaccgcatacccgagtaatggcttccaaggtgtacgaccccgagcaacgcaaacgcatgatcactgggcctcagtggtgggctcgctgcaagcaaatgaacgtgctggactccttcatcaactactatgattccgagaagcacgccgagaacgccgtgatttttctgcatggtaacgctgcctccagctacctgtggaggcacgtcgtgcctcacatcgagcccgtggctagatgcatcatccctgatctgatcggaatgggtaagtccggcaagagcgggaatggctcatatcgcctcctggatcactacaagtacctcaccgcttggttcgagctgctgaaccttccaaagaaaatcatctttgtgggccacgactggggggcttgtctggcctttcactactcctacgagcaccaagacaagatcaaggccatcgtccatgctgagagtgtcgtggacgtgatcgagtcctgggacgagtggcctgacatcgaggaggatatcgccctgatcaagagcgaagagggcgagaaaatggtgcttgagaataacttcttcgtcgagaccatgctcccaagcaagatcatgcggaaactggagcctgaggagttcgctgcctacctggagccattcaaggagaagggcgaggttagacggcctaccctctcctggcctcgcgagatccctctcgttaagggaggcaagcccgacgtcgtccagattgtccgcaactacaacgcctaccttcgggccagcgacgatctgcctaagatgttcatcgagtccgaccctgggttcttttccaacgctattgtcgagggagctaagaagttccctaacaccgagttcgtgaaggtgaagggcctccacttcagccaggaggacgctccagatgaaatgggtaagtacatcaagagcttcgtggagcgcgtgctgaagaacgagcagtaatacgtattgccatgtgtatgtgggagacggtcgggtccagatattcgtatctgtcgagtagagtgtgggctcccacatactctgatgatccttcgggatcattcatggcaactcgagatagcataaaataacgccccaccttcttaacgggaggtggggcgttattttta

SEQ ID NO: 8 - DNA, 1177 bp, synthetic construct
  source 1..1177: mol_type = other DNA
taatacgactcactatagggtaccacgtagaccgtacggcagtaataaccagctgaccgcatacccgagtaatggcgtccaaggtttacgaccctgagcagcggaagcgcatgatcacgggcccacagtggtgggcccgttgcaagcagatgaacgttctcgacagcttcatcaactattacgatagtgagaagcatgcagagaacgccgtcatcttcttgcacgggaatgcagcgagcagctatctatggcggcacgttgtgccgcacatagagcctgttgctcgctgcataatcccggaccttatagggatggggaagagcggtaagagcggcaacggctcttaccgccttctcgatcactataagtacttgacagcatggttcgagctcctcaatctgcccaagaagatcatcttcgttgggcacgattggggagcttgtctcgccttccattactcttacgagcaccaggacaagatcaaggccatcgtccacgcggagagcgtggtcgatgtgatcgagtcctgggatgagtggcccgatatcgaggaggatatcgcactcatcaagagtgaggaaggcgagaagatggtcctggagaataatttcttcgtggagaccatgctgccaagtaagatcatgcgcaagctcgagccggaggagtttgcggcgtacctcgagcccttcaaggagaagggcgaggtacgccgcccgactctctcctggcctcgagagatcccgctggtcaagggtggtaagccggacgtcgtgcagatagtgcgtaactacaacgcctatctgcgggcaagtgacgacttgcccaagatgttcattgagagcgaccccggcttcttctcgaacgccattgttgagggagctaagaagttccccaacacggagttcgtgaaggtgaaggggttgcatttcagtcaggaggacgcgcccgacgaaatgggcaagtacatcaagtccttcgtcgagcgcgtcctcaagaatgagcagtaatacgtattgccatgtgtatgtgggagacggtcgggtccagatattcgtatctgtcgagtagagtgtgggctcccacatactctgatgatccttcgggatcattcatggcaactcgagatagcataaaataacgccccaccttcttaacgggaggtggggcgttattttta

SEQ ID NO: 9 - DNA, 5794 bp, synthetic construct
  source 1..5794: mol_type = other DNA
ggatccctcgagctgcaggatatccatatggtgagcaagggcgaggagctgttcaccggggtggtgcccatcctggtcgagctggacggcgacgtaaacggccacaagttcagcgtgtccggcgagggcgagggcgatgccacctacggcaagctgaccctgaagctgatctgcaccaccggcaagctgcccgtgccctggcccaccctcgtgaccaccctgggctacggcctgcagtgcttcgcccgctaccccgaccacatgaagcagcacgacttcttcaagtccgccatgcccgaaggctacgtccaggagcgcaccatcttcttcaaggacgacggcaactacaagacccgcgccgaggtgaagttcgagggcgacaccctggtgaaccgcatcgagctgaagggcatcgacttcaaggaggacggcaacatcctggggcacaagctggagtacaactacaacagccacaacgtctatatcaccgccgacaagcagaagaacggcatcaaggccaacttcaagatccgccacaacatcgaggacggcggcgtgcagctcgccgaccactaccagcagaacacccccatcggcgacggccccgtgctgctgcccgacaaccactacctgagctaccagtccgccctgagcaaagaccccaacgagaagcgcgatcacatggtcctgctggagttcgtgaccgccgccgggatcactctcggcatggacgagctgtacaagtaacatatggatatctgtcgacggccgtcgttttacagccaagcttggctgttttggcggatgagagaagattttcagcctgatacagattaaatcagaacgcagaagcggtctgataaaacagaatttgcctggcggcagtagcgcggtggtcccacctgaccccatgccgaactcagaagtgaaacgccgtagcgccgatggtagtgtggggtctccccatgcgagagtagggaactgccaggcatcaaataaaacgaaaggctcagtcgaaagactgggcctttcgttttatctgttgtttgtcggtgaacgctctcctgagtaggacaaatccgccgggagcggatttgaacgttgcgaagcaacggcccggagggtggcgggcaggacgcccgccataaactgccaggcatcaaattaagcagaaggccatcctgacggatggcctttttgcgtttctacaaactcttttggtcgactctagagttccactgagcgtcagaccccgtagaaaagatcaaaggatcttcttgagatcctttttttctgcgcgtaatctgctgcttgcaaacaaaaaaaccaccgctaccagcggtggtttgtttgccggatcaagagctaccaactctttttccgaaggtaactggcttcagcagagcgcagataccaaatactgttcttctagtgtagccgtagttaggccaccacttcaagaactctgtagcaccgcctacatacctcgctctgctaatcctgttaccagtggctgctgccagtggcgataagtcgtgtcttaccgggttggactcaagacgatagttaccggataaggcgcagcggtcgggctgaacggggggttcgtgcacacagcccagcttggagcgaacgacctacaccgaactgagatacctacagcgtgagctatgagaaagcgccacgcttcccgaagggagaaaggcggacaggtatccggtaagcggcagggtcggaacaggagagcgcacgagggagcttccagggggaaacgcctggtatctttatagtcctgtcgggtttcgccacctctgacttgagcgtcgatttttgtgatgctcgtcaggggggcggagcctatggaaaaacgccagcaacgcggcctttttacggttcctggccttttgctggccttttgctcacatgttctttcctgcgttatcccctgattctgtggataaccgtattaccgcctttgagtgagctgataccgctcgccgcagccgaacgaccgagcgcagcgagtcagtgagcgaggaagcggaagatctagaagtactgctgactcataccaggcctgaatcgccccatcatccagccagaaagtgagggagccacggttgatgagagctttgttgtaggtggaccagttggtgattttgaacttttgctttgccacggaacggtctgcgttgtcgggaagatgcgtgatctgatccttcaactcagcaaaagttcgatttattcaacaaagccacgttgtgtctcaaaatctctgatgttacattgcacaagataaaaatatatcatcatgaacaataaaactgtctgcttacataaacagtaatacaaggggtgttatgagccatattcaacgggaaacgtcttgctcaaggccgcgattaaattccaacatggatgctgatttatatgggtataaatgggctcgcgataatgtcgggcaatcaggtgcgacaatctatcgattgtatgggaagcccgatgcgccagagttgtttctgaaacatggcaaaggtagcgttgccaatgatgttacagatgagatggtcagactaaactggctgacggaatttatgcctcttccgaccatcaagcattttatccgtactcctgatgatgcatggttactcaccactgcgatccccggaaaaacagcattccaggtattagaagaatatcctgattcaggtgaaaatattgttgatgcgctggcagtgttcctgcgccggttgcattcgattcctgtttgtaattgtccttttaacagcgatcgcgtatttcgtctcgctcaggcgcaatcacgaatgaataacggtttggttgatgcgagtgattttgatgacgagcgtaatggctggcctgttgaacaagtctggaaagaaatgcataagcttttgccattctcaccggattcagtcgtcactcatggtgatttctcacttgataaccttatttttgacgaggggaaattaataggttgtattgatgttggacgagtcggaatcgcagaccgataccaggatcttgccatcctatggaactgcctcggtgagttttctccttcattacagaaacggctttttcaaaaatatggtattgataatcctgatatgaataaattgcagtttcatttgatgctcgatgagtttttctaaggctagccccgggactagtgatctttgggagcagtccttgtgcgcttacgaggtgagccggtggggaaccgttatctgcctatggtgtgagcccccctagagagcttcaagagcaatcagcccgacctagaaaggaggccaagagagagacccctacggggggaaccgttttctgcctacgagatggcacatttactgggaagctttacggcgtcctcgtggaagttcaatgcccgcagacttaagtgctctattcacggtctgacgtgacacgctaaattcagacatagcttcattgattgtcggccacgagccagtctctccctcaacagtcataaaccaacctgcaatggtcaagcgattttctttagctttcctagcttgtcgttgactggacttagctagtttttctcgctgtgctcgggcgtactcactgtttgggtctttccagcgttctgcggcctttttaccgccacgtcttcccatagtggccagagcttttcgccctcggctgctctgcgtctctgtctgacgagcagggacgactggctggcctttagcgacgtagccgcgcacacgtcgcgccatcgtctggcggtcacgcatcggcggcagatcaggctcacggccgtctgctccgaccgcctgagcgacggtgtaggcacgctcgtaggcgtcgatgatcttggtgtcttttaggcgctcaccagccgcttttaactggtatcccacagtcaaagcgtggcgaaaagccgtctcatcacgggcggcacgccctggagcagtccagaggacacggacgccgtcgatcagctctccagacgcttcagcggcgctcggcaggcttgcttcaagcgtggcaagtgcttttgcttccgcagtggcttttcttgccgcttcgatacgtgcccgtccgctagaaaactcctgctcatagcgttttttaggtttttctgtgcctgagatcatgcgagcaacctccataagatcagctaggcgatccacgcgattgtgctgggcatgccagcggtacgcggtgggatcgtcggagacgtgcagtggccaccggctcagcctatgtgaaaaagcctggtcagcgccgaaaacgcgggtcatttcctcggtcgttgcagccagcaggcgcatattcgggctgctcatgcctgctgcggcatacaccggatcaatgagccagatgagctggcatttcccgctcagtggattcacgccgatccaagctggcgctttttccaggcgtgcccagcgctccaaaatcgcgtagacctcggggtttacgtgctcgattttcccgccggcctggtggctcggcacatcaatgtccaggacaagcacggctgcgtgctgcgcgtgcgtcagagcaacatactggcaccgggcaagcgattttgaaccaactcggtataacttcggctgtgtttctcccgtgtccgggtctttgatccaagcgctggcgaagtcgcgggtcttgctgccctggaaattttctctgcccaggtgagcgaggaattcgcggcggtcttcgctcgtccagccacgtgatcgcagcgcgagctcgggatgggtgtcgaacagatcagcggaaaatttccaggccggtgtgtcaatgtctcgtgaatccgctagagtcatttttgagcgctttctcccaggtttggactgggggttagccgacgccctgtgagttaccgctcacggggcgttcaacatttttcaggtattcgtgcagcttatcgcttcttgccgcctgtgcgctttttcgacgcgcgacgctgctgccgattcggtgcaggtggtggcggcgctgacacgtcctgggcggccacggccacacgaaacgcggcatttacgatgtttgtcatgcctgcgggcaccgcgccacgatcgcggataattctcgctgccgcttccagctctgtgacgaccatggccaaaatttcgctcgggggacgcacttccagcgccatttgcgacctagccgcctccagctcctcggcgtggcgtttgttggcgcgctcgcggctggctgcggcacgacacgcatctgagcaatattttgcgcgccgtcctcgcgggtcaggccggggaggaatcaggccaccgcagtaggcgcaactgattcgatcctccactactgtgcgtcctcctggcgctgccgagcacgcagctcgtcagccagctcctcaagatccgccacgagagtttctaggtcgctcgcggcactggcccagtctcgtgatgctggcgcgtccgtcgtatcgagagctcggaaaaatccgatcaccgtttttaaatcgacggcagcatcgagcgcgtcggactccagcgcgacatcagagagatccatagctgatgattcgggccaattttggtacttcgtcgtgaaggtcatgacaccattataacgaacgttcgttaaagtttttggcggaaaatcacgcggcacgaaaattttcacgaagcgggactttgcgcagctcaggggtgctaaaaattttgtatcgcacttgatttttccgaaagacagattatctgcaaacggtgtgtcgtatttctggcttggtttttaaaaaatctggaatcgaaaatttgcggggcga

SEQ ID NO: 10 - DNA, 6027 bp, synthetic construct
  source 1..6027: mol_type = other DNA
gatcctagtactcagctgtaatacgactcactatagggtaccacgtagaccgtacggcagtaataaccagctgaccgcatacccgagtaatggtgagcaagggcgaggagctgttcaccggggtggtgcccatcctggtcgagctggacggcgacgtaaacggccacaagttcagcgtgtccggcgagggcgagggcgatgccacctacggcaagctgaccctgaagttcatctgcaccaccggcaagctgcccgtgccctggcccaccctcgtgaccaccctgacctacggcgtgcagtgcttcagccgctaccccgaccacatgaagcagcacgacttcttcaagtccgccatgcccgaaggctacgtccaggagcgcaccatcttcttcaaggacgacggcaactacaagacccgcgccgaggtgaagttcgagggcgacaccctggtgaaccgcatcgagctgaagggcatcgacttcaaggaggacggcaacatcctggggcacaagctggagtacaactacaacagccacaacgtctatatcatggccgacaagcagaagaacggcatcaaggtgaacttcaagatccgccacaacatcgaggacggcagcgtgcagctcgccgaccactaccagcagaacacccccatcggcgacggccccgtgctgctgcccgacaaccactacctgagcacccagtccgccctgagcaaagaccccaacgagaagcgcgatcacatggtcctgctggagttcgtgaccgccgccgggatcactctcggcatggacgagctgtacaagtaatacgtattgccatgtgtatgtgggagacggtcgggtccagatattcgtatctgtcgagtagagtgtgggctcccacatactctgatgatccttcgggatcattcatggcaactcgagatagcataaaataacgccccaccttcttaacgggaggtggggcgttatttttactgaaagatatctgtcgacggccgtcgttttacagccaagcttggctgttttggcggatgagagaagattttcagcctgatacagattaaatcagaacgcagaagcggtctgataaaacagaatttgcctggcggcagtagcgcggtggtcccacctgaccccatgccgaactcagaagtgaaacgccgtagcgccgatggtagtgtggggtctccccatgcgagagtagggaactgccaggcatcaaataaaacgaaaggctcagtcgaaagactgggcctttcgttttatctgttgtttgtcggtgaacgctctcctgagtaggacaaatccgccgggagcggatttgaacgttgcgaagcaacggcccggagggtggcgggcaggacgcccgccataaactgccaggcatcaaattaagcagaaggccatcctgacggatggcctttttgcgtttctacaaactcttttggtcgactctagagttccactgagcgtcagaccccgtagaaaagatcaaaggatcttcttgagatcctttttttctgcgcgtaatctgctgcttgcaaacaaaaaaaccaccgctaccagcggtggtttgtttgccggatcaagagctaccaactctttttccgaaggtaactggcttcagcagagcgcagataccaaatactgtccttctagtgtagccgtagttaggccaccacttcaagaactctgtagcaccgcctacatacctcgctctgctaatcctgttaccagtggctgctgccagtggcgataagtcgtgtcttaccgggttggactcaagacgatagttaccggataaggcgcagcggtcgggctgaacggggggttcgtgcacacagcccagcttggagcgaacgacctacaccgaactgagatacctacagcgtgagctatgagaaagcgccacgcttcccgaagggagaaaggcggacaggtatccggtaagcggcagggtcggaacaggagagcgcacgagggagcttccagggggaaacgcctggtatctttatagtcctgtcgggtttcgccacctctgacttgagcgtcgatttttgtgatgctcgtcaggggggcggagcctatggaaaaacgccagcaacgcggcctttttacggttcctggccttttgctggccttttgctcacatgttctttcctgcgttatcccctgattctgtggataaccgtattaccgcctttgagtgagctgataccgctcgccgcagccgaacgaccgagcgcagcgagtcagtgagcgaggaagcggaagatctagaagtactgctgactcataccaggcctgaatcgccccatcatccagccagaaagtgagggagccacggttgatgagagctttgttgtaggtggaccagttggtgattttgaacttttgctttgccacggaacggtctgcgttgtcgggaagatgcgtgatctgatccttcaactcagcaaaagttcgatttattcaacaaagccacgttgtgtctcaaaatctctgatgttacattgcacaagataaaaatatatcatcatgaacaataaaactgtctgcttacataaacagtaatacaaggggtgttatgagccatattcaacgggaaacgtcttgctcaaggccgcgattaaattccaacatggatgctgatttatatgggtataaatgggctcgcgataatgtcgggcaatcaggtgcgacaatctatcgattgtatgggaagcccgatgcgccagagttgtttctgaaacatggcaaaggtagcgttgccaatgatgttacagatgagatggtcagactaaactggctgacggaatttatgcctcttccgaccatcaagcattttatccgtactcctgatgatgcatggttactcaccactgcgatccccggaaaaacagcattccaggtattagaagaatatcctgattcaggtgaaaatattgttgatgcgctggcagtgttcctgcgccggttgcattcgattcctgtttgtaattgtccttttaacagcgatcgcgtatttcgtctcgctcaggcgcaatcacgaatgaataacggtttggttgatgcgagtgattttgatgacgagcgtaatggctggcctgttgaacaagtctggaaagaaatgcataagcttttgccattctcaccggattcagtcgtcactcatggtgatttctcacttgataaccttatttttgacgaggggaaattaataggttgtattgatgttggacgagtcggaatcgcagaccgataccaggatcttgccatcctatggaactgcctcggtgagttttctccttcattacagaaacggctttttcaaaaatatggtattgataatcctgatatgaataaattgcagtttcatttgatgctcgatgagtttttctaaggctagccccgggactagtgatctttgggagcagtccttgtgcgcttacgaggtgagccggtggggaaccgttatctgcctatggtgtgagcccccctagagagcttcaagagcaatcagcccgacctagaaaggaggccaagagagagacccctacggggggaaccgttttctgcctacgagatggcacatttactgggaagctttacggcgtcctcgtggaagttcaatgcccgcagacttaagtgctctattcacggtctgacgtgacacgctaaattcagacatagcttcattgattgtcggccacgagccagtctctccctcaacagtcataaaccaacctgcaatggtcaagcgattttctttagctttcctagcttgtcgttgactggacttagctagtttttctcgctgtgctcgggcgtactcactgtttgggtctttccagcgttctgcggcctttttaccgccacgtcttcccatagtggccagagcttttcgccctcggctgctctgcgtctctgtctgacgagcagggacgactggctggcctttagcgacgtagccgcgcacacgtcgcgccatcgtctggcggtcacgcatcggcggcagatcaggctcacggccgtctgctccgaccgcctgagcgacggtgtaggcacgctcgtaggcgtcgatgatcttggtgtcttttaggcgctcaccagccgcttttaactggtatcccacagtcaaagcgtggcgaaaagccgtctcatcacgggcggcacgccctggagcagtccagaggacacggacgccgtcgatcagctctccagacgcttcagcggcgctcggcaggcttgcttcaagcgtggcaagtgcttttgcttccgcagtggcttttcttgccgcttcgatacgtgcccgtccgctagaaaactcctgctcatagcgttttttaggtttttctgtgcctgagatcatgcgagcaacctccataagatcagctaggcgatccacgcgattgtgctgggcatgccagcggtacgcggtgggatcgtcggagacgtgcagtggccaccggctcagcctatgtgaaaaagcctggtcagcgccgaaaacgcgggtcatttcctcggtcgttgcagccagcaggcgcatattcgggctgctcatgcctgctgcggcatacaccggatcaatgagccagatgagctggcatttcccgctcagtggattcacgccgatccaagctggcgctttttccaggcgtgcccagcgctccaaaatcgcgtagacctcggggtttacgtgctcgattttcccgccggcctggtggctcggcacatcaatgtccaggacaagcacggctgcgtgctgcgcgtgcgtcagagcaacatactggcaccgggcaagcgattttgaaccaactcggtataacttcggctgtgtttctcccgtgtccgggtctttgatccaagcgctggcgaagtcgcgggtcttgctgccctggaaattttctctgcccaggtgagcgaggaattcgcggcggtcttcgctcgtccagccacgtgatcgcagcgcgagctcgggatgggtgtcgaacagatcagcggaaaatttccaggccggtgtgtcaatgtctcgtgaatccgctagagtcatttttgagcgctttctcccaggtttggactgggggttagccgacgccctgtgagttaccgctcacggggcgttcaacatttttcaggtattcgtgcagcttatcgcttcttgccgcctgtgcgctttttcgacgcgcgacgctgctgccgattcggtgcaggtggtggcggcgctgacacgtcctgggcggccacggccacacgaaacgcggcatttacgatgtttgtcatgcctgcgggcaccgcgccacgatcgcggataattctcgctgccgcttccagctctgtgacgaccatggccaaaatttcgctcgggggacgcacttccagcgccatttgcgacctagccgcctccagctcctcggcgtggcgtttgttggcgcgctcgcggctggctgcggcacgacacgcatctgagcaatattttgcgcgccgtcctcgcgggtcaggccggggaggaatcaggccaccgcagtaggcgcaactgattcgatcctccactactgtgcgtcctcctggcgctgccgagcacgcagctcgtcagccagctcctcaagatccgccacgagagtttctaggtcgctcgcggcactggcccagtctcgtgatgctggcgcgtccgtcgtatcgagagctcggaaaaatccgatcaccgtttttaaatcgacggcagcatcgagcgcgtcggactccagcgcgacatcagagagatccatagctgatgattcgggccaattttggtacttcgtcgtgaaggtcatgacaccattataacgaacgttcgttaaagtttttggcggaaaatcacgcggcacgaaaattttcacgaagcgggactttgcgcagctcaggggtgctaaaaattttgtatcgcacttgatttttccgaaagacagattatctgcaaacggtgtgtcgtatttctggcttggtttttaaaaaatctggaatcgaaaatttgcggggcgag

SEQ ID NO: 11 - DNA, 6034 bp, synthetic construct
  source 1..6034: mol_type = other DNA
gtagtactcagctgtaatacgactcactatagggtaccacgtagaccgtacggcagtaataaccagctgaccgcatacccgagtaatggtcagcaagggtgaggagctattcaccggagtagttcccatccttgttgagctggacggggacgtgaacgggcacaagttctccgtgagtggggagggcgagggtgacgccacgtacgggaagcttaccctgaagttcatctgtactacagggaagcttcccgtaccgtggcccaccctcgtcactaccctcacttacggagtgcagtgcttttcacgttaccccgaccacatgaagcagcatgacttcttcaagtcggccatgcctgaaggatacgtccaggagcggacgatattcttcaaagacgatgggaattataagacccgtgccgaggttaagttcgagggtgataccctcgtcaatagaatcgagctgaagggcatcgattttaaggaggacggtaacatcctcggacataagctcgagtacaattataattcccataacgtctacataatggccgacaagcagaagaatggtatcaaggtgaacttcaagatccggcacaacatcgaagatgggagtgttcagcttgctgatcactatcagcaaaacactcccatcggcgatgggccggtcttgttacctgataaccattacttgtccacccagagtgccctgtcgaaggatccgaacgaaaagcgggaccacatggtcctgcttgagttcgtgaccgcggcagggatcactctgggtatggacgagttatataagtaatacgtattgccatgtgtatgtgggagacggtcgggtccagatattcgtatctgtcgagtagagtgtgggctcccacatactctgatgatccttcgggatcattcatggcaactcgagatagcataaaataacgccccaccttcttaacgggaggtggggcgttatttttactgaaagatatcatccaatggatctgtcgacggccgtcgttttacagccaagcttggctgttttggcggatgagagaagattttcagcctgatacagattaaatcagaacgcagaagcggtctgataaaacagaatttgcctggcggcagtagcgcggtggtcccacctgaccccatgccgaactcagaagtgaaacgccgtagcgccgatggtagtgtggggtctccccatgcgagagtagggaactgccaggcatcaaataaaacgaaaggctcagtcgaaagactgggcctttcgttttatctgttgtttgtcggtgaacgctctcctgagtaggacaaatccgccgggagcggatttgaacgttgcgaagcaacggcccggagggtggcgggcaggacgcccgccataaactgccaggcatcaaattaagcagaaggccatcctgacggatggcctttttgcgtttctacaaactcttttggtcgactctagagttccactgagcgtcagaccccgtagaaaagatcaaaggatcttcttgagatcctttttttctgcgcgtaatctgctgcttgcaaacaaaaaaaccaccgctaccagcggtggtttgtttgccggatcaagagctaccaactctttttccgaaggtaactggcttcagcagagcgcagataccaaatactgtccttctagtgtagccgtagttaggccaccacttcaagaactctgtagcaccgcctacatacctcgctctgctaatcctgttaccagtggctgctgccagtggcgataagtcgtgtcttaccgggttggactcaagacgatagttaccggataaggcgcagcggtcgggctgaacggggggttcgtgcacacagcccagcttggagcgaacgacctacaccgaactgagatacctacagcgtgagctatgagaaagcgccacgcttcccgaagggagaaaggcggacaggtatccggtaagcggcagggtcggaacaggagagcgcacgagggagcttccagggggaaacgcctggtatctttatagtcctgtcgggtttcgccacctctgacttgagcgtcgatttttgtgatgctcgtcaggggggcggagcctatggaaaaacgccagcaacgcggcctttttacggttcctggccttttgctggccttttgctcacatgttctttcctgcgttatcccctgattctgtggataaccgtattaccgcctttgagtgagctgataccgctcgccgcagccgaacgaccgagcgcagcgagtcagtgagcgaggaagcggaagatctagaagtactgctgactcataccaggcctgaatcgccccatcatccagccagaaagtgagggagccacggttgatgagagctttgttgtaggtggaccagttggtgattttgaacttttgctttgccacggaacggtctgcgttgtcgggaagatgcgtgatctgatccttcaactcagcaaaagttcgatttattcaacaaagccacgttgtgtctcaaaatctctgatgttacattgcacaagataaaaatatatcatcatgaacaataaaactgtctgcttacataaacagtaatacaaggggtgttatgagccatattcaacgggaaacgtcttgctcaaggccgcgattaaattccaacatggatgctgatttatatgggtataaatgggctcgcgataatgtcgggcaatcaggtgcgacaatctatcgattgtatgggaagcccgatgcgccagagttgtttctgaaacatggcaaaggtagcgttgccaatgatgttacagatgagatggtcagactaaactggctgacggaatttatgcctcttccgaccatcaagcattttatccgtactcctgatgatgcatggttactcaccactgcgatccccggaaaaacagcattccaggtattagaagaatatcctgattcaggtgaaaatattgttgatgcgctggcagtgttcctgcgccggttgcattcgattcctgtttgtaattgtccttttaacagcgatcgcgtatttcgtctcgctcaggcgcaatcacgaatgaataacggtttggttgatgcgagtgattttgatgacgagcgtaatggctggcctgttgaacaagtctggaaagaaatgcataagcttttgccattctcaccggattcagtcgtcactcatggtgatttctcacttgataaccttatttttgacgaggggaaattaataggttgtattgatgttggacgagtcggaatcgcagaccgataccaggatcttgccatcctatggaactgcctcggtgagttttctccttcattacagaaacggctttttcaaaaatatggtattgataatcctgatatgaataaattgcagtttcatttgatgctcgatgagtttttctaaggctagccccgggactagtgatctttgggagcagtccttgtgcgcttacgaggtgagccggtggggaaccgttatctgcctatggtgtgagcccccctagagagcttcaagagcaatcagcccgacctagaaaggaggccaagagagagacccctacggggggaaccgttttctgcctacgagatggcacatttactgggaagctttacggcgtcctcgtggaagttcaatgcccgcagacttaagtgctctattcacggtctgacgtgacacgctaaattcagacatagcttcattgattgtcggccacgagccagtctctccctcaacagtcataaaccaacctgcaatggtcaagcgattttctttagctttcctagcttgtcgttgactggacttagctagtttttctcgctgtgctcgggcgtactcactgtttgggtctttccagcgttctgcggcctttttaccgccacgtcttcccatagtggccagagcttttcgccctcggctgctctgcgtctctgtctgacgagcagggacgactggctggcctttagcgacgtagccgcgcacacgtcgcgccatcgtctggcggtcacgcatcggcggcagatcaggctcacggccgtctgctccgaccgcctgagcgacggtgtaggcacgctcgtaggcgtcgatgatcttggtgtcttttaggcgctcaccagccgcttttaactggtatcccacagtcaaagcgtggcgaaaagccgtctcatcacgggcggcacgccctggagcagtccagaggacacggacgccgtcgatcagctctccagacgcttcagcggcgctcggcaggcttgcttcaagcgtggcaagtgcttttgcttccgcagtggcttttcttgccgcttcgatacgtgcccgtccgctagaaaactcctgctcatagcgttttttaggtttttctgtgcctgagatcatgcgagcaacctccataagatcagctaggcgatccacgcgattgtgctgggcatgccagcggtacgcggtgggatcgtcggagacgtgcagtggccaccggctcagcctatgtgaaaaagcctggtcagcgccgaaaacgcgggtcatttcctcggtcgttgcagccagcaggcgcatattcgggctgctcatgcctgctgcggcatacaccggatcaatgagccagatgagctggcatttcccgctcagtggattcacgccgatccaagctggcgctttttccaggcgtgcccagcgctccaaaatcgcgtagacctcggggtttacgtgctcgattttcccgccggcctggtggctcggcacatcaatgtccaggacaagcacggctgcgtgctgcgcgtgcgtcagagcaacatactggcaccgggcaagcgattttgaaccaactcggtataacttcggctgtgtttctcccgtgtccgggtctttgatccaagcgctggcgaagtcgcgggtcttgctgccctggaaattttctctgcccaggtgagcgaggaattcgcggcggtcttcgctcgtccagccacgtgatcgcagcgcgagctcgggatgggtgtcgaacagatcagcggaaaatttccaggccggtgtgtcaatgtctcgtgaatccgctagagtcatttttgagcgctttctcccaggtttggactgggggttagccgacgccctgtgagttaccgctcacggggcgttcaacatttttcaggtattcgtgcagcttatcgcttcttgccgcctgtgcgctttttcgacgcgcgacgctgctgccgattcggtgcaggtggtggcggcgctgacacgtcctgggcggccacggccacacgaaacgcggcatttacgatgtttgtcatgcctgcgggcaccgcgccacgatcgcggataattctcgctgccgcttccagctctgtgacgaccatggccaaaatttcgctcgggggacgcacttccagcgccatttgcgacctagccgcctccagctcctcggcgtggcgtttgttggcgcgctcgcggctggctgcggcacgacacgcatctgagcaatattttgcgcgccgtcctcgcgggtcaggccggggaggaatcaggccaccgcagtaggcgcaactgattcgatcctccactactgtgcgtcctcctggcgctgccgagcacgcagctcgtcagccagctcctcaagatccgccacgagagtttctaggtcgctcgcggcactggcccagtctcgtgatgctggcgcgtccgtcgtatcgagagctcggaaaaatccgatcaccgtttttaaatcgacggcagcatcgagcgcgtcggactccagcgcgacatcagagagatccatagctgatgattcgggccaattttggtacttcgtcgtgaaggtcatgacaccattataacgaacgttcgttaaagtttttggcggaaaatcacgcggcacgaaaattttcacgaagcgggactttgcgcagctcaggggtgctaaaaattttgtatcgcacttgatttttccgaaagacagattatctgcaaacggtgtgtcgtatttctggcttggtttttaaaaaatctggaatcgaaaatttgcggggcga

SEQ ID NO: 12 - DNA, 6250 bp, synthetic construct
  source 1..6250: mol_type = other DNA
gtagtactcagctgtaatacgactcactatagggtaccacgtagaccgtacggcagtaataaccagctgaccgcatacccgagtaatggcttccaaggtgtacgaccccgagcaacgcaaacgcatgatcactgggcctcagtggtgggctcgctgcaagcaaatgaacgtgctggactccttcatcaactactatgattccgagaagcacgccgagaacgccgtgatttttctgcatggtaacgctgcctccagctacctgtggaggcacgtcgtgcctcacatcgagcccgtggctagatgcatcatccctgatctgatcggaatgggtaagtccggcaagagcgggaatggctcatatcgcctcctggatcactacaagtacctcaccgcttggttcgagctgctgaaccttccaaagaaaatcatctttgtgggccacgactggggggcttgtctggcctttcactactcctacgagcaccaagacaagatcaaggccatcgtccatgctgagagtgtcgtggacgtgatcgagtcctgggacgagtggcctgacatcgaggaggatatcgccctgatcaagagcgaagagggcgagaaaatggtgcttgagaataacttcttcgtcgagaccatgctcccaagcaagatcatgcggaaactggagcctgaggagttcgctgcctacctggagccattcaaggagaagggcgaggttagacggcctaccctctcctggcctcgcgagatccctctcgttaagggaggcaagcccgacgtcgtccagattgtccgcaactacaacgcctaccttcgggccagcgacgatctgcctaagatgttcatcgagtccgaccctgggttcttttccaacgctattgtcgagggagctaagaagttccctaacaccgagttcgtgaaggtgaagggcctccacttcagccaggaggacgctccagatgaaatgggtaagtacatcaagagcttcgtggagcgcgtgctgaagaacgagcagtaatacgtattgccatgtgtatgtgggagacggtcgggtccagatattcgtatctgtcgagtagagtgtgggctcccacatactctgatgatccttcgggatcattcatggcaactcgagatagcataaaataacgccccaccttcttaacgggaggtggggcgttatttttactgaaagatatcatccaatggatctgtcgacggccgtcgttttacagccaagcttggctgttttggcggatgagagaagattttcagcctgatacagattaaatcagaacgcagaagcggtctgataaaacagaatttgcctggcggcagtagcgcggtggtcccacctgaccccatgccgaactcagaagtgaaacgccgtagcgccgatggtagtgtggggtctccccatgcgagagtagggaactgccaggcatcaaataaaacgaaaggctcagtcgaaagactgggcctttcgttttatctgttgtttgtcggtgaacgctctcctgagtaggacaaatccgccgggagcggatttgaacgttgcgaagcaacggcccggagggtggcgggcaggacgcccgccataaactgccaggcatcaaattaagcagaaggccatcctgacggatggcctttttgcgtttctacaaactcttttggtcgactctagagttccactgagcgtcagaccccgtagaaaagatcaaaggatcttcttgagatcctttttttctgcgcgtaatctgctgcttgcaaacaaaaaaaccaccgctaccagcggtggtttgtttgccggatcaagagctaccaactctttttccgaaggtaactggcttcagcagagcgcagataccaaatactgtccttctagtgtagccgtagttaggccaccacttcaagaactctgtagcaccgcctacatacctcgctctgctaatcctgttaccagtggctgctgccagtggcgataagtcgtgtcttaccgggttggactcaagacgatagttaccggataaggcgcagcggtcgggctgaacggggggttcgtgcacacagcccagcttggagcgaacgacctacaccgaactgagatacctacagcgtgagctatgagaaagcgccacgcttcccgaagggagaaaggcggacaggtatccggtaagcggcagggtcggaacaggagagcgcacgagggagcttccagggggaaacgcctggtatctttatagtcctgtcgggtttcgccacctctgacttgagcgtcgatttttgtgatgctcgtcaggggggcggagcctatggaaaaacgccagcaacgcggcctttttacggttcctggccttttgctggccttttgctcacatgttctttcctgcgttatcccctgattctgtggataaccgtattaccgcctttgagtgagctgataccgctcgccgcagccgaacgaccgagcgcagcgagtcagtgagcgaggaagcggaagatctagaagtactgctgactcataccaggcctgaatcgccccatcatccagccagaaagtgagggagccacggttgatgagagctttgttgtaggtggaccagttggtgattttgaacttttgctttgccacggaacggtctgcgttgtcgggaagatgcgtgatctgatccttcaactcagcaaaagttcgatttattcaacaaagccacgttgtgtctcaaaatctctgatgttacattgcacaagataaaaatatatcatcatgaacaataaaactgtctgcttacataaacagtaatacaaggggtgttatgagccatattcaacgggaaacgtcttgctcaaggccgcgattaaattccaacatggatgctgatttatatgggtataaatgggctcgcgataatgtcgggcaatcaggtgcgacaatctatcgattgtatgggaagcccgatgcgccagagttgtttctgaaacatggcaaaggtagcgttgccaatgatgttacagatgagatggtcagactaaactggctgacggaatttatgcctcttccgaccatcaagcattttatccgtactcctgatgatgcatggttactcaccactgcgatccccggaaaaacagcattccaggtattagaagaatatcctgattcaggtgaaaatattgttgatgcgctggcagtgttcctgcgccggttgcattcgattcctgtttgtaattgtccttttaacagcgatcgcgtatttcgtctcgctcaggcgcaatcacgaatgaataacggtttggttgatgcgagtgattttgatgacgagcgtaatggctggcctgttgaacaagtctggaaagaaatgcataagcttttgccattctcaccggattcagtcgtcactcatggtgatttctcacttgataaccttatttttgacgaggggaaattaataggttgtattgatgttggacgagtcggaatcgcagaccgataccaggatcttgccatcctatggaactgcctcggtgagttttctccttcattacagaaacggctttttcaaaaatatggtattgataatcctgatatgaataaattgcagtttcatttgatgctcgatgagtttttctaaggctagccccgggactagtgatctttgggagcagtccttgtgcgcttacgaggtgagccggtggggaaccgttatctgcctatggtgtgagcccccctagagagcttcaagagcaatcagcccgacctagaaaggaggccaagagagagacccctacggggggaaccgttttctgcctacgagatggcacatttactgggaagctttacggcgtcctcgtggaagttcaatgcccgcagacttaagtgctctattcacggtctgacgtgacacgctaaattcagacatagcttcattgattgtcggccacgagccagtctctccctcaacagtcataaaccaacctgcaatggtcaagcgattttctttagctttcctagcttgtcgttgactggacttagctagtttttctcgctgtgctcgggcgtactcactgtttgggtctttccagcgttctgcggcctttttaccgccacgtcttcccatagtggccagagcttttcgccctcggctgctctgcgtctctgtctgacgagcagggacgactggctggcctttagcgacgtagccgcgcacacgtcgcgccatcgtctggcggtcacgcatcggcggcagatcaggctcacggccgtctgctccgaccgcctgagcgacggtgtaggcacgctcgtaggcgtcgatgatcttggtgtcttttaggcgctcaccagccgcttttaactggtatcccacagtcaaagcgtggcgaaaagccgtctcatcacgggcggcacgccctggagcagtccagaggacacggacgccgtcgatcagctctccagacgcttcagcggcgctcggcaggcttgcttcaagcgtggcaagtgcttttgcttccgcagtggcttttcttgccgcttcgatacgtgcccgtccgctagaaaactcctgctcatagcgttttttaggtttttctgtgcctgagatcatgcgagcaacctccataagatcagctaggcgatccacgcgattgtgctgggcatgccagcggtacgcggtgggatcgtcggagacgtgcagtggccaccggctcagcctatgtgaaaaagcctggtcagcgccgaaaacgcgggtcatttcctcggtcgttgcagccagcaggcgcatattcgggctgctcatgcctgctgcggcatacaccggatcaatgagccagatgagctggcatttcccgctcagtggattcacgccgatccaagctggcgctttttccaggcgtgcccagcgctccaaaatcgcgtagacctcggggtttacgtgctcgattttcccgccggcctggtggctcggcacatcaatgtccaggacaagcacggctgcgtgctgcgcgtgcgtcagagcaacatactggcaccgggcaagcgattttgaaccaactcggtataacttcggctgtgtttctcccgtgtccgggtctttgatccaagcgctggcgaagtcgcgggtcttgctgccctggaaattttctctgcccaggtgagcgaggaattcgcggcggtcttcgctcgtccagccacgtgatcgcagcgcgagctcgggatgggtgtcgaacagatcagcggaaaatttccaggccggtgtgtcaatgtctcgtgaatccgctagagtcatttttgagcgctttctcccaggtttggactgggggttagccgacgccctgtgagttaccgctcacggggcgttcaacatttttcaggtattcgtgcagcttatcgcttcttgccgcctgtgcgctttttcgacgcgcgacgctgctgccgattcggtgcaggtggtggcggcgctgacacgtcctgggcggccacggccacacgaaacgcggcatttacgatgtttgtcatgcctgcgggcaccgcgccacgatcgcggataattctcgctgccgcttccagctctgtgacgaccatggccaaaatttcgctcgggggacgcacttccagcgccatttgcgacctagccgcctccagctcctcggcgtggcgtttgttggcgcgctcgcggctggctgcggcacgacacgcatctgagcaatattttgcgcgccgtcctcgcgggtcaggccggggaggaatcaggccaccgcagtaggcgcaactgattcgatcctccactactgtgcgtcctcctggcgctgccgagcacgcagctcgtcagccagctcctcaagatccgccacgagagtttctaggtcgctcgcggcactggcccagtctcgtgatgctggcgcgtccgtcgtatcgagagctcggaaaaatccgatcaccgtttttaaatcgacggcagcatcgagcgcgtcggactccagcgcgacatcagagagatccatagctgatgattcgggccaattttggtacttcgtcgtgaaggtcatgacaccattataacgaacgttcgttaaagtttttggcggaaaatcacgcggcacgaaaattttcacgaagcgggactttgcgcagctcaggggtgctaaaaattttgtatcgcacttgatttttccgaaagacagattatctgcaaacggtgtgtcgtatttctggcttggtttttaaaaaatctggaatcgaaaatttgcggggcga

SEQ ID NO: 13 - DNA, 6250 bp, synthetic construct
  source 1..6250: mol_type = other DNA
gtagtactcagctgtaatacgactcactatagggtaccacgtagaccgtacggcagtaataaccagctgaccgcatacccgagtaatggcgtccaaggtttacgaccctgagcagcggaagcgcatgatcacgggcccacagtggtgggcccgttgcaagcagatgaacgttctcgacagcttcatcaactattacgatagtgagaagcatgcagagaacgccgtcatcttcttgcacgggaatgcagcgagcagctatctatggcggcacgttgtgccgcacatagagcctgttgctcgctgcataatcccggaccttatagggatggggaagagcggtaagagcggcaacggctcttaccgccttctcgatcactataagtacttgacagcatggttcgagctcctcaatctgcccaagaagatcatcttcgttgggcacgattggggagcttgtctcgccttccattactcttacgagcaccaggacaagatcaaggccatcgtccacgcggagagcgtggtcgatgtgatcgagtcctgggatgagtggcccgatatcgaggaggatatcgcactcatcaagagtgaggaaggcgagaagatggtcctggagaataatttcttcgtggagaccatgctgccaagtaagatcatgcgcaagctcgagccggaggagtttgcggcgtacctcgagcccttcaaggagaagggcgaggtacgccgcccgactctctcctggcctcgagagatcccgctggtcaagggtggtaagccggacgtcgtgcagatagtgcgtaactacaacgcctatctgcgggcaagtgacgacttgcccaagatgttcattgagagcgaccccggcttcttctcgaacgccattgttgagggagctaagaagttccccaacacggagttcgtgaaggtgaaggggttgcatttcagtcaggaggacgcgcccgacgaaatgggcaagtacatcaagtccttcgtcgagcgcgtcctcaagaatgagcagtaatacgtattgccatgtgtatgtgggagacggtcgggtccagatattcgtatctgtcgagtagagtgtgggctcccacatactctgatgatccttcgggatcattcatggcaactcgagatagcataaaataacgccccaccttcttaacgggaggtggggcgttatttttactgaaagatatcatccaatggatctgtcgacggccgtcgttttacagccaagcttggctgttttggcggatgagagaagattttcagcctgatacagattaaatcagaacgcagaagcggtctgataaaacagaatttgcctggcggcagtagcgcggtggtcccacctgaccccatgccgaactcagaagtgaaacgccgtagcgccgatggtagtgtggggtctccccatgcgagagtagggaactgccaggcatcaaataaaacgaaaggctcagtcgaaagactgggcctttcgttttatctgttgtttgtcggtgaacgctctcctgagtaggacaaatccgccgggagcggatttgaacgttgcgaagcaacggcccggagggtggcgggcaggacgcccgccataaactgccaggcatcaaattaagcagaaggccatcctgacggatggcctttttgcgtttctacaaactcttttggtcgactctagagttccactgagcgtcagaccccgtagaaaagatcaaaggatcttcttgagatcctttttttctgcgcgtaatctgctgcttgcaaacaaaaaaaccaccgctaccagcggtggtttgtttgccggatcaagagctaccaactctttttccgaaggtaactggcttcagcagagcgcagataccaaatactgtccttctagtgtagccgtagttaggccaccacttcaagaactctgtagcaccgcctacatacctcgctctgctaatcctgttaccagtggctgctgccagtggcgataagtcgtgtcttaccgggttggactcaagacgatagttaccggataaggcgcagcggtcgggctgaacggggggttcgtgcacacagcccagcttggagcgaacgacctacaccgaactgagatacctacagcgtgagctatgagaaagcgccacgcttcccgaagggagaaaggcggacaggtatccggtaagcggcagggtcggaacaggagagcgcacgagggagcttccagggggaaacgcctggtatctttatagtcctgtcgggtttcgccacctctgacttgagcgtcgatttttgtgatgctcgtcaggggggcggagcctatggaaaaacgccagcaacgcggcctttttacggttcctggccttttgctggccttttgctcacatgttctttcctgcgttatcccctgattctgtggataaccgtattaccgcctttgagtgagctgataccgctcgccgcagccgaacgaccgagcgcagcgagtcagtgagcgaggaagcggaagatctagaagtactgctgactcataccaggcctgaatcgccccatcatccagccagaaagtgagggagccacggttgatgagagctttgttgtaggtggaccagttggtgattttgaacttttgctttgccacggaacggtctgcgttgtcgggaagatgcgtgatctgatccttcaactcagcaaaagttcgatttattcaacaaagccacgttgtgtctcaaaatctctgatgttacattgcacaagataaaaatatatcatcatgaacaataaaactgtctgcttacataaacagtaatacaaggggtgttatgagccatattcaacgggaaacgtcttgctcaaggccgcgattaaattccaacatggatgctgatttatatgggtataaatgggctcgcgataatgtcgggcaatcaggtgcgacaatctatcgattgtatgggaagcccgatgcgccagagttgtttctgaaacatggcaaaggtagcgttgccaatgatgttacagatgagatggtcagactaaactggctgacggaatttatgcctcttccgaccatcaagcattttatccgtactcctgatgatgcatggttactcaccactgcgatccccggaaaaacagcattccaggtattagaagaatatcctgattcaggtgaaaatattgttgatgcgctggcagtgttcctgcgccggttgcattcgattcctgtttgtaattgtccttttaacagcgatcgcgtatttcgtctcgctcaggcgcaatcacgaatgaataacggtttggttgatgcgagtgattttgatgacgagcgtaatggctggcctgttgaacaagtctggaaagaaatgcataagcttttgccattctcaccggattcagtcgtcactcatggtgatttctcacttgataaccttatttttgacgaggggaaattaataggttgtattgatgttggacgagtcggaatcgcagaccgataccaggatcttgccatcctatggaactgcctcggtgagttttctccttcattacagaaacggctttttcaaaaatatggtattgataatcctgatatgaataaattgcagtttcatttgatgctcgatgagtttttctaaggctagccccgggactagtgatctttgggagcagtccttgtgcgcttacgaggtgagccggtggggaaccgttatctgcctatggtgtgagcccccctagagagcttcaagagcaatcagcccgacctagaaaggaggccaagagagagacccctacggggggaaccgttttctgcctacgagatggcacatttactgggaagctttacggcgtcctcgtggaagttcaatgcccgcagacttaagtgctctattcacggtctgacgtgacacgctaaattcagacatagcttcattgattgtcggccacgagccagtctctccctcaacagtcataaaccaacctgcaatggtcaagcgattttctttagctttcctagcttgtcgttgactggacttagctagtttttctcgctgtgctcgggcgtactcactgtttgggtctttccagcgttctgcggcctttttaccgccacgtcttcccatagtggccagagcttttcgccctcggctgctctgcgtctctgtctgacgagcagggacgactggctggcctttagcgacgtagccgcgcacacgtcgcgccatcgtctggcggtcacgcatcggcggcagatcaggctcacggccgtctgctccgaccgcctgagcgacggtgtaggcacgctcgtaggcgtcgatgatcttggtgtcttttaggcgctcaccagccgcttttaactggtatcccacagtcaaagcgtggcgaaaagccgtctcatcacgggcggcacgccctggagcagtccagaggacacggacgccgtcgatcagctctccagacgcttcagcggcgctcggcaggcttgcttcaagcgtggcaagtgcttttgcttccgcagtggcttttcttgccgcttcgatacgtgcccgtccgctagaaaactcctgctcatagcgttttttaggtttttctgtgcctgagatcatgcgagcaacctccataagatcagctaggcgatccacgcgattgtgctgggcatgccagcggtacgcggtgggatcgtcggagacgtgcagtggccaccggctcagcctatgtgaaaaagcctggtcagcgccgaaaacgcgggtcatttcctcggtcgttgcagccagcaggcgcatattcgggctgctcatgcctgctgcggcatacaccggatcaatgagccagatgagctggcatttcccgctcagtggattcacgccgatccaagctggcgctttttccaggcgtgcccagcgctccaaaatcgcgtagacctcggggtttacgtgctcgattttcccgccggcctggtggctcggcacatcaatgtccaggacaagcacggctgcgtgctgcgcgtgcgtcagagcaacatactggcaccgggcaagcgattttgaaccaactcggtataacttcggctgtgtttctcccgtgtccgggtctttgatccaagcgctggcgaagtcgcgggtcttgctgccctggaaattttctctgcccaggtgagcgaggaattcgcggcggtcttcgctcgtccagccacgtgatcgcagcgcgagctcgggatgggtgtcgaacagatcagcggaaaatttccaggccggtgtgtcaatgtctcgtgaatccgctagagtcatttttgagcgctttctcccaggtttggactgggggttagccgacgccctgtgagttaccgctcacggggcgttcaacatttttcaggtattcgtgcagcttatcgcttcttgccgcctgtgcgctttttcgacgcgcgacgctgctgccgattcggtgcaggtggtggcggcgctgacacgtcctgggcggccacggccacacgaaacgcggcatttacgatgtttgtcatgcctgcgggcaccgcgccacgatcgcggataattctcgctgccgcttccagctctgtgacgaccatggccaaaatttcgctcgggggacgcacttccagcgccatttgcgacctagccgcctccagctcctcggcgtggcgtttgttggcgcgctcgcggctggctgcggcacgacacgcatctgagcaatattttgcgcgccgtcctcgcgggtcaggccggggaggaatcaggccaccgcagtaggcgcaactgattcgatcctccactactgtgcgtcctcctggcgctgccgagcacgcagctcgtcagccagctcctcaagatccgccacgagagtttctaggtcgctcgcggcactggcccagtctcgtgatgctggcgcgtccgtcgtatcgagagctcggaaaaatccgatcaccgtttttaaatcgacggcagcatcgagcgcgtcggactccagcgcgacatcagagagatccatagctgatgattcgggccaattttggtacttcgtcgtgaaggtcatgacaccattataacgaacgttcgttaaagtttttggcggaaaatcacgcggcacgaaaattttcacgaagcgggactttgcgcagctcaggggtgctaaaaattttgtatcgcacttgatttttccgaaagacagattatctgcaaacggtgtgtcgtatttctggcttggtttttaaaaaatctggaatcgaaaatttgcggggcga

SEQ ID NO: 14 - DNA, 936 bp, synthetic construct
  source 1..936: mol_type = other DNA
atggcgagtaaagtatatgatcccgaacaaagaaaaagaatgataacagggccccaatggtgggcgagatgtaaacaaatgaatgtattagatagttttataaattattatgatagtgaaaaacatgcggaaaatgcggtaatatttttacatgggaatgcggcgagtagttatttatggagacatgtagtaccccatatagaacccgtagcgagatgtataatacccgatttaatagggatggggaaaagtgggaaaagtgggaatgggagttatagattattagatcattataaatatttaacagcgtggtttgaattattaaatttacccaaaaaaataatatttgtagggcatgattggggggcgtgtttagcgtttcattatagttatgaacatcaagataaaataaaagcgatagtacatgcggaaagtgtagtagatgtaatagaaagttgggatgaatggcccgatatagaagaagatatagcgttaataaaaagtgaagaaggggaaaaaatggtattagaaaataatttttttgtagaaacaatgttacccagtaaaataatgagaaaattagaacccgaagaatttgcggcgtatttagaaccctttaaagaaaaaggggaagtaagaagacccacattaagttggcccagagaaatacccttagtaaaaggggggaaacccgatgtagtacaaatagtaagaaattataatgcgtatttaagagcgagtgatgatttacccaaaatgtttatagaaagtgatcccgggttttttagtaatgcgatagtagaaggggcgaaaaaatttcccaatacagaatttgtaaaagtaaaagggttacattttagtcaagaagatgcgcccgatgaaatggggaaatatataaaaagttttgtagaaagagtattaaaaaatgaacaataa

SEQ ID NO: 15 - DNA, 1177 bp, synthetic construct
  source 1..1177: mol_type = other DNA
taatacgactcactatagggtaccacgtagaccgtacggcagtaataaccagctgaccgcatacccgagtaatggcgagtaaagtatatgatcccgaacaaagaaaaagaatgataacagggccccaatggtgggcgagatgtaaacaaatgaatgtattagatagttttataaattattatgatagtgaaaaacatgcggaaaatgcggtaatatttttacatgggaatgcggcgagtagttatttatggagacatgtagtaccccatatagaacccgtagcgagatgtataatacccgatttaatagggatggggaaaagtgggaaaagtgggaatgggagttatagattattagatcattataaatatttaacagcgtggtttgaattattaaatttacccaaaaaaataatatttgtagggcatgattggggggcgtgtttagcgtttcattatagttatgaacatcaagataaaataaaagcgatagtacatgcggaaagtgtagtagatgtaatagaaagttgggatgaatggcccgatatagaagaagatatagcgttaataaaaagtgaagaaggggaaaaaatggtattagaaaataatttttttgtagaaacaatgttacccagtaaaataatgagaaaattagaacccgaagaatttgcggcgtatttagaaccctttaaagaaaaaggggaagtaagaagacccacattaagttggcccagagaaatacccttagtaaaaggggggaaacccgatgtagtacaaatagtaagaaattataatgcgtatttaagagcgagtgatgatttacccaaaatgtttatagaaagtgatcccgggttttttagtaatgcgatagtagaaggggcgaaaaaatttcccaatacagaatttgtaaaagtaaaagggttacattttagtcaagaagatgcgcccgatgaaatggggaaatatataaaaagttttgtagaaagagtattaaaaaatgaacaataatacgtattgccatgtgtatgtgggagacggtcgggtccagatattcgtatctgtcgagtagagtgtgggctcccacatactctgatgatccttcgggatcattcatggcaactcgagatagcataaaataacgccccaccttcttaacgggaggtggggcgttattttta

SEQ ID NO: 16 - DNA, 6243 bp, synthetic construct
  source 1..6243: mol_type = other DNA
gatcctagtactcagctgtaatacgactcactatagggtaccacgtagaccgtacggcagtaataaccagctgaccgcatacccgagtaatggcgagtaaagtatatgatcccgaacaaagaaaaagaatgataacagggccccaatggtgggcgagatgtaaacaaatgaatgtattagatagttttataaattattatgatagtgaaaaacatgcggaaaatgcggtaatatttttacatgggaatgcggcgagtagttatttatggagacatgtagtaccccatatagaacccgtagcgagatgtataatacccgatttaatagggatggggaaaagtgggaaaagtgggaatgggagttatagattattagatcattataaatatttaacagcgtggtttgaattattaaatttacccaaaaaaataatatttgtagggcatgattggggggcgtgtttagcgtttcattatagttatgaacatcaagataaaataaaagcgatagtacatgcggaaagtgtagtagatgtaatagaaagttgggatgaatggcccgatatagaagaagatatagcgttaataaaaagtgaagaaggggaaaaaatggtattagaaaataatttttttgtagaaacaatgttacccagtaaaataatgagaaaattagaacccgaagaatttgcggcgtatttagaaccctttaaagaaaaaggggaagtaagaagacccacattaagttggcccagagaaatacccttagtaaaaggggggaaacccgatgtagtacaaatagtaagaaattataatgcgtatttaagagcgagtgatgatttacccaaaatgtttatagaaagtgatcccgggttttttagtaatgcgatagtagaaggggcgaaaaaatttcccaatacagaatttgtaaaagtaaaagggttacattttagtcaagaagatgcgcccgatgaaatggggaaatatataaaaagttttgtagaaagagtattaaaaaatgaacaataatacgtattgccatgtgtatgtgggagacggtcgggtccagatattcgtatctgtcgagtagagtgtgggctcccacatactctgatgatccttcgggatcattcatggcaactcgagatagcataaaataacgccccaccttcttaacgggaggtggggcgttatttttactgaaagatatctgtcgacggccgtcgttttacagccaagcttggctgttttggcggatgagagaagattttcagcctgatacagattaaatcagaacgcagaagcggtctgataaaacagaatttgcctggcggcagtagcgcggtggtcccacctgaccccatgccgaactcagaagtgaaacgccgtagcgccgatggtagtgtggggtctccccatgcgagagtagggaactgccaggcatcaaataaaacgaaaggctcagtcgaaagactgggcctttcgttttatctgttgtttgtcggtgaacgctctcctgagtaggacaaatccgccgggagcggatttgaacgttgcgaagcaacggcccggagggtggcgggcaggacgcccgccataaactgccaggcatcaaattaagcagaaggccatcctgacggatggcctttttgcgtttctacaaactcttttggtcgactctagagttccactgagcgtcagaccccgtagaaaagatcaaaggatcttcttgagatcctttttttctgcgcgtaatctgctgcttgcaaacaaaaaaaccaccgctaccagcggtggtttgtttgccggatcaagagctaccaactctttttccgaaggtaactggcttcagcagagcgcagataccaaatactgtccttctagtgtagccgtagttaggccaccacttcaagaactctgtagcaccgcctacatacctcgctctgctaatcctgttaccagtggctgctgccagtggcgataagtcgtgtcttaccgggttggactcaagacgatagttaccggataaggcgcagcggtcgggctgaacggggggttcgtgcacacagcccagcttggagcgaacgacctacaccgaactgagatacctacagcgtgagctatgagaaagcgccacgcttcccgaagggagaaaggcggacaggtatccggtaagcggcagggtcggaacaggagagcgcacgagggagcttccagggggaaacgcctggtatctttatagtcctgtcgggtttcgccacctctgacttgagcgtcgatttttgtgatgctcgtcaggggggcggagcctatggaaaaacgccagcaacgcggcctttttacggttcctggccttttgctggccttttgctcacatgttctttcctgcgttatcccctgattctgtggataaccgtattaccgcctttgagtgagctgataccgctcgccgcagccgaacgaccgagcgcagcgagtcagtgagcgaggaagcggaagatctagaagtactgctgactcataccaggcctgaatcgccccatcatccagccagaaagtgagggagccacggttgatgagagctttgttgtaggtggaccagttggtgattttgaacttttgctttgccacggaacggtctgcgttgtcgggaagatgcgtgatctgatccttcaactcagcaaaagttcgatttattcaacaaagccacgttgtgtctcaaaatctctgatgttacattgcacaagataaaaatatatcatcatgaacaataaaactgtctgcttacataaacagtaatacaaggggtgttatgagccatattcaacgggaaacgtcttgctcaaggccgcgattaaattccaacatggatgctgatttatatgggtataaatgggctcgcgataatgtcgggcaatcaggtgcgacaatctatcgattgtatgggaagcccgatgcgccagagttgtttctgaaacatggcaaaggtagcgttgccaatgatgttacagatgagatggtcagactaaactggctgacggaatttatgcctcttccgaccatcaagcattttatccgtactcctgatgatgcatggttactcaccactgcgatccccggaaaaacagcattccaggtattagaagaatatcctgattcaggtgaaaatattgttgatgcgctggcagtgttcctgcgccggttgcattcgattcctgtttgtaattgtccttttaacagcgatcgcgtatttcgtctcgctcaggcgcaatcacgaatgaataacggtttggttgatgcgagtgattttgatgacgagcgtaatggctggcctgttgaacaagtctggaaagaaatgcataagcttttgccattctcaccggattcagtcgtcactcatggtgatttctcacttgataaccttatttttgacgaggggaaattaataggttgtattgatgttggacgagtcggaatcgcagaccgataccaggatcttgccatcctatggaactgcctcggtgagttttctccttcattacagaaacggctttttcaaaaatatggtattgataatcctgatatgaataaattgcagtttcatttgatgctcgatgagtttttctaaggctagccccgggactagtgatctttgggagcagtccttgtgcgcttacgaggtgagccggtggggaaccgttatctgcctatggtgtgagcccccctagagagcttcaagagcaatcagcccgacctagaaaggaggccaagagagagacccctacggggggaaccgttttctgcctacgagatggcacatttactgggaagctttacggcgtcctcgtggaagttcaatgcccgcagacttaagtgctctattcacggtctgacgtgacacgctaaattcagacatagcttcattgattgtcggccacgagccagtctctccctcaacagtcataaaccaacctgcaatggtcaagcgattttctttagctttcctagcttgtcgttgactggacttagctagtttttctcgctgtgctcgggcgtactcactgtttgggtctttccagcgttctgcggcctttttaccgccacgtcttcccatagtggccagagcttttcgccctcggctgctctgcgtctctgtctgacgagcagggacgactggctggcctttagcgacgtagccgcgcacacgtcgcgccatcgtctggcggtcacgcatcggcggcagatcaggctcacggccgtctgctccgaccgcctgagcgacggtgtaggcacgctcgtaggcgtcgatgatcttggtgtcttttaggcgctcaccagccgcttttaactggtatcccacagtcaaagcgtggcgaaaagccgtctcatcacgggcggcacgccctggagcagtccagaggacacggacgccgtcgatcagctctccagacgcttcagcggcgctcggcaggcttgcttcaagcgtggcaagtgcttttgcttccgcagtggcttttcttgccgcttcgatacgtgcccgtccgctagaaaactcctgctcatagcgttttttaggtttttctgtgcctgagatcatgcgagcaacctccataagatcagctaggcgatccacgcgattgtgctgggcatgccagcggtacgcggtgggatcgtcggagacgtgcagtggccaccggctcagcctatgtgaaaaagcctggtcagcgccgaaaacgcgggtcatttcctcggtcgttgcagccagcaggcgcatattcgggctgctcatgcctgctgcggcatacaccggatcaatgagccagatgagctggcatttcccgctcagtggattcacgccgatccaagctggcgctttttccaggcgtgcccagcgctccaaaatcgcgtagacctcggggtttacgtgctcgattttcccgccggcctggtggctcggcacatcaatgtccaggacaagcacggctgcgtgctgcgcgtgcgtcagagcaacatactggcaccgggcaagcgattttgaaccaactcggtataacttcggctgtgtttctcccgtgtccgggtctttgatccaagcgctggcgaagtcgcgggtcttgctgccctggaaattttctctgcccaggtgagcgaggaattcgcggcggtcttcgctcgtccagccacgtgatcgcagcgcgagctcgggatgggtgtcgaacagatcagcggaaaatttccaggccggtgtgtcaatgtctcgtgaatccgctagagtcatttttgagcgctttctcccaggtttggactgggggttagccgacgccctgtgagttaccgctcacggggcgttcaacatttttcaggtattcgtgcagcttatcgcttcttgccgcctgtgcgctttttcgacgcgcgacgctgctgccgattcggtgcaggtggtggcggcgctgacacgtcctgggcggccacggccacacgaaacgcggcatttacgatgtttgtcatgcctgcgggcaccgcgccacgatcgcggataattctcgctgccgcttccagctctgtgacgaccatggccaaaatttcgctcgggggacgcacttccagcgccatttgcgacctagccgcctccagctcctcggcgtggcgtttgttggcgcgctcgcggctggctgcggcacgacacgcatctgagcaatattttgcgcgccgtcctcgcgggtcaggccggggaggaatcaggccaccgcagtaggcgcaactgattcgatcctccactactgtgcgtcctcctggcgctgccgagcacgcagctcgtcagccagctcctcaagatccgccacgagagtttctaggtcgctcgcggcactggcccagtctcgtgatgctggcgcgtccgtcgtatcgagagctcggaaaaatccgatcaccgtttttaaatcgacggcagcatcgagcgcgtcggactccagcgcgacatcagagagatccatagctgatgattcgggccaattttggtacttcgtcgtgaaggtcatgacaccattataacgaacgttcgttaaagtttttggcggaaaatcacgcggcacgaaaattttcacgaagcgggactttgcgcagctcaggggtgctaaaaattttgtatcgcacttgatttttccgaaagacagattatctgcaaacggtgtgtcgtatttctggcttggtttttaaaaaatctggaatcgaaaatttgcggggcgag

SEQ ID NO: 17 - DNA, 1653 bp, synthetic construct
  source 1..1653: mol_type = other DNA
atggaagatgccaaaaacattaagaagggcccagcgccattctacccactcgaagacgggaccgccggcgagcagctgcacaaagccatgaagcgctacgccctggtgcccggcaccatcgcctttaccgacgcacatatcgaggtggacattacctacgccgagtacttcgagatgagcgttcggctggcagaagctatgaagcgctatgggctgaatacaaaccatcggatcgtggtgtgcagcgagaatagcttgcagttcttcatgcccgtgttgggtgccctgttcatcggtgtggctgtggccccagctaacgacatctacaacgagcgcgagctgctgaacagcatgggcatcagccagcccaccgtcgtattcgtgagcaagaaagggctgcaaaagatcctcaacgtgcaaaagaagctaccgatcatacaaaagatcatcatcatggatagcaagaccgactaccagggcttccaaagcatgtacaccttcgtgacttcccatttgccacccggcttcaacgagtacgacttcgtgcccgagagcttcgaccgggacaaaaccatcgccctgatcatgaacagtagtggcagtaccggattgcccaagggcgtagccctaccgcaccgcaccgcttgtgtccgattcagtcatgcccgcgaccccatcttcggcaaccagatcatccccgacaccgctatcctcagcgtggtgccatttcaccacggcttcggcatgttcaccacgctgggctacttgatctgcggctttcgggtcgtgctcatgtaccgcttcgaggaggagctattcttgcgcagcttgcaagactataagattcaatctgccctgctggtgcccacactatttagcttcttcgctaagagcactctcatcgacaagtacgacctaagcaacttgcacgagatcgccagcggcggggcgccgctcagcaaggaggtaggtgaggccgtggccaaacgcttccacctaccaggcatccgccagggctacggcctgacagaaacaaccagcgccattctgatcacccccgaaggggacgacaagcctggcgcagtaggcaaggtggtgcccttcttcgaggctaaggtggtggacttggacaccggtaagacactgggtgtgaaccagcgcggcgagctgtgcgtccgtggccccatgatcatgagcggctacgttaacaaccccgaggctacaaacgctctcatcgacaaggacggctggctgcacagcggcgacatcgcctactgggacgaggacgagcacttcttcatcgtggaccggctgaagagcctgatcaaatacaagggctaccaggtagccccagccgaactggagagcatcctgctgcaacaccccaacatcttcgacgccggggtcgccggcctgcccgacgacgatgccggcgagctgcccgccgcagtcgtcgtgctggaacacggtaaaaccatgaccgagaaggagatcgtggactatgtggccagccaggttacaaccgccaagaagctgcgcggtggtgttgtgttcgtggacgaggtgcctaaaggactgaccggcaagttggacgcccgcaagatccgcgagattctcattaaggccaagaagggcggcaagatcgccgtgtaa

SEQ ID NO: 18 - DNA, 1653 bp, synthetic construct
  source 1..1653: mol_type = other DNA
atggaggacgcaaagaatattaagaagggccctgcgcccttctatcctttggaggacggtactgccggggagcagctgcataaggctatgaagcgttatgcgctggtccccggcactatcgccttcacggacgctcatatcgaagtagacatcacatatgctgagtacttcgaaatgagcgtccgtctcgctgaggccatgaagcggtatggtttgaacacaaaccaccgcatcgtggtctgcagcgagaattctttgcagttcttcatgcctgttctgggagccctgtttatcggtgttgctgtcgcacctgctaatgatatttataatgaacgggagcttcttaatagcatggggatctcgcagcccactgttgttttcgtgagcaagaaggggctgcagaagatcctcaatgtgcagaagaagctcccgatcattcagaaaatcattatcatggacagcaagaccgattatcagggcttccagagcatgtatacttttgtcacatcgcacttgccccccggctttaatgagtatgattttgtcccggagagttttgatcgggacaagactattgccctgatcatgaactcttcgggatccacgggtcttcctaagggcgtcgcgcttccccaccgaaccgcgtgtgtgagatttagccacgctcgggatcccatattcgggaatcaaattatcccggatacggcgatcctgagcgtggttccgtttcaccacgggttcggtatgttcacgacccttgggtacctcatctgcggattccgcgtagtcctgatgtatcgctttgaggaggaactgtttctccgcagcctccaagactacaagattcagtcggcgctcctagtcccgacgctattctcgttctttgccaagtcgaccttgattgacaagtacgacttgagcaatttgcacgagatagcgtcgggaggagcgccgctgagtaaggaagtcggggaggctgtggcgaaacggttccacctcccagggatacgtcagggctacggcctgactgagacgacgtccgcgatccttatcaccccggagggggatgataagccgggtgctgtcggcaaggtggttccgttcttcgaggccaaagtggtagaccttgatactggtaagactcttggggtgaatcaacgaggagaattgtgcgtccgtggtcccatgattatgtcaggctatgtcaataaccccgaggcaaccaacgccttgattgacaaggacggttggttgcactcgggggacatagcctactgggacgaggacgagcatttcttcatcgttgatcgcctcaagagtcttatcaagtacaagggctaccaggtggccccggcagaactggaatccatcttgctgcagcacccgaatatcttcgacgctggtgttgccgggctcccggacgacgacgccggggaacttcccgcggccgtcgtcgtcctggagcacggcaagaccatgacggagaaggagatcgtggactacgtcgccagtcaggtcaccaccgcgaagaaacttcgcggtggtgtggtgttcgtagatgaggtacccaagggtctgacggggaagctcgacgcccggaagatccgtgaaatactcattaaagccaaaaaggggggcaagattgcggtgtga

SEQ ID NO: 19 - DNA, 3822 bp, synthetic construct
  source 1..3822: mol_type = other DNA
atgtttgtttttcttgttttattgccactagtctctagtcagtgtgttaatcttacaaccagaactcaattaccccctgcatacactaattctttcacacgtggtgtttattaccctgacaaagttttcagatcctcagttttacattcaactcaggacttgttcttacctttcttttccaatgttacttggttccatgctatacatgtctctgggaccaatggtactaagaggtttgataaccctgtcctaccatttaatgatggtgtttattttgcttccactgagaagtctaacataataagaggctggatttttggtactactttagattcgaagacccagtccctacttattgttaataacgctactaatgttgttattaaagtctgtgaatttcaattttgtaatgatccatttttgggtgtttattaccacaaaaacaacaaaagttggatggaaagtgagttcagagtttattctagtgcgaataattgcacttttgaatatgtctctcagccttttcttatggaccttgaaggaaaacagggtaatttcaaaaatcttagggaatttgtgtttaagaatattgatggttattttaaaatatattctaagcacacgcctattaatttagtgcgtgatctccctcagggtttttcggctttagaaccattggtagatttgccaataggtattaacatcactaggtttcaaactttacttgctttacatagaagttatttgactcctggtgattcttcttcaggttggacagctggtgctgcagcttattatgtgggttatcttcaacctaggacttttctattaaaatataatgaaaatggaaccattacagatgctgtagactgtgcacttgaccctctctcagaaacaaagtgtacgttgaaatccttcactgtagaaaaaggaatctatcaaacttctaactttagagtccaaccaacagaatctattgttagatttcctaatattacaaacttgtgcccttttggtgaagtttttaacgccaccagatttgcatctgtttatgcttggaacaggaagagaatcagcaactgtgttgctgattattctgtcctatataattccgcatcattttccacttttaagtgttatggagtgtctcctactaaattaaatgatctctgctttactaatgtctatgcagattcatttgtaattagaggtgatgaagtcagacaaatcgctccagggcaaactggaaagattgctgattataattataaattaccagatgattttacaggctgcgttatagcttggaattctaacaatcttgattctaaggttggtggtaattataattacctgtatagattgtttaggaagtctaatctcaaaccttttgagagagatatttcaactgaaatctatcaggccggtagcacaccttgtaatggtgttgaaggttttaattgttactttcctttacaatcatatggtttccaacccactaatggtgttggttaccaaccatacagagtagtagtactttcttttgaacttctacatgcaccagcaactgtttgtggacctaaaaagtctactaatttggttaaaaacaaatgtgtcaatttcaacttcaatggtttaacaggcacaggtgttcttactgagtctaacaaaaagtttctgcctttccaacaatttggcagagacattgctgacactactgatgctgtccgtgatccacagacacttgagattcttgacattacaccatgttcttttggtggtgtcagtgttataacaccaggaacaaatacttctaaccaggttgctgttctttatcaggatgttaactgcacagaagtccctgttgctattcatgcagatcaacttactcctacttggcgtgtttattctacaggttctaatgtttttcaaacacgtgcaggctgtttaataggggctgaacatgtcaacaactcatatgagtgtgacatacccattggtgcaggtatatgcgctagttatcagactcagactaattctcctcggcgggcacgtagtgtagctagtcaatccatcattgcctacactatgtcacttggtgcagaaaattcagttgcttactctaataactctattgccatacccacaaattttactattagtgttaccacagaaattctaccagtgtctatgaccaagacatcagtagattgtacaatgtacatttgtggtgattcaactgaatgcagcaatcttttgttgcaatatggcagtttttgtacacaattaaaccgtgctttaactggaatagctgttgaacaagacaaaaacacccaagaagtttttgcacaagtcaaacaaatttacaaaacaccaccaattaaagattttggtggttttaatttttcacaaatattaccagatccatcaaaaccaagcaagaggtcatttattgaagatctacttttcaacaaagtgacacttgcagatgctggcttcatcaaacaatatggtgattgccttggtgatattgctgctagagacctcatttgtgcacaaaagtttaacggccttactgttttgccacctttgctcacagatgaaatgattgctcaatacacttctgcactgttagcgggtacaatcacttctggttggacctttggtgcaggtgctgcattacaaataccatttgctatgcaaatggcttataggtttaatggtattggagttacacagaatgttctctatgagaaccaaaaattgattgccaaccaatttaatagtgctattggcaaaattcaagactcactttcttccacagcaagtgcacttggaaaacttcaagatgtggtcaaccaaaatgcacaagctttaaacacgcttgttaaacaacttagctccaattttggtgcaatttcaagtgttttaaatgatatcctttcacgtcttgacaaagttgaggctgaagtgcaaattgataggttgatcacaggcagacttcaaagtttgcagacatatgtgactcaacaattaattagagctgcagaaatcagagcttctgctaatcttgctgctactaaaatgtcagagtgtgtacttggacaatcaaaaagagttgatttttgtggaaagggctatcatcttatgtccttccctcagtcagcacctcatggtgtagtcttcttgcatgtgacttatgtccctgcacaagaaaagaacttcacaactgctcctgccatttgtcatgatggaaaagcacactttcctcgtgaaggtgtctttgtttcaaatggcacacactggtttgtaacacaaaggaatttttatgaaccacaaatcattactacagacaacacatttgtgtctggtaactgtgatgttgtaataggaattgtcaacaacacagtttatgatcctttgcaacctgaattagactcattcaaggaggagttagataaatattttaagaatcatacatcaccagatgttgatttaggtgacatctctggcattaatgcttcagttgtaaacattcaaaaagaaattgaccgcctcaatgaggttgccaagaatttaaatgaatctctcatcgatctccaagaacttggaaagtatgagcagtatataaaatggccatggtacatttggctaggttttatagctggcttgattgccatagtaatggtgacaattatgctttgctgtatgaccagttgctgtagttgtctcaagggctgttgttcttgtggatcctgctgcaaatttgatgaagacgactctgagccagtgctcaaaggagtcaaattacattacacataa

SEQ ID NO: 20 - DNA, 3822 bp, synthetic construct
  source 1..3822: mol_type = other DNA
atgtttgtgtttcttgtcctccttccactggtttcgagtcagtgcgtcaatcttacaacacgaacccagctgccgccagcctacacgaactccttcacgcggggagtgtactaccccgacaaggtgttccgctcgtctgttctgcacagcacgcaggacctcttcctcccgttcttctcgaacgtgacgtggttccatgccattcacgtttcgggaacgaacgggacgaagaggttcgataaccctgttctaccgtttaacgacggggtgtacttcgcttcgacagagaagtccaacattattcgcggatggatattcggaaccactctcgattccaagactcagtccttgttgatagtgaacaacgccacgaacgtggtcattaaggtctgtgagtttcagttctgtaatgacccgttcttgggtgtttactatcacaagaacaacaagtcttggatggagagtgagttccgagtgtattcatccgcgaataattgtaccttcgagtatgtcagtcagccgtttctgatggatcttgaaggcaaacagggcaatttcaagaatttgcgcgagtttgtcttcaagaacatcgacggctacttcaagatatactcgaagcacacgccaatcaacctcgtccgtgatctcccgcagggcttcagcgctctggaaccgctggtggacttgccgataggcatcaacatcacgcggttccagacgctgttagccctgcacaggagttacctgaccccaggtgactcctcgtccggttggactgcaggtgccgccgcgtactacgtggggtacctgcagccccggacgttcttgttgaagtacaacgagaacgggacgatcacggacgcggttgattgtgcgttggaccctctgtcggagacgaagtgcaccctgaagtcgtttacggtagaaaaggggatctatcagacctccaacttccgcgtccagccgactgagagtatcgttcggtttccgaacatcacgaacctgtgtccgtttggagaggtcttcaacgcgaccaggttcgcctccgtgtacgcttggaacaggaagaggatatcgaattgtgtagcagactacagtgtgctatacaattcggcgtccttttccactttcaagtgttacggagtgtcgcccacgaagttgaacgacctctgcttcaccaacgtgtacgcggattccttcgtcatccgtggtgacgaggttcggcagatcgcgcccggacagactggaaagatagcggactacaattataagttgcccgacgactttactggctgcgttattgcttggaatagcaataacttagacagtaaagtcgggggcaactataattacctgtatcgactgtttcggaaaagcaatctgaagcccttcgagcgcgacattagcacggagatctaccaggctggtagtactccgtgcaatggcgtggagggcttcaattgctattttccgttacagtcgtacgggtttcagcccaccaacggggtagggtaccagccctaccgcgtggtggtgctgtcgttcgaactccttcacgcacccgcgactgtctgtgggcccaagaagtcgacgaacttggtgaagaacaagtgcgtcaacttcaacttcaatgggctcacaggcacgggggtgctgacggagtcgaacaaaaagttcctacctttccagcagttcgggcgcgatattgccgacaccacggatgccgtaagggatccgcagacgcttgagattctggacatcacgccctgcagcttcgggggcgtcagtgtaatcacgcctggtaccaacacgagcaaccaggttgccgtgttgtaccaggacgtgaattgcactgaggtccccgtagcgatccacgcggatcagctaaccccaacgtggagggtgtactcgacagggagtaatgtcttccagactcgcgctggttgtctgattggcgctgagcatgtgaacaactcgtacgagtgtgacatccccattggagcggggatctgcgcgtcgtaccagacccagacgaacagcccgaggcgtgcccgctcagtagcgtcgcagtcgatcatcgcgtacacgatgagcttgggggcggagaacagtgtagcctattcgaacaacagcattgctatccccacaaattttacaattagtgtaaccaccgagatcttaccggtctccatgaccaagacctcggtggattgcactatgtatatttgtggggatagcactgagtgttctaacctcctgctccagtacggcagtttctgtacgcagctcaaccgagcgcttacaggaattgccgtggagcaggacaagaacactcaggaggtgtttgcccaggtcaagcagatctacaagacacctccgatcaaggactttggcggcttcaacttctcccagatactccccgaccccagcaagcccagcaagcgtagctttattgaagatctgctcttcaataaagttacgcttgctgatgctgggttcatcaagcagtacggggattgtctgggagatatagccgccagagacttgatctgtgctcagaagttcaatgggctcactgttctcccccccttgctcacggacgagatgatcgcccagtatacttcggcgctgctggcgggcacgatcacctcgggctggacgtttggggctggtgcggcgctgcagatccccttcgccatgcagatggcgtaccgcttcaatgggatcggtgtcacacagaacgttttgtacgagaatcagaagctcatcgccaatcagttcaacagcgcgatcgggaagatacaggactccctgtcgagtacagcctccgcgttggggaagctgcaggacgtggtgaaccagaatgctcaagcgttgaacacgttggtgaagcagttgtcgtccaacttcggggcgataagttcggtgctgaacgatattctcagtcggctggacaaggtggaagcggaggtccagatagatcggctcatcactggtcgcctccagagtttgcagacgtacgtaactcagcagctcatccgagctgctgagatacgtgcgtctgcaaacctggcggcgaccaagatgagcgagtgcgtgctggggcagagcaagcgagtggacttctgcgggaagggctatcacctgatgtccttcccgcagagcgcacctcacggggtagtctttctccacgtgacatatgtgccggcgcaggagaagaacttcaccactgcgccggccatatgtcacgatgggaaagcccacttcccgcgtgaaggagtttttgtatcaaacgggacgcattggttcgtcacgcagcgcaacttctatgagccacagataattaccactgacaatacctttgtcagtggtaattgtgatgtggtcatagggatcgtgaacaacacggtctacgatcccctgcagcccgagctagatagtttcaaggaggagcttgataagtacttcaagaatcatacttccccagacgtggatcttggcgacattagcggcatcaacgctagtgtcgtcaacatccagaaggagatcgacaggctcaatgaggttgccaagaacctcaacgagagcctgatcgatctccaggagctggggaagtatgagcagtacatcaagtggccttggtacatctggctcgggttcattgcagggttgatcgcgatcgtgatggtcacgatcatgttgtgctgcatgacgagctgttgctcctgtttgaagggctgctgcagctgtggttcgtgttgtaagtttgacgaggatgactcggagccagtgttgaagggggtcaagttacactacacataa

SEQ ID NO: 21 - DNA, 1909 bp, synthetic construct
  source 1..1909: mol_type = other DNA
taatacgactcactatagggagacccaagctggctagcgtttaaacttaagcttggcaatccggtactgttggtaaagccaccatggaagatgccaaaaacattaagaagggcccagcgccattctacccactcgaagacgggaccgccggcgagcagctgcacaaagccatgaagcgctacgccctggtgcccggcaccatcgcctttaccgacgcacatatcgaggtggacattacctacgccgagtacttcgagatgagcgttcggctggcagaagctatgaagcgctatgggctgaatacaaaccatcggatcgtggtgtgcagcgagaatagcttgcagttcttcatgcccgtgttgggtgccctgttcatcggtgtggctgtggccccagctaacgacatctacaacgagcgcgagctgctgaacagcatgggcatcagccagcccaccgtcgtattcgtgagcaagaaagggctgcaaaagatcctcaacgtgcaaaagaagctaccgatcatacaaaagatcatcatcatggatagcaagaccgactaccagggcttccaaagcatgtacaccttcgtgacttcccatttgccacccggcttcaacgagtacgacttcgtgcccgagagcttcgaccgggacaaaaccatcgccctgatcatgaacagtagtggcagtaccggattgcccaagggcgtagccctaccgcaccgcaccgcttgtgtccgattcagtcatgcccgcgaccccatcttcggcaaccagatcatccccgacaccgctatcctcagcgtggtgccatttcaccacggcttcggcatgttcaccacgctgggctacttgatctgcggctttcgggtcgtgctcatgtaccgcttcgaggaggagctattcttgcgcagcttgcaagactataagattcaatctgccctgctggtgcccacactatttagcttcttcgctaagagcactctcatcgacaagtacgacctaagcaacttgcacgagatcgccagcggcggggcgccgctcagcaaggaggtaggtgaggccgtggccaaacgcttccacctaccaggcatccgccagggctacggcctgacagaaacaaccagcgccattctgatcacccccgaaggggacgacaagcctggcgcagtaggcaaggtggtgcccttcttcgaggctaaggtggtggacttggacaccggtaagacactgggtgtgaaccagcgcggcgagctgtgcgtccgtggccccatgatcatgagcggctacgttaacaaccccgaggctacaaacgctctcatcgacaaggacggctggctgcacagcggcgacatcgcctactgggacgaggacgagcacttcttcatcgtggaccggctgaagagcctgatcaaatacaagggctaccaggtagccccagccgaactggagagcatcctgctgcaacaccccaacatcttcgacgccggggtcgccggcctgcccgacgacgatgccggcgagctgcccgccgcagtcgtcgtgctggaacacggtaaaaccatgaccgagaaggagatcgtggactatgtggccagccaggttacaaccgccaagaagctgcgcggtggtgttgtgttcgtggacgaggtgcctaaaggactgaccggcaagttggacgcccgcaagatccgcgagattctcattaaggccaagaagggcggcaagatcgccgtgtaataatacgtattgccatgtgtatgtgggagacggtcgggtccagatattcgtatctgtcgagtagagtgtgggctcccacatactctgatgatccttcgggatcattcatggcaactcgagatagcataaaataacgccccaccttcttaacgggaggtggggcgttattttta

SEQ ID NO: 22 - DNA, 1909 bp, synthetic construct
  source 1..1909: mol_type = other DNA
taatacgactcactatagggagacccaagctggctagcgtttaaacttaagcttggcaatccggtactgttggtaaagccaccatggaggacgcaaagaatattaagaagggccctgcgcccttctatcctttggaggacggtactgccggggagcagctgcataaggctatgaagcgttatgcgctggtccccggcactatcgccttcacggacgctcatatcgaagtagacatcacatatgctgagtacttcgaaatgagcgtccgtctcgctgaggccatgaagcggtatggtttgaacacaaaccaccgcatcgtggtctgcagcgagaattctttgcagttcttcatgcctgttctgggagccctgtttatcggtgttgctgtcgcacctgctaatgatatttataatgaacgggagcttcttaatagcatggggatctcgcagcccactgttgttttcgtgagcaagaaggggctgcagaagatcctcaatgtgcagaagaagctcccgatcattcagaaaatcattatcatggacagcaagaccgattatcagggcttccagagcatgtatacttttgtcacatcgcacttgccccccggctttaatgagtatgattttgtcccggagagttttgatcgggacaagactattgccctgatcatgaactcttcgggatccacgggtcttcctaagggcgtcgcgcttccccaccgaaccgcgtgtgtgagatttagccacgctcgggatcccatattcgggaatcaaattatcccggatacggcgatcctgagcgtggttccgtttcaccacgggttcggtatgttcacgacccttgggtacctcatctgcggattccgcgtagtcctgatgtatcgctttgaggaggaactgtttctccgcagcctccaagactacaagattcagtcggcgctcctagtcccgacgctattctcgttctttgccaagtcgaccttgattgacaagtacgacttgagcaatttgcacgagatagcgtcgggaggagcgccgctgagtaaggaagtcggggaggctgtggcgaaacggttccacctcccagggatacgtcagggctacggcctgactgagacgacgtccgcgatccttatcaccccggagggggatgataagccgggtgctgtcggcaaggtggttccgttcttcgaggccaaagtggtagaccttgatactggtaagactcttggggtgaatcaacgaggagaattgtgcgtccgtggtcccatgattatgtcaggctatgtcaataaccccgaggcaaccaacgccttgattgacaaggacggttggttgcactcgggggacatagcctactgggacgaggacgagcatttcttcatcgttgatcgcctcaagagtcttatcaagtacaagggctaccaggtggccccggcagaactggaatccatcttgctgcagcacccgaatatcttcgacgctggtgttgccgggctcccggacgacgacgccggggaacttcccgcggccgtcgtcgtcctggagcacggcaagaccatgacggagaaggagatcgtggactacgtcgccagtcaggtcaccaccgcgaagaaacttcgcggtggtgtggtgttcgtagatgaggtacccaagggtctgacggggaagctcgacgcccggaagatccgtgaaatactcattaaagccaaaaaggggggcaagattgcggtgtgataatacgtattgccatgtgtatgtgggagacggtcgggtccagatattcgtatctgtcgagtagagtgtgggctcccacatactctgatgatccttcgggatcattcatggcaactcgagatagcataaaataacgccccaccttcttaacgggaggtggggcgttattttta

SEQ ID NO: 23 - DNA, 4063 bp, synthetic construct
  source 1..4063: mol_type = other DNA
taatacgactcactatagggtaccacgtagaccgtacggcagtaataaccagctgaccgcatacccgagtaatgtttgtttttcttgttttattgccactagtctctagtcagtgtgttaatcttacaaccagaactcaattaccccctgcatacactaattctttcacacgtggtgtttattaccctgacaaagttttcagatcctcagttttacattcaactcaggacttgttcttacctttcttttccaatgttacttggttccatgctatacatgtctctgggaccaatggtactaagaggtttgataaccctgtcctaccatttaatgatggtgtttattttgcttccactgagaagtctaacataataagaggctggatttttggtactactttagattcgaagacccagtccctacttattgttaataacgctactaatgttgttattaaagtctgtgaatttcaattttgtaatgatccatttttgggtgtttattaccacaaaaacaacaaaagttggatggaaagtgagttcagagtttattctagtgcgaataattgcacttttgaatatgtctctcagccttttcttatggaccttgaaggaaaacagggtaatttcaaaaatcttagggaatttgtgtttaagaatattgatggttattttaaaatatattctaagcacacgcctattaatttagtgcgtgatctccctcagggtttttcggctttagaaccattggtagatttgccaataggtattaacatcactaggtttcaaactttacttgctttacatagaagttatttgactcctggtgattcttcttcaggttggacagctggtgctgcagcttattatgtgggttatcttcaacctaggacttttctattaaaatataatgaaaatggaaccattacagatgctgtagactgtgcacttgaccctctctcagaaacaaagtgtacgttgaaatccttcactgtagaaaaaggaatctatcaaacttctaactttagagtccaaccaacagaatctattgttagatttcctaatattacaaacttgtgcccttttggtgaagtttttaacgccaccagatttgcatctgtttatgcttggaacaggaagagaatcagcaactgtgttgctgattattctgtcctatataattccgcatcattttccacttttaagtgttatggagtgtctcctactaaattaaatgatctctgctttactaatgtctatgcagattcatttgtaattagaggtgatgaagtcagacaaatcgctccagggcaaactggaaagattgctgattataattataaattaccagatgattttacaggctgcgttatagcttggaattctaacaatcttgattctaaggttggtggtaattataattacctgtatagattgtttaggaagtctaatctcaaaccttttgagagagatatttcaactgaaatctatcaggccggtagcacaccttgtaatggtgttgaaggttttaattgttactttcctttacaatcatatggtttccaacccactaatggtgttggttaccaaccatacagagtagtagtactttcttttgaacttctacatgcaccagcaactgtttgtggacctaaaaagtctactaatttggttaaaaacaaatgtgtcaatttcaacttcaatggtttaacaggcacaggtgttcttactgagtctaacaaaaagtttctgcctttccaacaatttggcagagacattgctgacactactgatgctgtccgtgatccacagacacttgagattcttgacattacaccatgttcttttggtggtgtcagtgttataacaccaggaacaaatacttctaaccaggttgctgttctttatcaggatgttaactgcacagaagtccctgttgctattcatgcagatcaacttactcctacttggcgtgtttattctacaggttctaatgtttttcaaacacgtgcaggctgtttaataggggctgaacatgtcaacaactcatatgagtgtgacatacccattggtgcaggtatatgcgctagttatcagactcagactaattctcctcggcgggcacgtagtgtagctagtcaatccatcattgcctacactatgtcacttggtgcagaaaattcagttgcttactctaataactctattgccatacccacaaattttactattagtgttaccacagaaattctaccagtgtctatgaccaagacatcagtagattgtacaatgtacatttgtggtgattcaactgaatgcagcaatcttttgttgcaatatggcagtttttgtacacaattaaaccgtgctttaactggaatagctgttgaacaagacaaaaacacccaagaagtttttgcacaagtcaaacaaatttacaaaacaccaccaattaaagattttggtggttttaatttttcacaaatattaccagatccatcaaaaccaagcaagaggtcatttattgaagatctacttttcaacaaagtgacacttgcagatgctggcttcatcaaacaatatggtgattgccttggtgatattgctgctagagacctcatttgtgcacaaaagtttaacggccttactgttttgccacctttgctcacagatgaaatgattgctcaatacacttctgcactgttagcgggtacaatcacttctggttggacctttggtgcaggtgctgcattacaaataccatttgctatgcaaatggcttataggtttaatggtattggagttacacagaatgttctctatgagaaccaaaaattgattgccaaccaatttaatagtgctattggcaaaattcaagactcactttcttccacagcaagtgcacttggaaaacttcaagatgtggtcaaccaaaatgcacaagctttaaacacgcttgttaaacaacttagctccaattttggtgcaatttcaagtgttttaaatgatatcctttcacgtcttgacaaagttgaggctgaagtgcaaattgataggttgatcacaggcagacttcaaagtttgcagacatatgtgactcaacaattaattagagctgcagaaatcagagcttctgctaatcttgctgctactaaaatgtcagagtgtgtacttggacaatcaaaaagagttgatttttgtggaaagggctatcatcttatgtccttccctcagtcagcacctcatggtgtagtcttcttgcatgtgacttatgtccctgcacaagaaaagaacttcacaactgctcctgccatttgtcatgatggaaaagcacactttcctcgtgaaggtgtctttgtttcaaatggcacacactggtttgtaacacaaaggaatttttatgaaccacaaatcattactacagacaacacatttgtgtctggtaactgtgatgttgtaataggaattgtcaacaacacagtttatgatcctttgcaacctgaattagactcattcaaggaggagttagataaatattttaagaatcatacatcaccagatgttgatttaggtgacatctctggcattaatgcttcagttgtaaacattcaaaaagaaattgaccgcctcaatgaggttgccaagaatttaaatgaatctctcatcgatctccaagaacttggaaagtatgagcagtatataaaatggccatggtacatttggctaggttttatagctggcttgattgccatagtaatggtgacaattatgctttgctgtatgaccagttgctgtagttgtctcaagggctgttgttcttgtggatcctgctgcaaatttgatgaagacgactctgagccagtgctcaaaggagtcaaattacattacacataatacgtattgccatgtgtatgtgggagacggtcgggtccagatattcgtatctgtcgagtagagtgtgggctcccacatactctgatgatccttcgggatcattcatggcaactcgagatagcataaaataacgccccaccttcttaacgggaggtggggcgttattttta

SEQ ID NO: 24 - DNA, 4063 bp, synthetic construct
  source 1..4063: mol_type = other DNA
taatacgactcactatagggtaccacgtagaccgtacggcagtaataaccagctgaccgcatacccgagtaatgtttgtgtttcttgtcctccttccactggtttcgagtcagtgcgtcaatcttacaacacgaacccagctgccgccagcctacacgaactccttcacgcggggagtgtactaccccgacaaggtgttccgctcgtctgttctgcacagcacgcaggacctcttcctcccgttcttctcgaacgtgacgtggttccatgccattcacgtttcgggaacgaacgggacgaagaggttcgataaccctgttctaccgtttaacgacggggtgtacttcgcttcgacagagaagtccaacattattcgcggatggatattcggaaccactctcgattccaagactcagtccttgttgatagtgaacaacgccacgaacgtggtcattaaggtctgtgagtttcagttctgtaatgacccgttcttgggtgtttactatcacaagaacaacaagtcttggatggagagtgagttccgagtgtattcatccgcgaataattgtaccttcgagtatgtcagtcagccgtttctgatggatcttgaaggcaaacagggcaatttcaagaatttgcgcgagtttgtcttcaagaacatcgacggctacttcaagatatactcgaagcacacgccaatcaacctcgtccgtgatctcccgcagggcttcagcgctctggaaccgctggtggacttgccgataggcatcaacatcacgcggttccagacgctgttagccctgcacaggagttacctgaccccaggtgactcctcgtccggttggactgcaggtgccgccgcgtactacgtggggtacctgcagccccggacgttcttgttgaagtacaacgagaacgggacgatcacggacgcggttgattgtgcgttggaccctctgtcggagacgaagtgcaccctgaagtcgtttacggtagaaaaggggatctatcagacctccaacttccgcgtccagccgactgagagtatcgttcggtttccgaacatcacgaacctgtgtccgtttggagaggtcttcaacgcgaccaggttcgcctccgtgtacgcttggaacaggaagaggatatcgaattgtgtagcagactacagtgtgctatacaattcggcgtccttttccactttcaagtgttacggagtgtcgcccacgaagttgaacgacctctgcttcaccaacgtgtacgcggattccttcgtcatccgtggtgacgaggttcggcagatcgcgcccggacagactggaaagatagcggactacaattataagttgcccgacgactttactggctgcgttattgcttggaatagcaataacttagacagtaaagtcgggggcaactataattacctgtatcgactgtttcggaaaagcaatctgaagcccttcgagcgcgacattagcacggagatctaccaggctggtagtactccgtgcaatggcgtggagggcttcaattgctattttccgttacagtcgtacgggtttcagcccaccaacggggtagggtaccagccctaccgcgtggtggtgctgtcgttcgaactccttcacgcacccgcgactgtctgtgggcccaagaagtcgacgaacttggtgaagaacaagtgcgtcaacttcaacttcaatgggctcacaggcacgggggtgctgacggagtcgaacaaaaagttcctacctttccagcagttcgggcgcgatattgccgacaccacggatgccgtaagggatccgcagacgcttgagattctggacatcacgccctgcagcttcgggggcgtcagtgtaatcacgcctggtaccaacacgagcaaccaggttgccgtgttgtaccaggacgtgaattgcactgaggtccccgtagcgatccacgcggatcagctaaccccaacgtggagggtgtactcgacagggagtaatgtcttccagactcgcgctggttgtctgattggcgctgagcatgtgaacaactcgtacgagtgtgacatccccattggagcggggatctgcgcgtcgtaccagacccagacgaacagcccgaggcgtgcccgctcagtagcgtcgcagtcgatcatcgcgtacacgatgagcttgggggcggagaacagtgtagcctattcgaacaacagcattgctatccccacaaattttacaattagtgtaaccaccgagatcttaccggtctccatgaccaagacctcggtggattgcactatgtatatttgtggggatagcactgagtgttctaacctcctgctccagtacggcagtttctgtacgcagctcaaccgagcgcttacaggaattgccgtggagcaggacaagaacactcaggaggtgtttgcccaggtcaagcagatctacaagacacctccgatcaaggactttggcggcttcaacttctcccagatactccccgaccccagcaagcccagcaagcgtagctttattgaagatctgctcttcaataaagttacgcttgctgatgctgggttcatcaagcagtacggggattgtctgggagatatagccgccagagacttgatctgtgctcagaagttcaatgggctcactgttctcccccccttgctcacggacgagatgatcgcccagtatacttcggcgctgctggcgggcacgatcacctcgggctggacgtttggggctggtgcggcgctgcagatccccttcgccatgcagatggcgtaccgcttcaatgggatcggtgtcacacagaacgttttgtacgagaatcagaagctcatcgccaatcagttcaacagcgcgatcgggaagatacaggactccctgtcgagtacagcctccgcgttggggaagctgcaggacgtggtgaaccagaatgctcaagcgttgaacacgttggtgaagcagttgtcgtccaacttcggggcgataagttcggtgctgaacgatattctcagtcggctggacaaggtggaagcggaggtccagatagatcggctcatcactggtcgcctccagagtttgcagacgtacgtaactcagcagctcatccgagctgctgagatacgtgcgtctgcaaacctggcggcgaccaagatgagcgagtgcgtgctggggcagagcaagcgagtggacttctgcgggaagggctatcacctgatgtccttcccgcagagcgcacctcacggggtagtctttctccacgtgacatatgtgccggcgcaggagaagaacttcaccactgcgccggccatatgtcacgatgggaaagcccacttcccgcgtgaaggagtttttgtatcaaacgggacgcattggttcgtcacgcagcgcaacttctatgagccacagataattaccactgacaatacctttgtcagtggtaattgtgatgtggtcatagggatcgtgaacaacacggtctacgatcccctgcagcccgagctagatagtttcaaggaggagcttgataagtacttcaagaatcatacttccccagacgtggatcttggcgacattagcggcatcaacgctagtgtcgtcaacatccagaaggagatcgacaggctcaatgaggttgccaagaacctcaacgagagcctgatcgatctccaggagctggggaagtatgagcagtacatcaagtggccttggtacatctggctcgggttcattgcagggttgatcgcgatcgtgatggtcacgatcatgttgtgctgcatgacgagctgttgctcctgtttgaagggctgctgcagctgtggttcgtgttgtaagtttgacgaggatgactcggagccagtgttgaagggggtcaagttacactacacataatacgtattgccatgtgtatgtgggagacggtcgggtccagatattcgtatctgtcgagtagagtgtgggctcccacatactctgatgatccttcgggatcattcatggcaactcgagatagcataaaataacgccccaccttcttaacgggaggtggggcgttattttta

SEQ ID NO: 25 - DNA, 6982 bp, synthetic construct
  source 1..6982: mol_type = other DNA
gtagtactcagctgtaatacgactcactatagggagacccaagctggctagcgtttaaacttaagcttggcaatccggtactgttggtaaagccaccatggaagatgccaaaaacattaagaagggcccagcgccattctacccactcgaagacgggaccgccggcgagcagctgcacaaagccatgaagcgctacgccctggtgcccggcaccatcgcctttaccgacgcacatatcgaggtggacattacctacgccgagtacttcgagatgagcgttcggctggcagaagctatgaagcgctatgggctgaatacaaaccatcggatcgtggtgtgcagcgagaatagcttgcagttcttcatgcccgtgttgggtgccctgttcatcggtgtggctgtggccccagctaacgacatctacaacgagcgcgagctgctgaacagcatgggcatcagccagcccaccgtcgtattcgtgagcaagaaagggctgcaaaagatcctcaacgtgcaaaagaagctaccgatcatacaaaagatcatcatcatggatagcaagaccgactaccagggcttccaaagcatgtacaccttcgtgacttcccatttgccacccggcttcaacgagtacgacttcgtgcccgagagcttcgaccgggacaaaaccatcgccctgatcatgaacagtagtggcagtaccggattgcccaagggcgtagccctaccgcaccgcaccgcttgtgtccgattcagtcatgcccgcgaccccatcttcggcaaccagatcatccccgacaccgctatcctcagcgtggtgccatttcaccacggcttcggcatgttcaccacgctgggctacttgatctgcggctttcgggtcgtgctcatgtaccgcttcgaggaggagctattcttgcgcagcttgcaagactataagattcaatctgccctgctggtgcccacactatttagcttcttcgctaagagcactctcatcgacaagtacgacctaagcaacttgcacgagatcgccagcggcggggcgccgctcagcaaggaggtaggtgaggccgtggccaaacgcttccacctaccaggcatccgccagggctacggcctgacagaaacaaccagcgccattctgatcacccccgaaggggacgacaagcctggcgcagtaggcaaggtggtgcccttcttcgaggctaaggtggtggacttggacaccggtaagacactgggtgtgaaccagcgcggcgagctgtgcgtccgtggccccatgatcatgagcggctacgttaacaaccccgaggctacaaacgctctcatcgacaaggacggctggctgcacagcggcgacatcgcctactgggacgaggacgagcacttcttcatcgtggaccggctgaagagcctgatcaaatacaagggctaccaggtagccccagccgaactggagagcatcctgctgcaacaccccaacatcttcgacgccggggtcgccggcctgcccgacgacgatgccggcgagctgcccgccgcagtcgtcgtgctggaacacggtaaaaccatgaccgagaaggagatcgtggactatgtggccagccaggttacaaccgccaagaagctgcgcggtggtgttgtgttcgtggacgaggtgcctaaaggactgaccggcaagttggacgcccgcaagatccgcgagattctcattaaggccaagaagggcggcaagatcgccgtgtaataatacgtattgccatgtgtatgtgggagacggtcgggtccagatattcgtatctgtcgagtagagtgtgggctcccacatactctgatgatccttcgggatcattcatggcaactcgagatagcataaaataacgccccaccttcttaacgggaggtggggcgttatttttactgaaagatatcatccaatggatctgtcgacggccgtcgttttacagccaagcttggctgttttggcggatgagagaagattttcagcctgatacagattaaatcagaacgcagaagcggtctgataaaacagaatttgcctggcggcagtagcgcggtggtcccacctgaccccatgccgaactcagaagtgaaacgccgtagcgccgatggtagtgtggggtctccccatgcgagagtagggaactgccaggcatcaaataaaacgaaaggctcagtcgaaagactgggcctttcgttttatctgttgtttgtcggtgaacgctctcctgagtaggacaaatccgccgggagcggatttgaacgttgcgaagcaacggcccggagggtggcgggcaggacgcccgccataaactgccaggcatcaaattaagcagaaggccatcctgacggatggcctttttgcgtttctacaaactcttttggtcgactctagagttccactgagcgtcagaccccgtagaaaagatcaaaggatcttcttgagatcctttttttctgcgcgtaatctgctgcttgcaaacaaaaaaaccaccgctaccagcggtggtttgtttgccggatcaagagctaccaactctttttccgaaggtaactggcttcagcagagcgcagataccaaatactgtccttctagtgtagccgtagttaggccaccacttcaagaactctgtagcaccgcctacatacctcgctctgctaatcctgttaccagtggctgctgccagtggcgataagtcgtgtcttaccgggttggactcaagacgatagttaccggataaggcgcagcggtcgggctgaacggggggttcgtgcacacagcccagcttggagcgaacgacctacaccgaactgagatacctacagcgtgagctatgagaaagcgccacgcttcccgaagggagaaaggcggacaggtatccggtaagcggcagggtcggaacaggagagcgcacgagggagcttccagggggaaacgcctggtatctttatagtcctgtcgggtttcgccacctctgacttgagcgtcgatttttgtgatgctcgtcaggggggcggagcctatggaaaaacgccagcaacgcggcctttttacggttcctggccttttgctggccttttgctcacatgttctttcctgcgttatcccctgattctgtggataaccgtattaccgcctttgagtgagctgataccgctcgccgcagccgaacgaccgagcgcagcgagtcagtgagcgaggaagcggaagatctagaagtactgctgactcataccaggcctgaatcgccccatcatccagccagaaagtgagggagccacggttgatgagagctttgttgtaggtggaccagttggtgattttgaacttttgctttgccacggaacggtctgcgttgtcgggaagatgcgtgatctgatccttcaactcagcaaaagttcgatttattcaacaaagccacgttgtgtctcaaaatctctgatgttacattgcacaagataaaaatatatcatcatgaacaataaaactgtctgcttacataaacagtaatacaaggggtgttatgagccatattcaacgggaaacgtcttgctcaaggccgcgattaaattccaacatggatgctgatttatatgggtataaatgggctcgcgataatgtcgggcaatcaggtgcgacaatctatcgattgtatgggaagcccgatgcgccagagttgtttctgaaacatggcaaaggtagcgttgccaatgatgttacagatgagatggtcagactaaactggctgacggaatttatgcctcttccgaccatcaagcattttatccgtactcctgatgatgcatggttactcaccactgcgatccccggaaaaacagcattccaggtattagaagaatatcctgattcaggtgaaaatattgttgatgcgctggcagtgttcctgcgccggttgcattcgattcctgtttgtaattgtccttttaacagcgatcgcgtatttcgtctcgctcaggcgcaatcacgaatgaataacggtttggttgatgcgagtgattttgatgacgagcgtaatggctggcctgttgaacaagtctggaaagaaatgcataagcttttgccattctcaccggattcagtcgtcactcatggtgatttctcacttgataaccttatttttgacgaggggaaattaataggttgtattgatgttggacgagtcggaatcgcagaccgataccaggatcttgccatcctatggaactgcctcggtgagttttctccttcattacagaaacggctttttcaaaaatatggtattgataatcctgatatgaataaattgcagtttcatttgatgctcgatgagtttttctaaggctagccccgggactagtgatctttgggagcagtccttgtgcgcttacgaggtgagccggtggggaaccgttatctgcctatggtgtgagcccccctagagagcttcaagagcaatcagcccgacctagaaaggaggccaagagagagacccctacggggggaaccgttttctgcctacgagatggcacatttactgggaagctttacggcgtcctcgtggaagttcaatgcccgcagacttaagtgctctattcacggtctgacgtgacacgctaaattcagacatagcttcattgattgtcggccacgagccagtctctccctcaacagtcataaaccaacctgcaatggtcaagcgattttctttagctttcctagcttgtcgttgactggacttagctagtttttctcgctgtgctcgggcgtactcactgtttgggtctttccagcgttctgcggcctttttaccgccacgtcttcccatagtggccagagcttttcgccctcggctgctctgcgtctctgtctgacgagcagggacgactggctggcctttagcgacgtagccgcgcacacgtcgcgccatcgtctggcggtcacgcatcggcggcagatcaggctcacggccgtctgctccgaccgcctgagcgacggtgtaggcacgctcgtaggcgtcgatgatcttggtgtcttttaggcgctcaccagccgcttttaactggtatcccacagtcaaagcgtggcgaaaagccgtctcatcacgggcggcacgccctggagcagtccagaggacacggacgccgtcgatcagctctccagacgcttcagcggcgctcggcaggcttgcttcaagcgtggcaagtgcttttgcttccgcagtggcttttcttgccgcttcgatacgtgcccgtccgctagaaaactcctgctcatagcgttttttaggtttttctgtgcctgagatcatgcgagcaacctccataagatcagctaggcgatccacgcgattgtgctgggcatgccagcggtacgcggtgggatcgtcggagacgtgcagtggccaccggctcagcctatgtgaaaaagcctggtcagcgccgaaaacgcgggtcatttcctcggtcgttgcagccagcaggcgcatattcgggctgctcatgcctgctgcggcatacaccggatcaatgagccagatgagctggcatttcccgctcagtggattcacgccgatccaagctggcgctttttccaggcgtgcccagcgctccaaaatcgcgtagacctcggggtttacgtgctcgattttcccgccggcctggtggctcggcacatcaatgtccaggacaagcacggctgcgtgctgcgcgtgcgtcagagcaacatactggcaccgggcaagcgattttgaaccaactcggtataacttcggctgtgtttctcccgtgtccgggtctttgatccaagcgctggcgaagtcgcgggtcttgctgccctggaaattttctctgcccaggtgagcgaggaattcgcggcggtcttcgctcgtccagccacgtgatcgcagcgcgagctcgggatgggtgtcgaacagatcagcggaaaatttccaggccggtgtgtcaatgtctcgtgaatccgctagagtcatttttgagcgctttctcccaggtttggactgggggttagccgacgccctgtgagttaccgctcacggggcgttcaacatttttcaggtattcgtgcagcttatcgcttcttgccgcctgtgcgctttttcgacgcgcgacgctgctgccgattcggtgcaggtggtggcggcgctgacacgtcctgggcggccacggccacacgaaacgcggcatttacgatgtttgtcatgcctgcgggcaccgcgccacgatcgcggataattctcgctgccgcttccagctctgtgacgaccatggccaaaatttcgctcgggggacgcacttccagcgccatttgcgacctagccgcctccagctcctcggcgtggcgtttgttggcgcgctcgcggctggctgcggcacgacacgcatctgagcaatattttgcgcgccgtcctcgcgggtcaggccggggaggaatcaggccaccgcagtaggcgcaactgattcgatcctccactactgtgcgtcctcctggcgctgccgagcacgcagctcgtcagccagctcctcaagatccgccacgagagtttctaggtcgctcgcggcactggcccagtctcgtgatgctggcgcgtccgtcgtatcgagagctcggaaaaatccgatcaccgtttttaaatcgacggcagcatcgagcgcgtcggactccagcgcgacatcagagagatccatagctgatgattcgggccaattttggtacttcgtcgtgaaggtcatgacaccattataacgaacgttcgttaaagtttttggcggaaaatcacgcggcacgaaaattttcacgaagcgggactttgcgcagctcaggggtgctaaaaattttgtatcgcacttgatttttccgaaagacagattatctgcaaacggtgtgtcgtatttctggcttggtttttaaaaaatctggaatcgaaaatttgcggggcga

SEQ ID NO: 26 - DNA, 6982 bp, synthetic construct
  source 1..6982: mol_type = other DNA
gtagtactcagctgtaatacgactcactatagggagacccaagctggctagcgtttaaacttaagcttggcaatccggtactgttggtaaagccaccatggaggacgcaaagaatattaagaagggccctgcgcccttctatcctttggaggacggtactgccggggagcagctgcataaggctatgaagcgttatgcgctggtccccggcactatcgccttcacggacgctcatatcgaagtagacatcacatatgctgagtacttcgaaatgagcgtccgtctcgctgaggccatgaagcggtatggtttgaacacaaaccaccgcatcgtggtctgcagcgagaattctttgcagttcttcatgcctgttctgggagccctgtttatcggtgttgctgtcgcacctgctaatgatatttataatgaacgggagcttcttaatagcatggggatctcgcagcccactgttgttttcgtgagcaagaaggggctgcagaagatcctcaatgtgcagaagaagctcccgatcattcagaaaatcattatcatggacagcaagaccgattatcagggcttccagagcatgtatacttttgtcacatcgcacttgccccccggctttaatgagtatgattttgtcccggagagttttgatcgggacaagactattgccctgatcatgaactcttcgggatccacgggtcttcctaagggcgtcgcgcttccccaccgaaccgcgtgtgtgagatttagccacgctcgggatcccatattcgggaatcaaattatcccggatacggcgatcctgagcgtggttccgtttcaccacgggttcggtatgttcacgacccttgggtacctcatctgcggattccgcgtagtcctgatgtatcgctttgaggaggaactgtttctccgcagcctccaagactacaagattcagtcggcgctcctagtcccgacgctattctcgttctttgccaagtcgaccttgattgacaagtacgacttgagcaatttgcacgagatagcgtcgggaggagcgccgctgagtaaggaagtcggggaggctgtggcgaaacggttccacctcccagggatacgtcagggctacggcctgactgagacgacgtccgcgatccttatcaccccggagggggatgataagccgggtgctgtcggcaaggtggttccgttcttcgaggccaaagtggtagaccttgatactggtaagactcttggggtgaatcaacgaggagaattgtgcgtccgtggtcccatgattatgtcaggctatgtcaataaccccgaggcaaccaacgccttgattgacaaggacggttggttgcactcgggggacatagcctactgggacgaggacgagcatttcttcatcgttgatcgcctcaagagtcttatcaagtacaagggctaccaggtggccccggcagaactggaatccatcttgctgcagcacccgaatatcttcgacgctggtgttgccgggctcccggacgacgacgccggggaacttcccgcggccgtcgtcgtcctggagcacggcaagaccatgacggagaaggagatcgtggactacgtcgccagtcaggtcaccaccgcgaagaaacttcgcggtggtgtggtgttcgtagatgaggtacccaagggtctgacggggaagctcgacgcccggaagatccgtgaaatactcattaaagccaaaaaggggggcaagattgcggtgtgataatacgtattgccatgtgtatgtgggagacggtcgggtccagatattcgtatctgtcgagtagagtgtgggctcccacatactctgatgatccttcgggatcattcatggcaactcgagatagcataaaataacgccccaccttcttaacgggaggtggggcgttatttttactgaaagatatcatccaatggatctgtcgacggccgtcgttttacagccaagcttggctgttttggcggatgagagaagattttcagcctgatacagattaaatcagaacgcagaagcggtctgataaaacagaatttgcctggcggcagtagcgcggtggtcccacctgaccccatgccgaactcagaagtgaaacgccgtagcgccgatggtagtgtggggtctccccatgcgagagtagggaactgccaggcatcaaataaaacgaaaggctcagtcgaaagactgggcctttcgttttatctgttgtttgtcggtgaacgctctcctgagtaggacaaatccgccgggagcggatttgaacgttgcgaagcaacggcccggagggtggcgggcaggacgcccgccataaactgccaggcatcaaattaagcagaaggccatcctgacggatggcctttttgcgtttctacaaactcttttggtcgactctagagttccactgagcgtcagaccccgtagaaaagatcaaaggatcttcttgagatcctttttttctgcgcgtaatctgctgcttgcaaacaaaaaaaccaccgctaccagcggtggtttgtttgccggatcaagagctaccaactctttttccgaaggtaactggcttcagcagagcgcagataccaaatactgtccttctagtgtagccgtagttaggccaccacttcaagaactctgtagcaccgcctacatacctcgctctgctaatcctgttaccagtggctgctgccagtggcgataagtcgtgtcttaccgggttggactcaagacgatagttaccggataaggcgcagcggtcgggctgaacggggggttcgtgcacacagcccagcttggagcgaacgacctacaccgaactgagatacctacagcgtgagctatgagaaagcgccacgcttcccgaagggagaaaggcggacaggtatccggtaagcggcagggtcggaacaggagagcgcacgagggagcttccagggggaaacgcctggtatctttatagtcctgtcgggtttcgccacctctgacttgagcgtcgatttttgtgatgctcgtcaggggggcggagcctatggaaaaacgccagcaacgcggcctttttacggttcctggccttttgctggccttttgctcacatgttctttcctgcgttatcccctgattctgtggataaccgtattaccgcctttgagtgagctgataccgctcgccgcagccgaacgaccgagcgcagcgagtcagtgagcgaggaagcggaagatctagaagtactgctgactcataccaggcctgaatcgccccatcatccagccagaaagtgagggagccacggttgatgagagctttgttgtaggtggaccagttggtgattttgaacttttgctttgccacggaacggtctgcgttgtcgggaagatgcgtgatctgatccttcaactcagcaaaagttcgatttattcaacaaagccacgttgtgtctcaaaatctctgatgttacattgcacaagataaaaatatatcatcatgaacaataaaactgtctgcttacataaacagtaatacaaggggtgttatgagccatattcaacgggaaacgtcttgctcaaggccgcgattaaattccaacatggatgctgatttatatgggtataaatgggctcgcgataatgtcgggcaatcaggtgcgacaatctatcgattgtatgggaagcccgatgcgccagagttgtttctgaaacatggcaaaggtagcgttgccaatgatgttacagatgagatggtcagactaaactggctgacggaatttatgcctcttccgaccatcaagcattttatccgtactcctgatgatgcatggttactcaccactgcgatccccggaaaaacagcattccaggtattagaagaatatcctgattcaggtgaaaatattgttgatgcgctggcagtgttcctgcgccggttgcattcgattcctgtttgtaattgtccttttaacagcgatcgcgtatttcgtctcgctcaggcgcaatcacgaatgaataacggtttggttgatgcgagtgattttgatgacgagcgtaatggctggcctgttgaacaagtctggaaagaaatgcataagcttttgccattctcaccggattcagtcgtcactcatggtgatttctcacttgataaccttatttttgacgaggggaaattaataggttgtattgatgttggacgagtcggaatcgcagaccgataccaggatcttgccatcctatggaactgcctcggtgagttttctccttcattacagaaacggctttttcaaaaatatggtattgataatcctgatatgaataaattgcagtttcatttgatgctcgatgagtttttctaaggctagccccgggactagtgatctttgggagcagtccttgtgcgcttacgaggtgagccggtggggaaccgttatctgcctatggtgtgagcccccctagagagcttcaagagcaatcagcccgacctagaaaggaggccaagagagagacccctacggggggaaccgttttctgcctacgagatggcacatttactgggaagctttacggcgtcctcgtggaagttcaatgcccgcagacttaagtgctctattcacggtctgacgtgacacgctaaattcagacatagcttcattgattgtcggccacgagccagtctctccctcaacagtcataaaccaacctgcaatggtcaagcgattttctttagctttcctagcttgtcgttgactggacttagctagtttttctcgctgtgctcgggcgtactcactgtttgggtctttccagcgttctgcggcctttttaccgccacgtcttcccatagtggccagagcttttcgccctcggctgctctgcgtctctgtctgacgagcagggacgactggctggcctttagcgacgtagccgcgcacacgtcgcgccatcgtctggcggtcacgcatcggcggcagatcaggctcacggccgtctgctccgaccgcctgagcgacggtgtaggcacgctcgtaggcgtcgatgatcttggtgtcttttaggcgctcaccagccgcttttaactggtatcccacagtcaaagcgtggcgaaaagccgtctcatcacgggcggcacgccctggagcagtccagaggacacggacgccgtcgatcagctctccagacgcttcagcggcgctcggcaggcttgcttcaagcgtggcaagtgcttttgcttccgcagtggcttttcttgccgcttcgatacgtgcccgtccgctagaaaactcctgctcatagcgttttttaggtttttctgtgcctgagatcatgcgagcaacctccataagatcagctaggcgatccacgcgattgtgctgggcatgccagcggtacgcggtgggatcgtcggagacgtgcagtggccaccggctcagcctatgtgaaaaagcctggtcagcgccgaaaacgcgggtcatttcctcggtcgttgcagccagcaggcgcatattcgggctgctcatgcctgctgcggcatacaccggatcaatgagccagatgagctggcatttcccgctcagtggattcacgccgatccaagctggcgctttttccaggcgtgcccagcgctccaaaatcgcgtagacctcggggtttacgtgctcgattttcccgccggcctggtggctcggcacatcaatgtccaggacaagcacggctgcgtgctgcgcgtgcgtcagagcaacatactggcaccgggcaagcgattttgaaccaactcggtataacttcggctgtgtttctcccgtgtccgggtctttgatccaagcgctggcgaagtcgcgggtcttgctgccctggaaattttctctgcccaggtgagcgaggaattcgcggcggtcttcgctcgtccagccacgtgatcgcagcgcgagctcgggatgggtgtcgaacagatcagcggaaaatttccaggccggtgtgtcaatgtctcgtgaatccgctagagtcatttttgagcgctttctcccaggtttggactgggggttagccgacgccctgtgagttaccgctcacggggcgttcaacatttttcaggtattcgtgcagcttatcgcttcttgccgcctgtgcgctttttcgacgcgcgacgctgctgccgattcggtgcaggtggtggcggcgctgacacgtcctgggcggccacggccacacgaaacgcggcatttacgatgtttgtcatgcctgcgggcaccgcgccacgatcgcggataattctcgctgccgcttccagctctgtgacgaccatggccaaaatttcgctcgggggacgcacttccagcgccatttgcgacctagccgcctccagctcctcggcgtggcgtttgttggcgcgctcgcggctggctgcggcacgacacgcatctgagcaatattttgcgcgccgtcctcgcgggtcaggccggggaggaatcaggccaccgcagtaggcgcaactgattcgatcctccactactgtgcgtcctcctggcgctgccgagcacgcagctcgtcagccagctcctcaagatccgccacgagagtttctaggtcgctcgcggcactggcccagtctcgtgatgctggcgcgtccgtcgtatcgagagctcggaaaaatccgatcaccgtttttaaatcgacggcagcatcgagcgcgtcggactccagcgcgacatcagagagatccatagctgatgattcgggccaattttggtacttcgtcgtgaaggtcatgacaccattataacgaacgttcgttaaagtttttggcggaaaatcacgcggcacgaaaattttcacgaagcgggactttgcgcagctcaggggtgctaaaaattttgtatcgcacttgatttttccgaaagacagattatctgcaaacggtgtgtcgtatttctggcttggtttttaaaaaatctggaatcgaaaatttgcggggcga

SEQ ID NO: 27 - DNA, 9136 bp, synthetic construct
  source 1..9136: mol_type = other DNA
gtagtactcagctgtaatacgactcactatagggtaccacgtagaccgtacggcagtaataaccagctgaccgcatacccgagtaatgtttgtttttcttgttttattgccactagtctctagtcagtgtgttaatcttacaaccagaactcaattaccccctgcatacactaattctttcacacgtggtgtttattaccctgacaaagttttcagatcctcagttttacattcaactcaggacttgttcttacctttcttttccaatgttacttggttccatgctatacatgtctctgggaccaatggtactaagaggtttgataaccctgtcctaccatttaatgatggtgtttattttgcttccactgagaagtctaacataataagaggctggatttttggtactactttagattcgaagacccagtccctacttattgttaataacgctactaatgttgttattaaagtctgtgaatttcaattttgtaatgatccatttttgggtgtttattaccacaaaaacaacaaaagttggatggaaagtgagttcagagtttattctagtgcgaataattgcacttttgaatatgtctctcagccttttcttatggaccttgaaggaaaacagggtaatttcaaaaatcttagggaatttgtgtttaagaatattgatggttattttaaaatatattctaagcacacgcctattaatttagtgcgtgatctccctcagggtttttcggctttagaaccattggtagatttgccaataggtattaacatcactaggtttcaaactttacttgctttacatagaagttatttgactcctggtgattcttcttcaggttggacagctggtgctgcagcttattatgtgggttatcttcaacctaggacttttctattaaaatataatgaaaatggaaccattacagatgctgtagactgtgcacttgaccctctctcagaaacaaagtgtacgttgaaatccttcactgtagaaaaaggaatctatcaaacttctaactttagagtccaaccaacagaatctattgttagatttcctaatattacaaacttgtgcccttttggtgaagtttttaacgccaccagatttgcatctgtttatgcttggaacaggaagagaatcagcaactgtgttgctgattattctgtcctatataattccgcatcattttccacttttaagtgttatggagtgtctcctactaaattaaatgatctctgctttactaatgtctatgcagattcatttgtaattagaggtgatgaagtcagacaaatcgctccagggcaaactggaaagattgctgattataattataaattaccagatgattttacaggctgcgttatagcttggaattctaacaatcttgattctaaggttggtggtaattataattacctgtatagattgtttaggaagtctaatctcaaaccttttgagagagatatttcaactgaaatctatcaggccggtagcacaccttgtaatggtgttgaaggttttaattgttactttcctttacaatcatatggtttccaacccactaatggtgttggttaccaaccatacagagtagtagtactttcttttgaacttctacatgcaccagcaactgtttgtggacctaaaaagtctactaatttggttaaaaacaaatgtgtcaatttcaacttcaatggtttaacaggcacaggtgttcttactgagtctaacaaaaagtttctgcctttccaacaatttggcagagacattgctgacactactgatgctgtccgtgatccacagacacttgagattcttgacattacaccatgttcttttggtggtgtcagtgttataacaccaggaacaaatacttctaaccaggttgctgttctttatcaggatgttaactgcacagaagtccctgttgctattcatgcagatcaacttactcctacttggcgtgtttattctacaggttctaatgtttttcaaacacgtgcaggctgtttaataggggctgaacatgtcaacaactcatatgagtgtgacatacccattggtgcaggtatatgcgctagttatcagactcagactaattctcctcggcgggcacgtagtgtagctagtcaatccatcattgcctacactatgtcacttggtgcagaaaattcagttgcttactctaataactctattgccatacccacaaattttactattagtgttaccacagaaattctaccagtgtctatgaccaagacatcagtagattgtacaatgtacatttgtggtgattcaactgaatgcagcaatcttttgttgcaatatggcagtttttgtacacaattaaaccgtgctttaactggaatagctgttgaacaagacaaaaacacccaagaagtttttgcacaagtcaaacaaatttacaaaacaccaccaattaaagattttggtggttttaatttttcacaaatattaccagatccatcaaaaccaagcaagaggtcatttattgaagatctacttttcaacaaagtgacacttgcagatgctggcttcatcaaacaatatggtgattgccttggtgatattgctgctagagacctcatttgtgcacaaaagtttaacggccttactgttttgccacctttgctcacagatgaaatgattgctcaatacacttctgcactgttagcgggtacaatcacttctggttggacctttggtgcaggtgctgcattacaaataccatttgctatgcaaatggcttataggtttaatggtattggagttacacagaatgttctctatgagaaccaaaaattgattgccaaccaatttaatagtgctattggcaaaattcaagactcactttcttccacagcaagtgcacttggaaaacttcaagatgtggtcaaccaaaatgcacaagctttaaacacgcttgttaaacaacttagctccaattttggtgcaatttcaagtgttttaaatgatatcctttcacgtcttgacaaagttgaggctgaagtgcaaattgataggttgatcacaggcagacttcaaagtttgcagacatatgtgactcaacaattaattagagctgcagaaatcagagcttctgctaatcttgctgctactaaaatgtcagagtgtgtacttggacaatcaaaaagagttgatttttgtggaaagggctatcatcttatgtccttccctcagtcagcacctcatggtgtagtcttcttgcatgtgacttatgtccctgcacaagaaaagaacttcacaactgctcctgccatttgtcatgatggaaaagcacactttcctcgtgaaggtgtctttgtttcaaatggcacacactggtttgtaacacaaaggaatttttatgaaccacaaatcattactacagacaacacatttgtgtctggtaactgtgatgttgtaataggaattgtcaacaacacagtttatgatcctttgcaacctgaattagactcattcaaggaggagttagataaatattttaagaatcatacatcaccagatgttgatttaggtgacatctctggcattaatgcttcagttgtaaacattcaaaaagaaattgaccgcctcaatgaggttgccaagaatttaaatgaatctctcatcgatctccaagaacttggaaagtatgagcagtatataaaatggccatggtacatttggctaggttttatagctggcttgattgccatagtaatggtgacaattatgctttgctgtatgaccagttgctgtagttgtctcaagggctgttgttcttgtggatcctgctgcaaatttgatgaagacgactctgagccagtgctcaaaggagtcaaattacattacacataatacgtattgccatgtgtatgtgggagacggtcgggtccagatattcgtatctgtcgagtagagtgtgggctcccacatactctgatgatccttcgggatcattcatggcaactcgagatagcataaaataacgccccaccttcttaacgggaggtggggcgttatttttactgaaagatatcatccaatggatctgtcgacggccgtcgttttacagccaagcttggctgttttggcggatgagagaagattttcagcctgatacagattaaatcagaacgcagaagcggtctgataaaacagaatttgcctggcggcagtagcgcggtggtcccacctgaccccatgccgaactcagaagtgaaacgccgtagcgccgatggtagtgtggggtctccccatgcgagagtagggaactgccaggcatcaaataaaacgaaaggctcagtcgaaagactgggcctttcgttttatctgttgtttgtcggtgaacgctctcctgagtaggacaaatccgccgggagcggatttgaacgttgcgaagcaacggcccggagggtggcgggcaggacgcccgccataaactgccaggcatcaaattaagcagaaggccatcctgacggatggcctttttgcgtttctacaaactcttttggtcgactctagagttccactgagcgtcagaccccgtagaaaagatcaaaggatcttcttgagatcctttttttctgcgcgtaatctgctgcttgcaaacaaaaaaaccaccgctaccagcggtggtttgtttgccggatcaagagctaccaactctttttccgaaggtaactggcttcagcagagcgcagataccaaatactgtccttctagtgtagccgtagttaggccaccacttcaagaactctgtagcaccgcctacatacctcgctctgctaatcctgttaccagtggctgctgccagtggcgataagtcgtgtcttaccgggttggactcaagacgatagttaccggataaggcgcagcggtcgggctgaacggggggttcgtgcacacagcccagcttggagcgaacgacctacaccgaactgagatacctacagcgtgagctatgagaaagcgccacgcttcccgaagggagaaaggcggacaggtatccggtaagcggcagggtcggaacaggagagcgcacgagggagcttccagggggaaacgcctggtatctttatagtcctgtcgggtttcgccacctctgacttgagcgtcgatttttgtgatgctcgtcaggggggcggagcctatggaaaaacgccagcaacgcggcctttttacggttcctggccttttgctggccttttgctcacatgttctttcctgcgttatcccctgattctgtggataaccgtattaccgcctttgagtgagctgataccgctcgccgcagccgaacgaccgagcgcagcgagtcagtgagcgaggaagcggaagatctagaagtactgctgactcataccaggcctgaatcgccccatcatccagccagaaagtgagggagccacggttgatgagagctttgttgtaggtggaccagttggtgattttgaacttttgctttgccacggaacggtctgcgttgtcgggaagatgcgtgatctgatccttcaactcagcaaaagttcgatttattcaacaaagccacgttgtgtctcaaaatctctgatgttacattgcacaagataaaaatatatcatcatgaacaataaaactgtctgcttacataaacagtaatacaaggggtgttatgagccatattcaacgggaaacgtcttgctcaaggccgcgattaaattccaacatggatgctgatttatatgggtataaatgggctcgcgataatgtcgggcaatcaggtgcgacaatctatcgattgtatgggaagcccgatgcgccagagttgtttctgaaacatggcaaaggtagcgttgccaatgatgttacagatgagatggtcagactaaactggctgacggaatttatgcctcttccgaccatcaagcattttatccgtactcctgatgatgcatggttactcaccactgcgatccccggaaaaacagcattccaggtattagaagaatatcctgattcaggtgaaaatattgttgatgcgctggcagtgttcctgcgccggttgcattcgattcctgtttgtaattgtccttttaacagcgatcgcgtatttcgtctcgctcaggcgcaatcacgaatgaataacggtttggttgatgcgagtgattttgatgacgagcgtaatggctggcctgttgaacaagtctggaaagaaatgcataagcttttgccattctcaccggattcagtcgtcactcatggtgatttctcacttgataaccttatttttgacgaggggaaattaataggttgtattgatgttggacgagtcggaatcgcagaccgataccaggatcttgccatcctatggaactgcctcggtgagttttctccttcattacagaaacggctttttcaaaaatatggtattgataatcctgatatgaataaattgcagtttcatttgatgctcgatgagtttttctaaggctagccccgggactagtgatctttgggagcagtccttgtgcgcttacgaggtgagccggtggggaaccgttatctgcctatggtgtgagcccccctagagagcttcaagagcaatcagcccgacctagaaaggaggccaagagagagacccctacggggggaaccgttttctgcctacgagatggcacatttactgggaagctttacggcgtcctcgtggaagttcaatgcccgcagacttaagtgctctattcacggtctgacgtgacacgctaaattcagacatagcttcattgattgtcggccacgagccagtctctccctcaacagtcataaaccaacctgcaatggtcaagcgattttctttagctttcctagcttgtcgttgactggacttagctagtttttctcgctgtgctcgggcgtactcactgtttgggtctttccagcgttctgcggcctttttaccgccacgtcttcccatagtggccagagcttttcgccctcggctgctctgcgtctctgtctgacgagcagggacgactggctggcctttagcgacgtagccgcgcacacgtcgcgccatcgtctggcggtcacgcatcggcggcagatcaggctcacggccgtctgctccgaccgcctgagcgacggtgtaggcacgctcgtaggcgtcgatgatcttggtgtcttttaggcgctcaccagccgcttttaactggtatcccacagtcaaagcgtggcgaaaagccgtctcatcacgggcggcacgccctggagcagtccagaggacacggacgccgtcgatcagctctccagacgcttcagcggcgctcggcaggcttgcttcaagcgtggcaagtgcttttgcttccgcagtggcttttcttgccgcttcgatacgtgcccgtccgctagaaaactcctgctcatagcgttttttaggtttttctgtgcctgagatcatgcgagcaacctccataagatcagctaggcgatccacgcgattgtgctgggcatgccagcggtacgcggtgggatcgtcggagacgtgcagtggccaccggctcagcctatgtgaaaaagcctggtcagcgccgaaaacgcgggtcatttcctcggtcgttgcagccagcaggcgcatattcgggctgctcatgcctgctgcggcatacaccggatcaatgagccagatgagctggcatttcccgctcagtggattcacgccgatccaagctggcgctttttccaggcgtgcccagcgctccaaaatcgcgtagacctcggggtttacgtgctcgattttcccgccggcctggtggctcggcacatcaatgtccaggacaagcacggctgcgtgctgcgcgtgcgtcagagcaacatactggcaccgggcaagcgattttgaaccaactcggtataacttcggctgtgtttctcccgtgtccgggtctttgatccaagcgctggcgaagtcgcgggtcttgctgccctggaaattttctctgcccaggtgagcgaggaattcgcggcggtcttcgctcgtccagccacgtgatcgcagcgcgagctcgggatgggtgtcgaacagatcagcggaaaatttccaggccggtgtgtcaatgtctcgtgaatccgctagagtcatttttgagcgctttctcccaggtttggactgggggttagccgacgccctgtgagttaccgctcacggggcgttcaacatttttcaggtattcgtgcagcttatcgcttcttgccgcctgtgcgctttttcgacgcgcgacgctgctgccgattcggtgcaggtggtggcggcgctgacacgtcctgggcggccacggccacacgaaacgcggcatttacgatgtttgtcatgcctgcgggcaccgcgccacgatcgcggataattctcgctgccgcttccagctctgtgacgaccatggccaaaatttcgctcgggggacgcacttccagcgccatttgcgacctagccgcctccagctcctcggcgtggcgtttgttggcgcgctcgcggctggctgcggcacgacacgcatctgagcaatattttgcgcgccgtcctcgcgggtcaggccggggaggaatcaggccaccgcagtaggcgcaactgattcgatcctccactactgtgcgtcctcctggcgctgccgagcacgcagctcgtcagccagctcctcaagatccgccacgagagtttctaggtcgctcgcggcactggcccagtctcgtgatgctggcgcgtccgtcgtatcgagagctcggaaaaatccgatcaccgtttttaaatcgacggcagcatcgagcgcgtcggactccagcgcgacatcagagagatccatagctgatgattcgggccaattttggtacttcgtcgtgaaggtcatgacaccattataacgaacgttcgttaaagtttttggcggaaaatcacgcggcacgaaaattttcacgaagcgggactttgcgcagctcaggggtgctaaaaattttgtatcgcacttgatttttccgaaagacagattatctgcaaacggtgtgtcgtatttctggcttggtttttaaaaaatctggaatcgaaaatttgcggggcga

SEQ ID NO: 28 - DNA, 9136 bp, synthetic construct
  source 1..9136: mol_type = other DNA
gtagtactcagctgtaatacgactcactatagggtaccacgtagaccgtacggcagtaataaccagctgaccgcatacccgagtaatgtttgtgtttcttgtcctccttccactggtttcgagtcagtgcgtcaatcttacaacacgaacccagctgccgccagcctacacgaactccttcacgcggggagtgtactaccccgacaaggtgttccgctcgtctgttctgcacagcacgcaggacctcttcctcccgttcttctcgaacgtgacgtggttccatgccattcacgtttcgggaacgaacgggacgaagaggttcgataaccctgttctaccgtttaacgacggggtgtacttcgcttcgacagagaagtccaacattattcgcggatggatattcggaaccactctcgattccaagactcagtccttgttgatagtgaacaacgccacgaacgtggtcattaaggtctgtgagtttcagttctgtaatgacccgttcttgggtgtttactatcacaagaacaacaagtcttggatggagagtgagttccgagtgtattcatccgcgaataattgtaccttcgagtatgtcagtcagccgtttctgatggatcttgaaggcaaacagggcaatttcaagaatttgcgcgagtttgtcttcaagaacatcgacggctacttcaagatatactcgaagcacacgccaatcaacctcgtccgtgatctcccgcagggcttcagcgctctggaaccgctggtggacttgccgataggcatcaacatcacgcggttccagacgctgttagccctgcacaggagttacctgaccccaggtgactcctcgtccggttggactgcaggtgccgccgcgtactacgtggggtacctgcagccccggacgttcttgttgaagtacaacgagaacgggacgatcacggacgcggttgattgtgcgttggaccctctgtcggagacgaagtgcaccctgaagtcgtttacggtagaaaaggggatctatcagacctccaacttccgcgtccagccgactgagagtatcgttcggtttccgaacatcacgaacctgtgtccgtttggagaggtcttcaacgcgaccaggttcgcctccgtgtacgcttggaacaggaagaggatatcgaattgtgtagcagactacagtgtgctatacaattcggcgtccttttccactttcaagtgttacggagtgtcgcccacgaagttgaacgacctctgcttcaccaacgtgtacgcggattccttcgtcatccgtggtgacgaggttcggcagatcgcgcccggacagactggaaagatagcggactacaattataagttgcccgacgactttactggctgcgttattgcttggaatagcaataacttagacagtaaagtcgggggcaactataattacctgtatcgactgtttcggaaaagcaatctgaagcccttcgagcgcgacattagcacggagatctaccaggctggtagtactccgtgcaatggcgtggagggcttcaattgctattttccgttacagtcgtacgggtttcagcccaccaacggggtagggtaccagccctaccgcgtggtggtgctgtcgttcgaactccttcacgcacccgcgactgtctgtgggcccaagaagtcgacgaacttggtgaagaacaagtgcgtcaacttcaacttcaatgggctcacaggcacgggggtgctgacggagtcgaacaaaaagttcctacctttccagcagttcgggcgcgatattgccgacaccacggatgccgtaagggatccgcagacgcttgagattctggacatcacgccctgcagcttcgggggcgtcagtgtaatcacgcctggtaccaacacgagcaaccaggttgccgtgttgtaccaggacgtgaattgcactgaggtccccgtagcgatccacgcggatcagctaaccccaacgtggagggtgtactcgacagggagtaatgtcttccagactcgcgctggttgtctgattggcgctgagcatgtgaacaactcgtacgagtgtgacatccccattggagcggggatctgcgcgtcgtaccagacccagacgaacagcccgaggcgtgcccgctcagtagcgtcgcagtcgatcatcgcgtacacgatgagcttgggggcggagaacagtgtagcctattcgaacaacagcattgctatccccacaaattttacaattagtgtaaccaccgagatcttaccggtctccatgaccaagacctcggtggattgcactatgtatatttgtggggatagcactgagtgttctaacctcctgctccagtacggcagtttctgtacgcagctcaaccgagcgcttacaggaattgccgtggagcaggacaagaacactcaggaggtgtttgcccaggtcaagcagatctacaagacacctccgatcaaggactttggcggcttcaacttctcccagatactccccgaccccagcaagcccagcaagcgtagctttattgaagatctgctcttcaataaagttacgcttgctgatgctgggttcatcaagcagtacggggattgtctgggagatatagccgccagagacttgatctgtgctcagaagttcaatgggctcactgttctcccccccttgctcacggacgagatgatcgcccagtatacttcggcgctgctggcgggcacgatcacctcgggctggacgtttggggctggtgcggcgctgcagatccccttcgccatgcagatggcgtaccgcttcaatgggatcggtgtcacacagaacgttttgtacgagaatcagaagctcatcgccaatcagttcaacagcgcgatcgggaagatacaggactccctgtcgagtacagcctccgcgttggggaagctgcaggacgtggtgaaccagaatgctcaagcgttgaacacgttggtgaagcagttgtcgtccaacttcggggcgataagttcggtgctgaacgatattctcagtcggctggacaaggtggaagcggaggtccagatagatcggctcatcactggtcgcctccagagtttgcagacgtacgtaactcagcagctcatccgagctgctgagatacgtgcgtctgcaaacctggcggcgaccaagatgagcgagtgcgtgctggggcagagcaagcgagtggacttctgcgggaagggctatcacctgatgtccttcccgcagagcgcacctcacggggtagtctttctccacgtgacatatgtgccggcgcaggagaagaacttcaccactgcgccggccatatgtcacgatgggaaagcccacttcccgcgtgaaggagtttttgtatcaaacgggacgcattggttcgtcacgcagcgcaacttctatgagccacagataattaccactgacaatacctttgtcagtggtaattgtgatgtggtcatagggatcgtgaacaacacggtctacgatcccctgcagcccgagctagatagtttcaaggaggagcttgataagtacttcaagaatcatacttccccagacgtggatcttggcgacattagcggcatcaacgctagtgtcgtcaacatccagaaggagatcgacaggctcaatgaggttgccaagaacctcaacgagagcctgatcgatctccaggagctggggaagtatgagcagtacatcaagtggccttggtacatctggctcgggttcattgcagggttgatcgcgatcgtgatggtcacgatcatgttgtgctgcatgacgagctgttgctcctgtttgaagggctgctgcagctgtggttcgtgttgtaagtttgacgaggatgactcggagccagtgttgaagggggtcaagttacactacacataatacgtattgccatgtgtatgtgggagacggtcgggtccagatattcgtatctgtcgagtagagtgtgggctcccacatactctgatgatccttcgggatcattcatggcaactcgagatagcataaaataacgccccaccttcttaacgggaggtggggcgttatttttactgaaagatatcatccaatggatctgtcgacggccgtcgttttacagccaagcttggctgttttggcggatgagagaagattttcagcctgatacagattaaatcagaacgcagaagcggtctgataaaacagaatttgcctggcggcagtagcgcggtggtcccacctgaccccatgccgaactcagaagtgaaacgccgtagcgccgatggtagtgtggggtctccccatgcgagagtagggaactgccaggcatcaaataaaacgaaaggctcagtcgaaagactgggcctttcgttttatctgttgtttgtcggtgaacgctctcctgagtaggacaaatccgccgggagcggatttgaacgttgcgaagcaacggcccggagggtggcgggcaggacgcccgccataaactgccaggcatcaaattaagcagaaggccatcctgacggatggcctttttgcgtttctacaaactcttttggtcgactctagagttccactgagcgtcagaccccgtagaaaagatcaaaggatcttcttgagatcctttttttctgcgcgtaatctgctgcttgcaaacaaaaaaaccaccgctaccagcggtggtttgtttgccggatcaagagctaccaactctttttccgaaggtaactggcttcagcagagcgcagataccaaatactgtccttctagtgtagccgtagttaggccaccacttcaagaactctgtagcaccgcctacatacctcgctctgctaatcctgttaccagtggctgctgccagtggcgataagtcgtgtcttaccgggttggactcaagacgatagttaccggataaggcgcagcggtcgggctgaacggggggttcgtgcacacagcccagcttggagcgaacgacctacaccgaactgagatacctacagcgtgagctatgagaaagcgccacgcttcccgaagggagaaaggcggacaggtatccggtaagcggcagggtcggaacaggagagcgcacgagggagcttccagggggaaacgcctggtatctttatagtcctgtcgggtttcgccacctctgacttgagcgtcgatttttgtgatgctcgtcaggggggcggagcctatggaaaaacgccagcaacgcggcctttttacggttcctggccttttgctggccttttgctcacatgttctttcctgcgttatcccctgattctgtggataaccgtattaccgcctttgagtgagctgataccgctcgccgcagccgaacgaccgagcgcagcgagtcagtgagcgaggaagcggaagatctagaagtactgctgactcataccaggcctgaatcgccccatcatccagccagaaagtgagggagccacggttgatgagagctttgttgtaggtggaccagttggtgattttgaacttttgctttgccacggaacggtctgcgttgtcgggaagatgcgtgatctgatccttcaactcagcaaaagttcgatttattcaacaaagccacgttgtgtctcaaaatctctgatgttacattgcacaagataaaaatatatcatcatgaacaataaaactgtctgcttacataaacagtaatacaaggggtgttatgagccatattcaacgggaaacgtcttgctcaaggccgcgattaaattccaacatggatgctgatttatatgggtataaatgggctcgcgataatgtcgggcaatcaggtgcgacaatctatcgattgtatgggaagcccgatgcgccagagttgtttctgaaacatggcaaaggtagcgttgccaatgatgttacagatgagatggtcagactaaactggctgacggaatttatgcctcttccgaccatcaagcattttatccgtactcctgatgatgcatggttactcaccactgcgatccccggaaaaacagcattccaggtattagaagaatatcctgattcaggtgaaaatattgttgatgcgctggcagtgttcctgcgccggttgcattcgattcctgtttgtaattgtccttttaacagcgatcgcgtatttcgtctcgctcaggcgcaatcacgaatgaataacggtttggttgatgcgagtgattttgatgacgagcgtaatggctggcctgttgaacaagtctggaaagaaatgcataagcttttgccattctcaccggattcagtcgtcactcatggtgatttctcacttgataaccttatttttgacgaggggaaattaataggttgtattgatgttggacgagtcggaatcgcagaccgataccaggatcttgccatcctatggaactgcctcggtgagttttctccttcattacagaaacggctttttcaaaaatatggtattgataatcctgatatgaataaattgcagtttcatttgatgctcgatgagtttttctaaggctagccccgggactagtgatctttgggagcagtccttgtgcgcttacgaggtgagccggtggggaaccgttatctgcctatggtgtgagcccccctagagagcttcaagagcaatcagcccgacctagaaaggaggccaagagagagacccctacggggggaaccgttttctgcctacgagatggcacatttactgggaagctttacggcgtcctcgtggaagttcaatgcccgcagacttaagtgctctattcacggtctgacgtgacacgctaaattcagacatagcttcattgattgtcggccacgagccagtctctccctcaacagtcataaaccaacctgcaatggtcaagcgattttctttagctttcctagcttgtcgttgactggacttagctagtttttctcgctgtgctcgggcgtactcactgtttgggtctttccagcgttctgcggcctttttaccgccacgtcttcccatagtggccagagcttttcgccctcggctgctctgcgtctctgtctgacgagcagggacgactggctggcctttagcgacgtagccgcgcacacgtcgcgccatcgtctggcggtcacgcatcggcggcagatcaggctcacggccgtctgctccgaccgcctgagcgacggtgtaggcacgctcgtaggcgtcgatgatcttggtgtcttttaggcgctcaccagccgcttttaactggtatcccacagtcaaagcgtggcgaaaagccgtctcatcacgggcggcacgccctggagcagtccagaggacacggacgccgtcgatcagctctccagacgcttcagcggcgctcggcaggcttgcttcaagcgtggcaagtgcttttgcttccgcagtggcttttcttgccgcttcgatacgtgcccgtccgctagaaaactcctgctcatagcgttttttaggtttttctgtgcctgagatcatgcgagcaacctccataagatcagctaggcgatccacgcgattgtgctgggcatgccagcggtacgcggtgggatcgtcggagacgtgcagtggccaccggctcagcctatgtgaaaaagcctggtcagcgccgaaaacgcgggtcatttcctcggtcgttgcagccagcaggcgcatattcgggctgctcatgcctgctgcggcatacaccggatcaatgagccagatgagctggcatttcccgctcagtggattcacgccgatccaagctggcgctttttccaggcgtgcccagcgctccaaaatcgcgtagacctcggggtttacgtgctcgattttcccgccggcctggtggctcggcacatcaatgtccaggacaagcacggctgcgtgctgcgcgtgcgtcagagcaacatactggcaccgggcaagcgattttgaaccaactcggtataacttcggctgtgtttctcccgtgtccgggtctttgatccaagcgctggcgaagtcgcgggtcttgctgccctggaaattttctctgcccaggtgagcgaggaattcgcggcggtcttcgctcgtccagccacgtgatcgcagcgcgagctcgggatgggtgtcgaacagatcagcggaaaatttccaggccggtgtgtcaatgtctcgtgaatccgctagagtcatttttgagcgctttctcccaggtttggactgggggttagccgacgccctgtgagttaccgctcacggggcgttcaacatttttcaggtattcgtgcagcttatcgcttcttgccgcctgtgcgctttttcgacgcgcgacgctgctgccgattcggtgcaggtggtggcggcgctgacacgtcctgggcggccacggccacacgaaacgcggcatttacgatgtttgtcatgcctgcgggcaccgcgccacgatcgcggataattctcgctgccgcttccagctctgtgacgaccatggccaaaatttcgctcgggggacgcacttccagcgccatttgcgacctagccgcctccagctcctcggcgtggcgtttgttggcgcgctcgcggctggctgcggcacgacacgcatctgagcaatattttgcgcgccgtcctcgcgggtcaggccggggaggaatcaggccaccgcagtaggcgcaactgattcgatcctccactactgtgcgtcctcctggcgctgccgagcacgcagctcgtcagccagctcctcaagatccgccacgagagtttctaggtcgctcgcggcactggcccagtctcgtgatgctggcgcgtccgtcgtatcgagagctcggaaaaatccgatcaccgtttttaaatcgacggcagcatcgagcgcgtcggactccagcgcgacatcagagagatccatagctgatgattcgggccaattttggtacttcgtcgtgaaggtcatgacaccattataacgaacgttcgttaaagtttttggcggaaaatcacgcggcacgaaaattttcacgaagcgggactttgcgcagctcaggggtgctaaaaattttgtatcgcacttgatttttccgaaagacagattatctgcaaacggtgtgtcgtatttctggcttggtttttaaaaaatctggaatcgaaaatttgcggggcga

SEQ ID NO: 29 - DNA, 720 bp, synthetic construct
  source 1..720: mol_type = other DNA
atggtcagcaagggggaggagctgttcaccggtgttgtgccgatcttggttgagcttgatggcgatgtgaacggccataagttcagcgtgagtggcgagggtgagggcgacgctacgtacgggaagcttaccctgaagtttatttgtactacagggaagcttcccgtaccgtggcccaccctcgtcaccacgctgacttatggcgttcagtgcttcagcaggtaccccgaccacatgaaacagcacgacttttttaagtcggccatgccggaggggtacgtgcaggagcgcaccatcttctttaaagacgatggcaactataagactcgagcggaagtcaaattcgagggggataccctcgtgaaccgcatcgagcttaagggcatcgactttaaagaagatggtaatatactcgggcacaagctcgagtataattataacagccataatgtatacattatggctgataaacaaaaaaacggcatcaaggtcaacttcaagattcggcacaacatcgaggacggctccgtccaacttgctgaccattatcagcagaacacgcccatcggagatgggcctgttctgctgcctgataatcactacttgtccacccagagtgccctgtcgaaggatccgaacgaaaagcgggaccacatggtcctgcttgagttcgtgaccgcggcagggatcactctgggtatggacgagttatataagtga

SEQ ID NO: 30 - DNA, 936 bp, synthetic construct
  source 1..936: mol_type = other DNA
atggcctccaaagtctacgatccggagcagaggaagcgcatgatcacgggcccacaatggtgggcccggtgcaagcagatgaacgttctcgacagcttcatcaactattacgatagtgagaagcatgccgagaacgctgtcatcttcttgcacgggaatgcagcgagcagctatctatggcggcacgtagtgccgcacatagaaccagttgctcgctgcattatcccggacttgataggcatgggcaagtcggggaagagtggcaacggctcgtacaggctgttagatcactacaagtatctgacagcctggttcgagctgttgaatcttcccaaaaaaatcatcttcgtcggacatgattggggcgcatgtcttgcttttcattatagctacgagcaccaggacaagatcaaagccatcgtccacgcggaaagcgtggtcgatgtgatcgagtcctgggacgagtggcctgatatagaggaagacatcgccctaatcaagtccgaggaaggtgaaaaaatggtcttggagaataattttttcgtcgagaccatgcttccctccaagatcatgcggaaactcgagcccgaggagtttgcggcgtacctcgagcccttcaaagagaagggcgaggtacgccgcccgactctctcgtggcctcgagaaattccgctggtcaagggagggaagcccgacgtcgtgcagatagtgcgtaattataacgcctatctgcgcgcgtcggacgacttgcccaaaatgtttatcgagtccgatcctggcttcttcagcaacgcgatcgtagagggggccaaaaaattcccgaacacggagttcgtgaaggtaaaaggtctccatttcagtcaggaggacgctcctgacgagatggggaagtacatcaagagcttcgtggaacgggtgctcaaaaatgagcaataa

SEQ ID NO: 31 - DNA, 961 bp, synthetic construct
  source 1..961: mol_type = other DNA
taatacgactcactatagggtaccacgtagaccgtacggcagtaataaccagctgaccgcatacccgagtaatggtcagcaagggggaggagctgttcaccggtgttgtgccgatcttggttgagcttgatggcgatgtgaacggccataagttcagcgtgagtggcgagggtgagggcgacgctacgtacgggaagcttaccctgaagtttatttgtactacagggaagcttcccgtaccgtggcccaccctcgtcaccacgctgacttatggcgttcagtgcttcagcaggtaccccgaccacatgaaacagcacgacttttttaagtcggccatgccggaggggtacgtgcaggagcgcaccatcttctttaaagacgatggcaactataagactcgagcggaagtcaaattcgagggggataccctcgtgaaccgcatcgagcttaagggcatcgactttaaagaagatggtaatatactcgggcacaagctcgagtataattataacagccataatgtatacattatggctgataaacaaaaaaacggcatcaaggtcaacttcaagattcggcacaacatcgaggacggctccgtccaacttgctgaccattatcagcagaacacgcccatcggagatgggcctgttctgctgcctgataatcactacttgtccacccagagtgccctgtcgaaggatccgaacgaaaagcgggaccacatggtcctgcttgagttcgtgaccgcggcagggatcactctgggtatggacgagttatataagtgatacgtattgccatgtgtatgtgggagacggtcgggtccagatattcgtatctgtcgagtagagtgtgggctcccacatactctgatgatccttcgggatcattcatggcaactcgagatagcataaaataacgccccaccttcttaacgggaggtggggcgttattttta

SEQ ID NO: 32 - DNA, 1177 bp, synthetic construct
  source 1..1177: mol_type = other DNA
taatacgactcactatagggtaccacgtagaccgtacggcagtaataaccagctgaccgcatacccgagtaatggcctccaaagtctacgatccggagcagaggaagcgcatgatcacgggcccacaatggtgggcccggtgcaagcagatgaacgttctcgacagcttcatcaactattacgatagtgagaagcatgccgagaacgctgtcatcttcttgcacgggaatgcagcgagcagctatctatggcggcacgtagtgccgcacatagaaccagttgctcgctgcattatcccggacttgataggcatgggcaagtcggggaagagtggcaacggctcgtacaggctgttagatcactacaagtatctgacagcctggttcgagctgttgaatcttcccaaaaaaatcatcttcgtcggacatgattggggcgcatgtcttgcttttcattatagctacgagcaccaggacaagatcaaagccatcgtccacgcggaaagcgtggtcgatgtgatcgagtcctgggacgagtggcctgatatagaggaagacatcgccctaatcaagtccgaggaaggtgaaaaaatggtcttggagaataattttttcgtcgagaccatgcttccctccaagatcatgcggaaactcgagcccgaggagtttgcggcgtacctcgagcccttcaaagagaagggcgaggtacgccgcccgactctctcgtggcctcgagaaattccgctggtcaagggagggaagcccgacgtcgtgcagatagtgcgtaattataacgcctatctgcgcgcgtcggacgacttgcccaaaatgtttatcgagtccgatcctggcttcttcagcaacgcgatcgtagagggggccaaaaaattcccgaacacggagttcgtgaaggtaaaaggtctccatttcagtcaggaggacgctcctgacgagatggggaagtacatcaagagcttcgtggaacgggtgctcaaaaatgagcaataatacgtattgccatgtgtatgtgggagacggtcgggtccagatattcgtatctgtcgagtagagtgtgggctcccacatactctgatgatccttcgggatcattcatggcaactcgagatagcataaaataacgccccaccttcttaacgggaggtggggcgttattttta

SEQ ID NO: 33 - DNA, 6014 bp, synthetic construct
  source 1..6014: mol_type = other DNA
ggatcctaatacgactcactatagggtaccacgtagaccgtacggcagtaataaccagctgaccgcatacccgagtaatggtcagcaagggggaggagctgttcaccggtgttgtgccgatcttggttgagcttgatggcgatgtgaacggccataagttcagcgtgagtggcgagggtgagggcgacgctacgtacgggaagcttaccctgaagtttatttgtactacagggaagcttcccgtaccgtggcccaccctcgtcaccacgctgacttatggcgttcagtgcttcagcaggtaccccgaccacatgaaacagcacgacttttttaagtcggccatgccggaggggtacgtgcaggagcgcaccatcttctttaaagacgatggcaactataagactcgagcggaagtcaaattcgagggggataccctcgtgaaccgcatcgagcttaagggcatcgactttaaagaagatggtaatatactcgggcacaagctcgagtataattataacagccataatgtatacattatggctgataaacaaaaaaacggcatcaaggtcaacttcaagattcggcacaacatcgaggacggctccgtccaacttgctgaccattatcagcagaacacgcccatcggagatgggcctgttctgctgcctgataatcactacttgtccacccagagtgccctgtcgaaggatccgaacgaaaagcgggaccacatggtcctgcttgagttcgtgaccgcggcagggatcactctgggtatggacgagttatataagtgatacgtattgccatgtgtatgtgggagacggtcgggtccagatattcgtatctgtcgagtagagtgtgggctcccacatactctgatgatccttcgggatcattcatggcaactcgagatagcataaaataacgccccaccttcttaacgggaggtggggcgttatttttactgaaagatatctgtcgacggccgtcgttttacagccaagcttggctgttttggcggatgagagaagattttcagcctgatacagattaaatcagaacgcagaagcggtctgataaaacagaatttgcctggcggcagtagcgcggtggtcccacctgaccccatgccgaactcagaagtgaaacgccgtagcgccgatggtagtgtggggtctccccatgcgagagtagggaactgccaggcatcaaataaaacgaaaggctcagtcgaaagactgggcctttcgttttatctgttgtttgtcggtgaacgctctcctgagtaggacaaatccgccgggagcggatttgaacgttgcgaagcaacggcccggagggtggcgggcaggacgcccgccataaactgccaggcatcaaattaagcagaaggccatcctgacggatggcctttttgcgtttctacaaactcttttggtcgactctagagttccactgagcgtcagaccccgtagaaaagatcaaaggatcttcttgagatcctttttttctgcgcgtaatctgctgcttgcaaacaaaaaaaccaccgctaccagcggtggtttgtttgccggatcaagagctaccaactctttttccgaaggtaactggcttcagcagagcgcagataccaaatactgttcttctagtgtagccgtagttaggccaccacttcaagaactctgtagcaccgcctacatacctcgctctgctaatcctgttaccagtggctgctgccagtggcgataagtcgtgtcttaccgggttggactcaagacgatagttaccggataaggcgcagcggtcgggctgaacggggggttcgtgcacacagcccagcttggagcgaacgacctacaccgaactgagatacctacagcgtgagctatgagaaagcgccacgcttcccgaagggagaaaggcggacaggtatccggtaagcggcagggtcggaacaggagagcgcacgagggagcttccagggggaaacgcctggtatctttatagtcctgtcgggtttcgccacctctgacttgagcgtcgatttttgtgatgctcgtcaggggggcggagcctatggaaaaacgccagcaacgcggcctttttacggttcctggccttttgctggccttttgctcacatgttctttcctgcgttatcccctgattctgtggataaccgtattaccgcctttgagtgagctgataccgctcgccgcagccgaacgaccgagcgcagcgagtcagtgagcgaggaagcggaagatctagaagtactgctgactcataccaggcctgaatcgccccatcatccagccagaaagtgagggagccacggttgatgagagctttgttgtaggtggaccagttggtgattttgaacttttgctttgccacggaacggtctgcgttgtcgggaagatgcgtgatctgatccttcaactcagcaaaagttcgatttattcaacaaagccacgttgtgtctcaaaatctctgatgttacattgcacaagataaaaatatatcatcatgaacaataaaactgtctgcttacataaacagtaatacaaggggtgttatgagccatattcaacgggaaacgtcttgctcaaggccgcgattaaattccaacatggatgctgatttatatgggtataaatgggctcgcgataatgtcgggcaatcaggtgcgacaatctatcgattgtatgggaagcccgatgcgccagagttgtttctgaaacatggcaaaggtagcgttgccaatgatgttacagatgagatggtcagactaaactggctgacggaatttatgcctcttccgaccatcaagcattttatccgtactcctgatgatgcatggttactcaccactgcgatccccggaaaaacagcattccaggtattagaagaatatcctgattcaggtgaaaatattgttgatgcgctggcagtgttcctgcgccggttgcattcgattcctgtttgtaattgtccttttaacagcgatcgcgtatttcgtctcgctcaggcgcaatcacgaatgaataacggtttggttgatgcgagtgattttgatgacgagcgtaatggctggcctgttgaacaagtctggaaagaaatgcataagcttttgccattctcaccggattcagtcgtcactcatggtgatttctcacttgataaccttatttttgacgaggggaaattaataggttgtattgatgttggacgagtcggaatcgcagaccgataccaggatcttgccatcctatggaactgcctcggtgagttttctccttcattacagaaacggctttttcaaaaatatggtattgataatcctgatatgaataaattgcagtttcatttgatgctcgatgagtttttctaaggctagccccgggactagtgatctttgggagcagtccttgtgcgcttacgaggtgagccggtggggaaccgttatctgcctatggtgtgagcccccctagagagcttcaagagcaatcagcccgacctagaaaggaggccaagagagagacccctacggggggaaccgttttctgcctacgagatggcacatttactgggaagctttacggcgtcctcgtggaagttcaatgcccgcagacttaagtgctctattcacggtctgacgtgacacgctaaattcagacatagcttcattgattgtcggccacgagccagtctctccctcaacagtcataaaccaacctgcaatggtcaagcgattttctttagctttcctagcttgtcgttgactggacttagctagtttttctcgctgtgctcgggcgtactcactgtttgggtctttccagcgttctgcggcctttttaccgccacgtcttcccatagtggccagagcttttcgccctcggctgctctgcgtctctgtctgacgagcagggacgactggctggcctttagcgacgtagccgcgcacacgtcgcgccatcgtctggcggtcacgcatcggcggcagatcaggctcacggccgtctgctccgaccgcctgagcgacggtgtaggcacgctcgtaggcgtcgatgatcttggtgtcttttaggcgctcaccagccgcttttaactggtatcccacagtcaaagcgtggcgaaaagccgtctcatcacgggcggcacgccctggagcagtccagaggacacggacgccgtcgatcagctctccagacgcttcagcggcgctcggcaggcttgcttcaagcgtggcaagtgcttttgcttccgcagtggcttttcttgccgcttcgatacgtgcccgtccgctagaaaactcctgctcatagcgttttttaggtttttctgtgcctgagatcatgcgagcaacctccataagatcagctaggcgatccacgcgattgtgctgggcatgccagcggtacgcggtgggatcgtcggagacgtgcagtggccaccggctcagcctatgtgaaaaagcctggtcagcgccgaaaacgcgggtcatttcctcggtcgttgcagccagcaggcgcatattcgggctgctcatgcctgctgcggcatacaccggatcaatgagccagatgagctggcatttcccgctcagtggattcacgccgatccaagctggcgctttttccaggcgtgcccagcgctccaaaatcgcgtagacctcggggtttacgtgctcgattttcccgccggcctggtggctcggcacatcaatgtccaggacaagcacggctgcgtgctgcgcgtgcgtcagagcaacatactggcaccgggcaagcgattttgaaccaactcggtataacttcggctgtgtttctcccgtgtccgggtctttgatccaagcgctggcgaagtcgcgggtcttgctgccctggaaattttctctgcccaggtgagcgaggaattcgcggcggtcttcgctcgtccagccacgtgatcgcagcgcgagctcgggatgggtgtcgaacagatcagcggaaaatttccaggccggtgtgtcaatgtctcgtgaatccgctagagtcatttttgagcgctttctcccaggtttggactgggggttagccgacgccctgtgagttaccgctcacggggcgttcaacatttttcaggtattcgtgcagcttatcgcttcttgccgcctgtgcgctttttcgacgcgcgacgctgctgccgattcggtgcaggtggtggcggcgctgacacgtcctgggcggccacggccacacgaaacgcggcatttacgatgtttgtcatgcctgcgggcaccgcgccacgatcgcggataattctcgctgccgcttccagctctgtgacgaccatggccaaaatttcgctcgggggacgcacttccagcgccatttgcgacctagccgcctccagctcctcggcgtggcgtttgttggcgcgctcgcggctggctgcggcacgacacgcatctgagcaatattttgcgcgccgtcctcgcgggtcaggccggggaggaatcaggccaccgcagtaggcgcaactgattcgatcctccactactgtgcgtcctcctggcgctgccgagcacgcagctcgtcagccagctcctcaagatccgccacgagagtttctaggtcgctcgcggcactggcccagtctcgtgatgctggcgcgtccgtcgtatcgagagctcggaaaaatccgatcaccgtttttaaatcgacggcagcatcgagcgcgtcggactccagcgcgacatcagagagatccatagctgatgattcgggccaattttggtacttcgtcgtgaaggtcatgacaccattataacgaacgttcgttaaagtttttggcggaaaatcacgcggcacgaaaattttcacgaagcgggactttgcgcagctcaggggtgctaaaaattttgtatcgcacttgatttttccgaaagacagattatctgcaaacggtgtgtcgtatttctggcttggtttttaaaaaatctggaatcgaaaatttgcggggcga

SEQ ID NO: 34 - DNA, 6230 bp, synthetic construct
  source 1..6230: mol_type = other DNA
ggatcctaatacgactcactatagggtaccacgtagaccgtacggcagtaataaccagctgaccgcatacccgagtaatggcctccaaagtctacgatccggagcagaggaagcgcatgatcacgggcccacaatggtgggcccggtgcaagcagatgaacgttctcgacagcttcatcaactattacgatagtgagaagcatgccgagaacgctgtcatcttcttgcacgggaatgcagcgagcagctatctatggcggcacgtagtgccgcacatagaaccagttgctcgctgcattatcccggacttgataggcatgggcaagtcggggaagagtggcaacggctcgtacaggctgttagatcactacaagtatctgacagcctggttcgagctgttgaatcttcccaaaaaaatcatcttcgtcggacatgattggggcgcatgtcttgcttttcattatagctacgagcaccaggacaagatcaaagccatcgtccacgcggaaagcgtggtcgatgtgatcgagtcctgggacgagtggcctgatatagaggaagacatcgccctaatcaagtccgaggaaggtgaaaaaatggtcttggagaataattttttcgtcgagaccatgcttccctccaagatcatgcggaaactcgagcccgaggagtttgcggcgtacctcgagcccttcaaagagaagggcgaggtacgccgcccgactctctcgtggcctcgagaaattccgctggtcaagggagggaagcccgacgtcgtgcagatagtgcgtaattataacgcctatctgcgcgcgtcggacgacttgcccaaaatgtttatcgagtccgatcctggcttcttcagcaacgcgatcgtagagggggccaaaaaattcccgaacacggagttcgtgaaggtaaaaggtctccatttcagtcaggaggacgctcctgacgagatggggaagtacatcaagagcttcgtggaacgggtgctcaaaaatgagcaataatacgtattgccatgtgtatgtgggagacggtcgggtccagatattcgtatctgtcgagtagagtgtgggctcccacatactctgatgatccttcgggatcattcatggcaactcgagatagcataaaataacgccccaccttcttaacgggaggtggggcgttatttttactgaaagatatctgtcgacggccgtcgttttacagccaagcttggctgttttggcggatgagagaagattttcagcctgatacagattaaatcagaacgcagaagcggtctgataaaacagaatttgcctggcggcagtagcgcggtggtcccacctgaccccatgccgaactcagaagtgaaacgccgtagcgccgatggtagtgtggggtctccccatgcgagagtagggaactgccaggcatcaaataaaacgaaaggctcagtcgaaagactgggcctttcgttttatctgttgtttgtcggtgaacgctctcctgagtaggacaaatccgccgggagcggatttgaacgttgcgaagcaacggcccggagggtggcgggcaggacgcccgccataaactgccaggcatcaaattaagcagaaggccatcctgacggatggcctttttgcgtttctacaaactcttttggtcgactctagagttccactgagcgtcagaccccgtagaaaagatcaaaggatcttcttgagatcctttttttctgcgcgtaatctgctgcttgcaaacaaaaaaaccaccgctaccagcggtggtttgtttgccggatcaagagctaccaactctttttccgaaggtaactggcttcagcagagcgcagataccaaatactgttcttctagtgtagccgtagttaggccaccacttcaagaactctgtagcaccgcctacatacctcgctctgctaatcctgttaccagtggctgctgccagtggcgataagtcgtgtcttaccgggttggactcaagacgatagttaccggataaggcgcagcggtcgggctgaacggggggttcgtgcacacagcccagcttggagcgaacgacctacaccgaactgagatacctacagcgtgagctatgagaaagcgccacgcttcccgaagggagaaaggcggacaggtatccggtaagcggcagggtcggaacaggagagcgcacgagggagcttccagggggaaacgcctggtatctttatagtcctgtcgggtttcgccacctctgacttgagcgtcgatttttgtgatgctcgtcaggggggcggagcctatggaaaaacgccagcaacgcggcctttttacggttcctggccttttgctggccttttgctcacatgttctttcctgcgttatcccctgattctgtggataaccgtattaccgcctttgagtgagctgataccgctcgccgcagccgaacgaccgagcgcagcgagtcagtgagcgaggaagcggaagatctagaagtactgctgactcataccaggcctgaatcgccccatcatccagccagaaagtgagggagccacggttgatgagagctttgttgtaggtggaccagttggtgattttgaacttttgctttgccacggaacggtctgcgttgtcgggaagatgcgtgatctgatccttcaactcagcaaaagttcgatttattcaacaaagccacgttgtgtctcaaaatctctgatgttacattgcacaagataaaaatatatcatcatgaacaataaaactgtctgcttacataaacagtaatacaaggggtgttatgagccatattcaacgggaaacgtcttgctcaaggccgcgattaaattccaacatggatgctgatttatatgggtataaatgggctcgcgataatgtcgggcaatcaggtgcgacaatctatcgattgtatgggaagcccgatgcgccagagttgtttctgaaacatggcaaaggtagcgttgccaatgatgttacagatgagatggtcagactaaactggctgacggaatttatgcctcttccgaccatcaagcattttatccgtactcctgatgatgcatggttactcaccactgcgatccccggaaaaacagcattccaggtattagaagaatatcctgattcaggtgaaaatattgttgatgcgctggcagtgttcctgcgccggttgcattcgattcctgtttgtaattgtccttttaacagcgatcgcgtatttcgtctcgctcaggcgcaatcacgaatgaataacggtttggttgatgcgagtgattttgatgacgagcgtaatggctggcctgttgaacaagtctggaaagaaatgcataagcttttgccattctcaccggattcagtcgtcactcatggtgatttctcacttgataaccttatttttgacgaggggaaattaataggttgtattgatgttggacgagtcggaatcgcagaccgataccaggatcttgccatcctatggaactgcctcggtgagttttctccttcattacagaaacggctttttcaaaaatatggtattgataatcctgatatgaataaattgcagtttcatttgatgctcgatgagtttttctaaggctagccccgggactagtgatctttgggagcagtccttgtgcgcttacgaggtgagccggtggggaaccgttatctgcctatggtgtgagcccccctagagagcttcaagagcaatcagcccgacctagaaaggaggccaagagagagacccctacggggggaaccgttttctgcctacgagatggcacatttactgggaagctttacggcgtcctcgtggaagttcaatgcccgcagacttaagtgctctattcacggtctgacgtgacacgctaaattcagacatagcttcattgattgtcggccacgagccagtctctccctcaacagtcataaaccaacctgcaatggtcaagcgattttctttagctttcctagcttgtcgttgactggacttagctagtttttctcgctgtgctcgggcgtactcactgtttgggtctttccagcgttctgcggcctttttaccgccacgtcttcccatagtggccagagcttttcgccctcggctgctctgcgtctctgtctgacgagcagggacgactggctggcctttagcgacgtagccgcgcacacgtcgcgccatcgtctggcggtcacgcatcggcggcagatcaggctcacggccgtctgctccgaccgcctgagcgacggtgtaggcacgctcgtaggcgtcgatgatcttggtgtcttttaggcgctcaccagccgcttttaactggtatcccacagtcaaagcgtggcgaaaagccgtctcatcacgggcggcacgccctggagcagtccagaggacacggacgccgtcgatcagctctccagacgcttcagcggcgctcggcaggcttgcttcaagcgtggcaagtgcttttgcttccgcagtggcttttcttgccgcttcgatacgtgcccgtccgctagaaaactcctgctcatagcgttttttaggtttttctgtgcctgagatcatgcgagcaacctccataagatcagctaggcgatccacgcgattgtgctgggcatgccagcggtacgcggtgggatcgtcggagacgtgcagtggccaccggctcagcctatgtgaaaaagcctggtcagcgccgaaaacgcgggtcatttcctcggtcgttgcagccagcaggcgcatattcgggctgctcatgcctgctgcggcatacaccggatcaatgagccagatgagctggcatttcccgctcagtggattcacgccgatccaagctggcgctttttccaggcgtgcccagcgctccaaaatcgcgtagacctcggggtttacgtgctcgattttcccgccggcctggtggctcggcacatcaatgtccaggacaagcacggctgcgtgctgcgcgtgcgtcagagcaacatactggcaccgggcaagcgattttgaaccaactcggtataacttcggctgtgtttctcccgtgtccgggtctttgatccaagcgctggcgaagtcgcgggtcttgctgccctggaaattttctctgcccaggtgagcgaggaattcgcggcggtcttcgctcgtccagccacgtgatcgcagcgcgagctcgggatgggtgtcgaacagatcagcggaaaatttccaggccggtgtgtcaatgtctcgtgaatccgctagagtcatttttgagcgctttctcccaggtttggactgggggttagccgacgccctgtgagttaccgctcacggggcgttcaacatttttcaggtattcgtgcagcttatcgcttcttgccgcctgtgcgctttttcgacgcgcgacgctgctgccgattcggtgcaggtggtggcggcgctgacacgtcctgggcggccacggccacacgaaacgcggcatttacgatgtttgtcatgcctgcgggcaccgcgccacgatcgcggataattctcgctgccgcttccagctctgtgacgaccatggccaaaatttcgctcgggggacgcacttccagcgccatttgcgacctagccgcctccagctcctcggcgtggcgtttgttggcgcgctcgcggctggctgcggcacgacacgcatctgagcaatattttgcgcgccgtcctcgcgggtcaggccggggaggaatcaggccaccgcagtaggcgcaactgattcgatcctccactactgtgcgtcctcctggcgctgccgagcacgcagctcgtcagccagctcctcaagatccgccacgagagtttctaggtcgctcgcggcactggcccagtctcgtgatgctggcgcgtccgtcgtatcgagagctcggaaaaatccgatcaccgtttttaaatcgacggcagcatcgagcgcgtcggactccagcgcgacatcagagagatccatagctgatgattcgggccaattttggtacttcgtcgtgaaggtcatgacaccattataacgaacgttcgttaaagtttttggcggaaaatcacgcggcacgaaaattttcacgaagcgggactttgcgcagctcaggggtgctaaaaattttgtatcgcacttgatttttccgaaagacagattatctgcaaacggtgtgtcgtatttctggcttggtttttaaaaaatctggaatcgaaaatttgcggggcga

SEQ ID NO: 35 - DNA, 720 bp, synthetic construct; identical to SEQ ID NO: 2
  source 1..720: mol_type = other DNA

SEQ ID NO: 36 - DNA, 1247 bp, synthetic construct
  source 1..1247: mol_type = other DNA
gatcagcgacgccgcagggggctggaagaaaaacttggcgatgaaccgaatgcacttttaaggaaaaagcaggctcgtcaagcagctcgcgctgtgctgcccaacgctacagagtccagaatcgtggtgtctggaaacttccgcacctggaggcatttcattggcatgcgagccagtgaacatgcagacgtcgaaatccgcgaagtagcggtagaatgtttaagaaagctgcaggtagcagcgccaactgttttcggtgattttgagattgaaactttggcagacggatcgcaaatggcaacaagcccgtatgtcatggacttttaacgcaaagctcacacccacgagctaaaaattcatatagttaagacaacatttttggctgtaaaagacagccgtaaaaacctcttgctcgtgtcaattgttcttatcggaatgtggcttgggcgattgttatgcaaaagttgttaggttttttgcggggttgtttaacccccaaatgagggaagatggtaaccttgaactctatggtgagcaagggcgaggagctgttcaccggggtggtgcccatcctggtcgagctggacggcgacgtaaacggccacaagttcagcgtgtccggcgagggcgagggcgatgccacctacggcaagctgaccctgaagttcatctgcaccaccggcaagctgcccgtgccctggcccaccctcgtgaccaccctgacctacggcgtgcagtgcttcagccgctaccccgaccacatgaagcagcacgacttcttcaagtccgccatgcccgaaggctacgtccaggagcgcaccatcttcttcaaggacgacggcaactacaagacccgcgccgaggtgaagttcgagggcgacaccctggtgaaccgcatcgagctgaagggcatcgacttcaaggaggacggcaacatcctggggcacaagctggagtacaactacaacagccacaacgtctatatcatggccgacaagcagaagaacggcatcaaggtgaacttcaagatccgccacaacatcgaggacggcagcgtgcagctcgccgaccactaccagcagaacacccccatcggcgacggccccgtgctgctgcccgacaaccactacctgagcacccagtccgccctgagcaaagaccccaacgagaagcgcgatcacatggtcctgctggagttcgtgaccgccgccgggatcactctcggcatggacgagctgtacaagtaa

SEQ ID NO: 37 - DNA, 1247 bp, synthetic construct
  source 1..1247: mol_type = other DNA
gatcagcgacgccgcagggggctggaagaaaaacttggcgatgaaccgaatgcacttttaaggaaaaagcaggctcgtcaagcagctcgcgctgtgctgcccaacgctacagagtccagaatcgtggtgtctggaaacttccgcacctggaggcatttcattggcatgcgagccagtgaacatgcagacgtcgaaatccgcgaagtagcggtagaatgtttaagaaagctgcaggtagcagcgccaactgttttcggtgattttgagattgaaactttggcagacggatcgcaaatggcaacaagcccgtatgtcatggacttttaacgcaaagctcacacccacgagctaaaaattcatatagttaagacaacatttttggctgtaaaagacagccgtaaaaacctcttgctcgtgtcaattgttcttatcggaatgtggcttgggcgattgttatgcaaaagttgttaggttttttgcggggttgtttaacccccaaatgagggaagatggtaaccttgaactctatggtcagcaagggtgaggagctattcaccggagtagttcccatccttgttgagctggacggggacgtgaacgggcacaagttctccgtgagtggggagggcgagggtgacgccacgtacgggaagcttaccctgaagttcatctgtactacagggaagcttcccgtaccgtggcccaccctcgtcactaccctcacttacggagtgcagtgcttttcacgttaccccgaccacatgaagcagcatgacttcttcaagtcggccatgcctgaaggatacgtccaggagcggacgatattcttcaaagacgatgggaattataagacccgtgccgaggttaagttcgagggtgataccctcgtcaatagaatcgagctgaagggcatcgattttaaggaggacggtaacatcctcggacataagctcgagtacaattataattcccataacgtctacataatggccgacaagcagaagaatggtatcaaggtgaacttcaagatccggcacaacatcgaagatgggagtgttcagcttgctgatcactatcagcaaaacactcccatcggcgatgggccggtcttgttacctgataaccattacttgtccacccagagtgccctgtcgaaggatccgaacgaaaagcgggaccacatggtcctgcttgagttcgtgaccgcggcagggatcactctgggtatggacgagttatataagtaa

SEQ ID NO: 38 - DNA, 5794 bp, synthetic construct
  source 1..5794: mol_type = other DNA
ggatccctcgagctgcaggatatccatatggtgagcaagggcgaggagctgttcaccggggtggtgcccatcctggtcgagctggacggcgacgtaaacggccacaagttcagcgtgtccggcgagggcgagggcgatgccacctacggcaagctgaccctgaagctgatctgcaccaccggcaagctgcccgtgccctggcccaccctcgtgaccaccctgggctacggcctgcagtgcttcgcccgctaccccgaccacatgaagcagcacgacttcttcaagtccgccatgcccgaaggctacgtccaggagcgcaccatcttcttcaaggacgacggcaactacaagacccgcgccgaggtgaagttcgagggcgacaccctggtgaaccgcatcgagctgaagggcatcgacttcaaggaggacggcaacatcctggggcacaagctggagtacaactacaacagccacaacgtctatatcaccgccgacaagcagaagaacggcatcaaggccaacttcaagatccgccacaacatcgaggacggcggcgtgcagctcgccgaccactaccagcagaacacccccatcggcgacggccccgtgctgctgcccgacaaccactacctgagctaccagtccgccctgagcaaagaccccaacgagaagcgcgatcacatggtcctgctggagttcgtgaccgccgccgggatcactctcggcatggacgagctgtacaagtaacatatggatatctgtcgacggccgtcgttttacagccaagcttggctgttttggcggatgagagaagattttcagcctgatacagattaaatcagaacgcagaagcggtctgataaaacagaatttgcctggcggcagtagcgcggtggtcccacctgaccccatgccgaactcagaagtgaaacgccgtagcgccgatggtagtgtggggtctccccatgcgagagtagggaactgccaggcatcaaataaaacgaaaggctcagtcgaaagactgggcctttcgttttatctgttgtttgtcggtgaacgctctcctgagtaggacaaatccgccgggagcggatttgaacgttgcgaagcaacggcccggagggtggcgggcaggacgcccgccataaactgccaggcatcaaattaagcagaaggccatcctgacggatggcctttttgcgtttctacaaactcttttggtcgactctagagttccactgagcgtcagaccccgtagaaaagatcaaaggatcttcttgagatcctttttttctgcgcgtaatctgctgcttgcaaacaaaaaaaccaccgctaccagcggtggtttgtttgccggatcaagagctaccaactctttttccgaaggtaactggcttcagcagagcgcagataccaaatactgtccttctagtgtagccgtagttaggccaccacttcaagaactctgtagcaccgcctacatacctcgctctgctaatcctgttaccagtggctgctgccagtggcgataagtcgtgtcttaccgggttggactcaagacgatagttaccggataaggcgcagcggtcgggctgaacggggggttcgtgcacacagcccagcttggagcgaacgacctacaccgaactgagatacctacagcgtgagctatgagaaagcgccacgcttcccgaagggagaaaggcggacaggtatccggtaagcggcagggtcggaacaggagagcgcacgagggagcttccagggggaaacgcctggtatctttatagtcctgtcgggtttcgccacctctgacttgagcgtcgatttttgtgatgctcgtcaggggggcggagcctatggaaaaacgccagcaacgcggcctttttacggttcctggccttttgctggccttttgctcacatgttctttcctgcgttatcccctgattctgtggataaccgtattaccgcctttgagtgagctgataccgctcgccgcagccgaacgaccgagcgcagcgagtcagtgagcgaggaagcggaagatctagaagtactgctgactcataccaggcctgaatcgccccatcatccagccagaaagtgagggagccacggttgatgagagctttgttgtaggtggaccagttggtgattttgaacttttgctttgccacggaacggtctgcgttgtcgggaagatgcgtgatctgatccttcaactcagcaaaagttcgatttattcaacaaagccacgttgtgtctcaaaatctctgatgttacattgcacaagataaaaatatatcatcatgaacaataaaactgtctgcttacataaacagtaatacaaggggtgttatgagccatattcaacgggaaacgtcttgctcaaggccgcgattaaattccaacatggatgctgatttatatgggtataaatgggctcgcgataatgtcgggcaatcaggtgcgacaatctatcgattgtatgggaagcccgatgcgccagagttgtttctgaaacatggcaaaggtagcgttgccaatgatgttacagatgagatggtcagactaaactggctgacggaatttatgcctcttccgaccatcaagcattttatccgtactcctgatgatgcatggttactcaccactgcgatccccggaaaaacagcattccaggtattagaagaatatcctgattcaggtgaaaatattgttgatgcgctggcagtgttcctgcgccggttgcattcgattcctgtttgtaattgtccttttaacagcgatcgcgtatttcgtctcgctcaggcgcaatcacgaatgaataacggtttggttgatgcgagtgattttgatgacgagcgtaatggctggcctgttgaacaagtctggaaagaaatgcataagcttttgccattctcaccggattcagtcgtcactcatggtgatttctcacttgataaccttatttttgacgaggggaaattaataggttgtattgatgttggacgagtcggaatcgcagaccgataccaggatcttgccatcctatggaactgcctcggtgagttttctccttcattacagaaacggctttttcaaaaatatggtattgataatcctgatatgaataaattgcagtttcatttgatgctcgatgagtttttctaaggctagccccgggactagtgatctttgggagcagtccttgtgcgcttacgaggtgagccggtggggaaccgttatctgcctatggtgtgagcccccctagagagcttcaagagcaatcagcccgacctagaaaggaggccaagagagagacccctacggggggaaccgttttctgcctacgagatggcacatttactgggaagctttacggcgtcctcgtggaagttcaatgcccgcagacttaagtgctctattcacggtctgacgtgacacgctaaattcagacatagcttcattgattgtcggccacgagccagtctctccctcaacagtcataaaccaacctgcaatggtcaagcgatttcctttagctttcctagcttgtcgttgactggacttagctagtttttctcgctgtgctcgggcgtactcactgtttgggtctttccagcgttctgcggcctttttaccgccacgtcttcccatagtggccagagcttttcgccctcggctgctctgcgtctctgtctgacgagcagggacgactggctggcctttagcgacgtagccgcgcacacgtcgcgccatcgtctggcggtcacgcatcggcggcagatcaggctcacggccgtctgctccgaccgcctgagcgacggtgtaggcacgctcgtaggcgtcgatgatcttggtgtcttttaggcgctcaccagccgcttttaactggtatcccacagtcaaagcgtggcgaaaagccgtctcatcacgggcggcacgccctggagcagtccagaggacacggacgccgtcgatcagctctccagacgcttcagcggcgctcggcaggcttgcttcaagcgtggcaagtgcttttgcttccgcagtggcttttcttgccgcttcgatacgtgcccgtccgctagaaaactcctgctcatagcgttttttaggtttttctgtgcctgagatcatgcgagcaacctccataagatcagctaggcgatccacgcgattgtgctgggcatgccagcggtacgcggtgggatcgtcggagacgtgcagtggccaccggctcagcctatgtgaaaaagcctggtcagcgccgaaaacgcgggtcatttcctcggtcgttgcagccagcaggcgcatattcgggctgctcatgcctgctgcggcatacaccggatcaatgagccagatgagctggcatttcccgctcagtggattcacgccgatccaagctggcgctttttccaggcgtgcccagcgctccaaaatcgcgtagacctcggggtttacgtgctcgattttcccgccggcctggtggctcggcacatcaatgtccaggacaagcacggctgcgtgctgcgcgtgcgtcagagcaacatactggcaccgggcaagcgattttgaaccaactcggtataacttcggctgtgtttctcccgtgtccgggtctttgatccaagcgctggcgaagtcgcgggtcttgctgccctggaaattttctctgcccaggtgagcgaggaattcgcggcggtcttcgctcgtccagccacgtgatcgcagcgcgagctcgggatgggtgtcgaacagatcagcggaaaatttccaggccggtgtgtcaatgtctcgtgaatccgctagagtcatttttgagcgctttctcccaggtttggactgggggttagccgacgccctgtgagttaccgctcacggggcgttcaacatttttcaggtattcgtgcagcttatcgcttcttgccgcctgtgcgctttttcgacgcgcgacgctgctgccgattcggtgcaggtggtggcggcgctgacacgtcctgggcggccacggccacacgaaacgcggcatttacgatgtttgtcatgcctgcgggcaccgcgccacgatcgcggataattctcgctgccgcttccagctctgtgacgaccatggccaaaatttcgctcgggggacgcacttccagcgccatttgcgacctagccgcctccagctcctcggcgtggcgtttgttggcgcgctcgcggctggctgcggcacgacacgcatctgagcaatattttgcgcgccgtcctcgcgggtcaggccggggaggaatcaggccaccgcagtaggcgcaactgattcgatcctccactactgtgcgtcctcctggcgctgccgagcacgcagctcgtcagccagctcctcaagatccgccacgagagtttctaggtcgctcgcggcactggcccagtctcgtgatgctggcgcgtccgtcgtatcgagagctcggaaaaatccgatcaccgtttttaaatcgacggcagcatcgagcgcgtcggactccagcgcgacatcagagagatccatagctgatgattcgggccaattttggtacttcgtcgtgaaggtcatgacaccattataacgaacgttcgttaaagtttttggcggaaaatcacgcggcacgaaaattttcacgaagcgggactttgcgcagctcaggggtgctaaaaattttgtatcgcacttgatttttccgaaagacagattatctgcaaacggtgtgtcgtatttctggcttggtttttaaaaaatctggaatcgaaaatttgcggggcga

SEQ ID NO: 39 - DNA, 6292 bp, synthetic construct
  source 1..6292: mol_type = other DNA
gcgatcagcgacgccgcagggggctggaagaaaaacttggcgatgaaccgaatgcacttttaaggaaaaagcaggctcgtcaagcagctcgcgctgtgctgcccaacgctacagagtccagaatcgtggtgtctggaaacttccgcacctggaggcatttcattggcatgcgagccagtgaacatgcagacgtcgaaatccgcgaagtagcggtagaatgtttaagaaagctgcaggtagcagcgccaactgttttcggtgattttgagattgaaactttggcagacggatcgcaaatggcaacaagcccgtatgtcatggacttttaacgcaaagctcacacccacgagctaaaaattcatatagttaagacaacatttttggctgtaaaagacagccgtaaaaacctcttgctcgtgtcaattgttcttatcggaatgtggcttgggcgattgttatgcaaaagttgttaggttttttgcggggttgtttaacccccaaatgagggaagatggtaaccttgaactctatggtgagcaagggcgaggagctgttcaccggggtggtgcccatcctggtcgagctggacggcgacgtaaacggccacaagttcagcgtgtccggcgagggcgagggcgatgccacctacggcaagctgaccctgaagttcatctgcaccaccggcaagctgcccgtgccctggcccaccctcgtgaccaccctgacctacggcgtgcagtgcttcagccgctaccccgaccacatgaagcagcacgacttcttcaagtccgccatgcccgaaggctacgtccaggagcgcaccatcttcttcaaggacgacggcaactacaagacccgcgccgaggtgaagttcgagggcgacaccctggtgaaccgcatcgagctgaagggcatcgacttcaaggaggacggcaacatcctggggcacaagctggagtacaactacaacagccacaacgtctatatcatggccgacaagcagaagaacggcatcaaggtgaacttcaagatccgccacaacatcgaggacggcagcgtgcagctcgccgaccactaccagcagaacacccccatcggcgacggccccgtgctgctgcccgacaaccactacctgagcacccagtccgccctgagcaaagaccccaacgagaagcgcgatcacatggtcctgctggagttcgtgaccgccgccgggatcactctcggcatggacgagctgtacaagtaatggatatctgtcgacggccgtcgttttacagccaagcttggctgttttggcggatgagagaagattttcagcctgatacagattaaatcagaacgcagaagcggtctgataaaacagaatttgcctggcggcagtagcgcggtggtcccacctgaccccatgccgaactcagaagtgaaacgccgtagcgccgatggtagtgtggggtctccccatgcgagagtagggaactgccaggcatcaaataaaacgaaaggctcagtcgaaagactgggcctttcgttttatctgttgtttgtcggtgaacgctctcctgagtaggacaaatccgccgggagcggatttgaacgttgcgaagcaacggcccggagggtggcgggcaggacgcccgccataaactgccaggcatcaaattaagcagaaggccatcctgacggatggcctttttgcgtttctacaaactcttttggtcgactctagagttccactgagcgtcagaccccgtagaaaagatcaaaggatcttcttgagatcctttttttctgcgcgtaatctgctgcttgcaaacaaaaaaaccaccgctaccagcggtggtttgtttgccggatcaagagctaccaactctttttccgaaggtaactggcttcagcagagcgcagataccaaatactgtccttctagtgtagccgtagttaggccaccacttcaagaactctgtagcaccgcctacatacctcgctctgctaatcctgttaccagtggctgctgccagtggcgataagtcgtgtcttaccgggttggactcaagacgatagttaccggataaggcgcagcggtcgggctgaacggggggttcgtgcacacagcccagcttggagcgaacgacctacaccgaactgagatacctacagcgtgagctatgagaaagcgccacgcttcccgaagggagaaaggcggacaggtatccggtaagcggcagggtcggaacaggagagcgcacgagggagcttccagggggaaacgcctggtatctttatagtcctgtcgggtttcgccacctctgacttgagcgtcgatttttgtgatgctcgtcaggggggcggagcctatggaaaaacgccagcaacgcggcctttttacggttcctggccttttgctggccttttgctcacatgttctttcctgcgttatcccctgattctgtggataaccgtattaccgcctttgagtgagctgataccgctcgccgcagccgaacgaccgagcgcagcgagtcagtgagcgaggaagcggaagatctagaagtactgctgactcataccaggcctgaatcgccccatcatccagccagaaagtgagggagccacggttgatgagagctttgttgtaggtggaccagttggtgattttgaacttttgctttgccacggaacggtctgcgttgtcgggaagatgcgtgatctgatccttcaactcagcaaaagttcgatttattcaacaaagccacgttgtgtctcaaaatctctgatgttacattgcacaagataaaaatatatcatcatgaacaataaaactgtctgcttacataaacagtaatacaaggggtgttatgagccatattcaacgggaaacgtcttgctcaaggccgcgattaaattccaacatggatgctgatttatatgggtataaatgggctcgcgataatgtcgggcaatcaggtgcgacaatctatcgattgtatgggaagcccgatgcgccagagttgtttctgaaacatggcaaaggtagcgttgccaatgatgttacagatgagatggtcagactaaactggctgacggaatttatgcctcttccgaccatcaagcattttatccgtactcctgatgatgcatggttactcaccactgcgatccccggaaaaacagcattccaggtattagaagaatatcctgattcaggtgaaaatattgttgatgcgctggcagtgttcctgcgccggttgcattcgattcctgtttgtaattgtccttttaacagcgatcgcgtatttcgtctcgctcaggcgcaatcacgaatgaataacggtttggttgatgcgagtgattttgatgacgagcgtaatggctggcctgttgaacaagtctggaaagaaatgcataagcttttgccattctcaccggattcagtcgtcactcatggtgatttctcacttgataaccttatttttgacgaggggaaattaataggttgtattgatgttggacgagtcggaatcgcagaccgataccaggatcttgccatcctatggaactgcctcggtgagttttctccttcattacagaaacggctttttcaaaaatatggtattgataatcctgatatgaataaattgcagtttcatttgatgctcgatgagtttttctaaggctagccccgggactagtgatctttgggagcagtccttgtgcgcttacgaggtgagccggtggggaaccgttatctgcctatggtgtgagcccccctagagagcttcaagagcaatcagcccgacctagaaaggaggccaagagagagacccctacggggggaaccgttttctgcctacgagatggcacatttactgggaagctttacggcgtcctcgtggaagttcaatgcccgcagacttaagtgctctattcacggtctgacgtgacacgctaaattcagacatagcttcattgattgtcggccacgagccagtctctccctcaacagtcataaaccaacctgcaatggtcaagcgatttcctttagctttcctagcttgtcgttgactggacttagctagtttttctcgctgtgctcgggcgtactcactgtttgggtctttccagcgttctgcggcctttttaccgccacgtcttcccatagtggccagagcttttcgccctcggctgctctgcgtctctgtctgacgagcagggacgactggctggcctttagcgacgtagccgcgcacacgtcgcgccatcgtctggcggtcacgcatcggcggcagatcaggctcacggccgtctgctccgaccgcctgagcgacggtgtaggcacgctcgtaggcgtcgatgatcttggtgtcttttaggcgctcaccagccgcttttaactggtatcccacagtcaaagcgtggcgaaaagccgtctcatcacgggcggcacgccctggagcagtccagaggacacggacgccgtcgatcagctctccagacgcttcagcggcgctcggcaggcttgcttcaagcgtggcaagtgcttttgcttccgcagtggcttttcttgccgcttcgatacgtgcccgtccgctagaaaactcctgctcatagcgttttttaggtttttctgtgcctgagatcatgcgagcaacctccataagatcagctaggcgatccacgcgattgtgctgggcatgccagcggtacgcggtgggatcgtcggagacgtgcagtggccaccggctcagcctatgtgaaaaagcctggtcagcgccgaaaacgcgggtcatttcctcggtcgttgcagccagcaggcgcatattcgggctgctcatgcctgctgcggcatacaccggatcaatgagccagatgagctggcatttcccgctcagtggattcacgccgatccaagctggcgctttttccaggcgtgcccagcgctccaaaatcgcgtagacctcggggtttacgtgctcgattttcccgccggcctggtggctcggcacatcaatgtccaggacaagcacggctgcgtgctgcgcgtgcgtcagagcaacatactggcaccgggcaagcgattttgaaccaactcggtataacttcggctgtgtttctcccgtgtccgggtctttgatccaagcgctggcgaagtcgcgggtcttgctgccctggaaattttctctgcccaggtgagcgaggaattcgcggcggtcttcgctcgtccagccacgtgatcgcagcgcgagctcgggatgggtgtcgaacagatcagcggaaaatttccaggccggtgtgtcaatgtctcgtgaatccgctagagtcatttttgagcgctttctcccaggtttggactgggggttagccgacgccctgtgagttaccgctcacggggcgttcaacatttttcaggtattcgtgcagcttatcgcttcttgccgcctgtgcgctttttcgacgcgcgacgctgctgccgattcggtgcaggtggtggcggcgctgacacgtcctgggcggccacggccacacgaaacgcggcatttacgatgtttgtcatgcctgcgggcaccgcgccacgatcgcggataattctcgctgccgcttccagctctgtgacgaccatggccaaaatttcgctcgggggacgcacttccagcgccatttgcgacctagccgcctccagctcctcggcgtggcgtttgttggcgcgctcgcggctggctgcggcacgacacgcatctgagcaatattttgcgcgccgtcctcgcgggtcaggccggggaggaatcaggccaccgcagtaggcgcaactgattcgatcctccactactgtgcgtcctcctggcgctgccgagcacgcagctcgtcagccagctcctcaagatccgccacgagagtttctaggtcgctcgcggcactggcccagtctcgtgatgctggcgcgtccgtcgtatcgagagctcggaaaaatccgatcaccgtttttaaatcgacggcagcatcgagcgcgtcggactccagcgcgacatcagagagatccatagctgatgattcgggccaattttggtacttcgtcgtgaaggtcatgacaccattataacgaacgttcgttaaagtttttggcggaaaatcacgcggcacgaaaattttcacgaagcgggactttgcgcagctcaggggtgctaaaaattttgtatcgcacttgatttttccgaaagacagattatctgcaaacggtgtgtcgtatttctggcttggtttttaaaaaatctggaatcgaaaatttgcggggcga

SEQ ID NO: 40 - DNA, 6292 bp, synthetic construct
  source 1..6292: mol_type = other DNA
gcgatcagcgacgccgcagggggctggaagaaaaacttggcgatgaaccgaatgcacttttaaggaaaaagcaggctcgtcaagcagctcgcgctgtgctgcccaacgctacagagtccagaatcgtggtgtctggaaacttccgcacctggaggcatttcattggcatgcgagccagtgaacatgcagacgtcgaaatccgcgaagtagcggtagaatgtttaagaaagctgcaggtagcagcgccaactgttttcggtgattttgagattgaaactttggcagacggatcgcaaatggcaacaagcccgtatgtcatggacttttaacgcaaagctcacacccacgagctaaaaattcatatagttaagacaacatttttggctgtaaaagacagccgtaaaaacctcttgctcgtgtcaattgttcttatcggaatgtggcttgggcgattgttatgcaaaagttgttaggttttttgcggggttgtttaacccccaaatgagggaagatggtaaccttgaactctatggtcagcaagggtgaggagctattcaccggagtagttcccatccttgttgagctggacggggacgtgaacgggcacaagttctccgtgagtggggagggcgagggtgacgccacgtacgggaagcttaccctgaagttcatctgtactacagggaagcttcccgtaccgtggcccaccctcgtcactaccctcacttacggagtgcagtgcttttcacgttaccccgaccacatgaagcagcatgacttcttcaagtcggccatgcctgaaggatacgtccaggagcggacgatattcttcaaagacgatgggaattataagacccgtgccgaggttaagttcgagggtgataccctcgtcaatagaatcgagctgaagggcatcgattttaaggaggacggtaacatcctcggacataagctcgagtacaattataattcccataacgtctacataatggccgacaagcagaagaatggtatcaaggtgaacttcaagatccggcacaacatcgaagatgggagtgttcagcttgctgatcactatcagcaaaacactcccatcggcgatgggccggtcttgttacctgataaccattacttgtccacccagagtgccctgtcgaaggatccgaacgaaaagcgggaccacatggtcctgcttgagttcgtgaccgcggcagggatcactctgggtatggacgagttatataagtaatggatatctgtcgacggccgtcgttttacagccaagcttggctgttttggcggatgagagaagattttcagcctgatacagattaaatcagaacgcagaagcggtctgataaaacagaatttgcctggcggcagtagcgcggtggtcccacctgaccccatgccgaactcagaagtgaaacgccgtagcgccgatggtagtgtggggtctccccatgcgagagtagggaactgccaggcatcaaataaaacgaaaggctcagtcgaaagactgggcctttcgttttatctgttgtttgtcggtgaacgctctcctgagtaggacaaatccgccgggagcggatttgaacgttgcgaagcaacggcccggagggtggcgggcaggacgcccgccataaactgccaggcatcaaattaagcagaaggccatcctgacggatggcctttttgcgtttctacaaactcttttggtcgactctagagttccactgagcgtcagaccccgtagaaaagatcaaaggatcttcttgagatcctttttttctgcgcgtaatctgctgcttgcaaacaaaaaaaccaccgctaccagcggtggtttgtttgccggatcaagagctaccaactctttttccgaaggtaactggcttcagcagagcgcagataccaaatactgtccttctagtgtagccgtagttaggccaccacttcaagaactctgtagcaccgcctacatacctcgctctgctaatcctgttaccagtggctgctgccagtggcgataagtcgtgtcttaccgggttggactcaagacgatagttaccggataaggcgcagcggtcgggctgaacggggggttcgtgcacacagcccagcttggagcgaacgacctacaccgaactgagatacctacagcgtgagctatgagaaagcgccacgcttcccgaagggagaaaggcggacaggtatccggtaagcggcagggtcggaacaggagagcgcacgagggagcttccagggggaaacgcctggtatctttatagtcctgtcgggtttcgccacctctgacttgagcgtcgatttttgtgatgctcgtcaggggggcggagcctatggaaaaacgccagcaacgcggcctttttacggttcctggccttttgctggccttttgctcacatgttctttcctgcgttatcccctgattctgtggataaccgtattaccgcctttgagtgagctgataccgctcgccgcagccgaacgaccgagcgcagcgagtcagtgagcgaggaagcggaagatctagaagtactgctgactcataccaggcctgaatcgccccatcatccagccagaaagtgagggagccacggttgatgagagctttgttgtaggtggaccagttggtgattttgaacttttgctttgccacggaacggtctgcgttgtcgggaagatgcgtgatctgatccttcaactcagcaaaagttcgatttattcaacaaagccacgttgtgtctcaaaatctctgatgttacattgcacaagataaaaatatatcatcatgaacaataaaactgtctgcttacataaacagtaatacaaggggtgttatgagccatattcaacgggaaacgtcttgctcaaggccgcgattaaattccaacatggatgctgatttatatgggtataaatgggctcgcgataatgtcgggcaatcaggtgcgacaatctatcgattgtatgggaagcccgatgcgccagagttgtttctgaaacatggcaaaggtagcgttgccaatgatgttacagatgagatggtcagactaaactggctgacggaatttatgcctcttccgaccatcaagcattttatccgtactcctgatgatgcatggttactcaccactgcgatccccggaaaaacagcattccaggtattagaagaatatcctgattcaggtgaaaatattgttgatgcgctggcagtgttcctgcgccggttgcattcgattcctgtttgtaattgtccttttaacagcgatcgcgtatttcgtctcgctcaggcgcaatcacgaatgaataacggtttggttgatgcgagtgattttgatgacgagcgtaatggctggcctgttgaacaagtctggaaagaaatgcataagcttttgccattctcaccggattcagtcgtcactcatggtgatttctcacttgataaccttatttttgacgaggggaaattaataggttgtattgatgttggacgagtcggaatcgcagaccgataccaggatcttgccatcctatggaactgcctcggtgagttttctccttcattacagaaacggctttttcaaaaatatggtattgataatcctgatatgaataaattgcagtttcatttgatgctcgatgagtttttctaaggctagccccgggactagtgatctttgggagcagtccttgtgcgcttacgaggtgagccggtggggaaccgttatctgcctatggtgtgagcccccctagagagcttcaagagcaatcagcccgacctagaaaggaggccaagagagagacccctacggggggaaccgttttctgcctacgagatggcacatttactgggaagctttacggcgtcctcgtggaagttcaatgcccgcagacttaagtgctctattcacggtctgacgtgacacgctaaattcagacatagcttcattgattgtcggccacgagccagtctctccctcaacagtcataaaccaacctgcaatggtcaagcgatttcctttagctttcctagcttgtcgttgactggacttagctagtttttctcgctgtgctcgggcgtactcactgtttgggtctttccagcgttctgcggcctttttaccgccacgtcttcccatagtggccagagcttttcgccctcggctgctctgcgtctctgtctgacgagcagggacgactggctggcctttagcgacgtagccgcgcacacgtcgcgccatcgtctggcggtcacgcatcggcggcagatcaggctcacggccgtctgctccgaccgcctgagcgacggtgtaggcacgctcgtaggcgtcgatgatcttggtgtcttttaggcgctcaccagccgcttttaactggtatcccacagtcaaagcgtggcgaaaagccgtctcatcacgggcggcacgccctggagcagtccagaggacacggacgccgtcgatcagctctccagacgcttcagcggcgctcggcaggcttgcttcaagcgtggcaagtgcttttgcttccgcagtggcttttcttgccgcttcgatacgtgcccgtccgctagaaaactcctgctcatagcgttttttaggtttttctgtgcctgagatcatgcgagcaacctccataagatcagctaggcgatccacgcgattgtgctgggcatgccagcggtacgcggtgggatcgtcggagacgtgcagtggccaccggctcagcctatgtgaaaaagcctggtcagcgccgaaaacgcgggtcatttcctcggtcgttgcagccagcaggcgcatattcgggctgctcatgcctgctgcggcatacaccggatcaatgagccagatgagctggcatttcccgctcagtggattcacgccgatccaagctggcgctttttccaggcgtgcccagcgctccaaaatcgcgtagacctcggggtttacgtgctcgattttcccgccggcctggtggctcggcacatcaatgtccaggacaagcacggctgcgtgctgcgcgtgcgtcagagcaacatactggcaccgggcaagcgattttgaaccaactcggtataacttcggctgtgtttctcccgtgtccgggtctttgatccaagcgctggcgaagtcgcgggtcttgctgccctggaaattttctctgcccaggtgagcgaggaattcgcggcggtcttcgctcgtccagccacgtgatcgcagcgcgagctcgggatgggtgtcgaacagatcagcggaaaatttccaggccggtgtgtcaatgtctcgtgaatccgctagagtcatttttgagcgctttctcccaggtttggactgggggttagccgacgccctgtgagttaccgctcacggggcgttcaacatttttcaggtattcgtgcagcttatcgcttcttgccgcctgtgcgctttttcgacgcgcgacgctgctgccgattcggtgcaggtggtggcggcgctgacacgtcctgggcggccacggccacacgaaacgcggcatttacgatgtttgtcatgcctgcgggcaccgcgccacgatcgcggataattctcgctgccgcttccagctctgtgacgaccatggccaaaatttcgctcgggggacgcacttccagcgccatttgcgacctagccgcctccagctcctcggcgtggcgtttgttggcgcgctcgcggctggctgcggcacgacacgcatctgagcaatattttgcgcgccgtcctcgcgggtcaggccggggaggaatcaggccaccgcagtaggcgcaactgattcgatcctccactactgtgcgtcctcctggcgctgccgagcacgcagctcgtcagccagctcctcaagatccgccacgagagtttctaggtcgctcgcggcactggcccagtctcgtgatgctggcgcgtccgtcgtatcgagagctcggaaaaatccgatcaccgtttttaaatcgacggcagcatcgagcgcgtcggactccagcgcgacatcagagagatccatagctgatgattcgggccaattttggtacttcgtcgtgaaggtcatgacaccattataacgaacgttcgttaaagtttttggcggaaaatcacgcggcacgaaaattttcacgaagcgggactttgcgcagctcaggggtgctaaaaattttgtatcgcacttgatttttccgaaagacagattatctgcaaacggtgtgtcgtatttctggcttggtttttaaaaaatctggaatcgaaaatttgcggggcga

SEQ ID NO: 41 - DNA, 1266 bp, Corynebacterium glutamicum
  source 1..1266: mol_type = genomic DNA
gtggccctggtcgtacagaaatatggcggttcctcgcttgagagtgcggaacgcattagaaacgtcgctgaacggatcgttgccaccaagaaggctggaaatgatgtcgtggttgtctgctccgcaatgggagacaccacggatgaacttctagaacttgcagcggcagtgaatcccgttccgccagctcgtgaaatggatatgctcctgactgctggtgagcgtatttctaacgctctcgtcgccatggctattgagtcccttggcgcagaagcccaatctttcacgggctctcaggctggtgtgctcaccaccgagcgccacggaaacgcacgcattgttgatgtcactccaggtcgtgtgcgtgaagcactcgatgagggcaagatctgcattgttgctggtttccagggtgttaataaagaaacccgcgatgtcaccacgttgggtcgtggtggttctgacaccactgcagttgcgttggcagctgctttgaacgctgatgtgtgtgagatttactcggacgttgacggtgtgtataccgctgacccgcgcatcgttcctaatgcacagaagctggaaaagctcagcttcgaagaaatgctggaacttgctgctgttggctccaagattttggtgctgcgcagtgttgaatacgctcgtgcattcaatgtgccacttcgcgtacgctcgtcttatagtaatgatcccggcactttgattgccggctctatggaggatattcctgtggaagaagcagtccttaccggtgtcgcaaccgacaagtccgaagccaaagtaaccgttctgggtatttccgataagccaggcgaggctgcgaaggttttccgtgcgttggctgatgcagaaatcaacattgacatggttctgcagaacgtctcttctgtagaagacggcaccaccgacatcatcttcacctgccctcgttccgacggccgccgcgcgatggagatcttgaagaagcttcaggttcagggcaactggaccaatgtgctttacgacgaccaggtcggcaaagtctccctcgtgggtgctggcatgaagtctcacccaggtgttaccgcagagttcatggaagctctgcgcgatgtcaacgtgaacatcgaattgatttccacctctgagattcgtatttccgtgctgatccgtgaagatgatctggatgctgctgcacgtgcattgcatgagcagttccagctgggcggcgaagacgaagccgtcgtttatgcaggcaccggacgctaa

SEQ ID NO: 42 - DNA, 1266 bp, synthetic construct
  source 1..1266: mol_type = other DNA
gttgctttagttgttcaaaaatatggtggttcttctttagaatctgctgaaagaattagaaatgttgctgaaagaattgttgctactaaaaaagctggtaatgatgttgttgttgtttgttctgctatgggtgatactactgatgaattattagaattagctgctgctgttaatcctgttcctcctgctagagaaatggatatgttattaactgctggtgaaagaatttctaatgctttagttgctatggctattgaatctttaggtgctgaagctcaatcttttactggttctcaagctggtgttttaactactgaaagacatggtaatgctagaattgttgatgttactcctggtagagttagagaagctttagatgaaggtaaaatttgtattgttgctggttttcaaggtgttaataaagaaactagagatgttactactttaggtagaggtggttctgatactactgctgttgctttagctgctgctttaaatgctgatgtttgtgaaatttattctgatgttgatggtgtttatactgctgatcctagaattgttcctaatgctcaaaaattagaaaaattatcttttgaagaaatgttagaattagctgctgttggttctaaaattttagttttaagatctgttgaatatgctagagcttttaatgttcctttaagagttagatcttcttattctaatgatcctggtactttaattgctggttctatggaagatattcctgttgaagaagctgttttaactggtgttgctactgataaatctgaagctaaagttactgttttaggtatttctgataaacctggtgaagctgctaaagtttttagagctttagctgatgctgaaattaatattgatatggttttacaaaatgtttcttctgttgaagatggtactactgatattatttttacttgtcctagatctgatggtagaagagctatggaaattttaaaaaaattacaagttcaaggtaattggactaatgttttatatgatgatcaagttggtaaagtttctttagttggtgctggtatgaaatctcatcctggtgttactgctgaatttatggaagctttaagagatgttaatgttaatattgaattaatttctacttctgaaattagaatttctgttttaattagagaagatgatttagatgctgctgctagagctttacatgaacaatttcaattaggtggtgaagatgaagctgttgtttatgctggtactggtagataa

SEQ ID NO: 43 - DNA, 1338 bp, Corynebacterium glutamicum
  source 1..1338: mol_type = genomic DNA
atgacctcagcatctgccccaagctttaaccccggcaagggtcccggctcagcagtcggaattgcccttttaggattcggaacagtcggcactgaggtgatgcgtctgatgaccgagtacggtgatgaacttgcgcaccgcattggtggcccactggaggttcgtggcattgctgtttctgatatctcaaagccacgtgaaggcgttgcacctgagctgctcactgaggacgcttttgcactcatcgagcgcgaggatgttgacatcgtcgttgaggttatcggcggcattgagtacccacgtgaggtagttctcgcagctctgaaggccggcaagtctgttgttaccgccaataaggctcttgttgcagctcactctgctgagcttgctgatgcagcggaagccgcaaacgttgacctgtacttcgaggctgctgttgcaggcgcaattccagtggttggcccactgcgtcgctccctggctggcgatcagatccagtctgtgatgggcatcgttaacggcaccaccaacttcatcttggacgccatggattccaccggcgctgactatgcagattctttggctgaggcaactcgtttgggttacgccgaagctgatccaactgcagacgtcgaaggccatgacgccgcatccaaggctgcaattttggcatccatcgctttccacacccgtgttaccgcggatgatgtgtactgcgaaggtatcagcaacatcagcgctgccgacattgaggcagcacagcaggcaggccacaccatcaagttgttggccatctgtgagaagttcaccaacaaggaaggaaagtcggctatttctgctcgcgtgcacccgactctattacctgtgtcccacccactggcgtcggtaaacaagtcctttaatgcaatctttgttgaagcagaagcagctggtcgcctgatgttctacggaaacggtgcaggtggcgcgccaaccgcgtctgctgtgcttggcgacgtcgttggtgccgcacgaaacaaggtgcacggtggccgtgctccaggtgagtccacctacgctaacctgccgatcgctgatttcggtgagaccaccactcgttaccacctcgacatggatgtggaagatcgcgtgggggttttggctgaattggctagcctgttctctgagcaaggaatctccctgcgtacaatccgacaggaagagcgcgatgatgatgcacgtctgatcgtggtcacccactctgcgctggaatctgatctttcccgcaccgttgaactgctgaaggctaagcctgttgttaaggcaatcaacagtgtgatccgcctcgaaagggactaa

SEQ ID NO: 44 - DNA, 1335 bp, synthetic construct
  source 1..1335: mol_type = other DNA
atgacgagcgcgtcggcgccgtcatttaatcccggcaaggggccgggtagcgctgttggtatcgcgttgttgggctttgggacggtaggcacagaggtgatgagactgatgacagagtacggcgatgagctcgcccaccgtatcggcggcccgctcgaagtgcgaggcatcgcggtcagcgacatcagcaagccacgcgagggcgtggctcctgagttgctgaccgaggatgccttcgcacttatcgagcgggaggacgtcgatatagtggtcgaggtcatcggcggaatagagtatccacgtgaggtggtcttggcggcgttgaaagccggcaagagtgtggtgaccgccaacaaggcgttggtggcagcacactctgccgagcttgccgacgccgccgaggccgccaacgtggatctctatttcgaggccgcggtcgccggagcgatcccagtggtgggaccgctccggcgatcgctggccggggatcagatacagtcggtcatgggtattgtcaatggcaccacgaattttattctggatgccatggacagtaccggtgccgactatgctgattccctagccgaggccactcggctgggctatgctgaggcagatccgacggccgacgtggaggggcacgatgccgcctccaaggccgcgattctggccagcatagcctttcacacgcgcgtgacggcggacgatgtctattgtgagggaatttctaacatatcggcagcagacattgaggcggcccagcaggctgggcacaccatcaagctgctggcgatatgtgagaagttcaccaacaaggagggcaagtccgccatcagcgcgcgtgtgcacccgactctgttaccagtctctcaccctctggcctccgtcaataagtccttcaacgcgatcttcgtggaggcggaggcggcggggcgcctcatgttctatggcaatggagcaggaggcgccccgaccgcctccgccgtcctcggagacgtggtgggcgccgcccggaacaaggttcacggggggcgcgcaccaggggagagtacgtacgcgaacctccccatcgccgacttcggcgagaccaccacccggtaccacctcgacatggatgtcgaggaccgggtgggggtcttggcggagttggcgagtctcttcagtgagcagggcatctcgttgcgcaccatccggcaggaggagcgcgacgacgatgcccggctcattgtggtgacccacagtgcgctcgagtccgacttgagccgcactgtggagctcttgaaggccaagccggtcgtcaaggctatcaacagcgttatccggctcgagcgggat

SEQ ID NO: 45 - DNA, 5722 bp, synthetic construct
  source 1..5722: mol_type = other DNA
attaggcaccccaggctttacactttatgcttccggctcgtatgttgtgtggaattgtgagcggataacaatttcacacaggaaacagctatgaccatgattacgccaagcttgcatgcctgcaggtcgactctagaggatccccgggtaccgagctcgaattcactggccgtcgttttacaacgtcgtgactgggaaaaccctggcgttacccaacttaatcgccttgcagcacatccccctttcgccagctggcgtaatagcgaagaggcccgcaccgatcgcccttcccaacagttgcgcagcctgaatggcgaatggcgcgataagctagcttcacgctgccgcaagcactcagggcgcaagggctgctaaaggaagcggaacacgtagaaagccagtccgcagaaacggtgctgaccccggatgaatgtcagctactgggctatctggacaagggaaaacgcaagcgcaaagagaaagcaggtagcttgcagtgggcttacatggcgatagctagactgggcggttttatggacagcaagcgaaccggaattgccagctggggcgccctctggtaaggttgggaagccctgcaaagtaaactggatggctttcttgccgccaaggatctgatggcgcaggggatcaagatctgatcaagagacaggatgaggatcgtttcgcatgattgaacaagatggattgcacgcaggttctccggccgcttgggtggagaggctattcggctatgactgggcacaacagacaatcggctgctctgatgccgccgtgttccggctgtcagcgcaggggcgcccggttctttttgtcaagaccgacctgtccggtgccctgaatgaactccaagacgaggcagcgcggctatcgtggctggccacgacgggcgttccttgcgcagctgtgctcgacgttgtcactgaagcgggaagggactggctgctattgggcgaagtgccggggcaggatctcctgtcatctcaccttgctcctgccgagaaagtatccatcatggctgatgcaatgcggcggctgcatacgcttgatccggctacctgcccattcgaccaccaagcgaaacatcgcatcgagcgagcacgtactcggatggaagccggtcttgtcgatcaggatgatctggacgaagagcatcaggggctcgcgccagccgaactgttcgccaggctcaaggcgcggatgcccgacggcgaggatctcgtcgtgacccatggcgatgcctgcttgccgaatatcatggtggaaaatggccgcttttctggattcatcgactgtggccggctgggtgtggcggaccgctatcaggacatagcgttggctacccgtgatattgctgaagagcttggcggcgaatgggctgaccgcttcctcgtgctttacggtatcgccgctcccgattcgcagcgcatcgccttctatcgccttcttgacgagttcttctgagcgggactctggggttcgctagaggatcgatcctttttaacccatcacatatacctgccgttcactattatttagtgaaatgagatattatgatattttctgaattgtgattaaaaaggcaactttatgcccatgcaacagaaactataaaaaatacagagaatgaaaagaaacagatagattttttagttctttaggcccgtagtctgcaaatccttttatgattttctatcaaacaaaagaggaaaatagaccagttgcaatccaaacgagagtctaatagaatgaggtcgaaaagtaaatcgcgcgggtttgttactgataaagcaggcaagacctaaaatgtgtaaagggcaaagtgtatactttggcgtcaccccttacatattttaggtctttttttattgtgcgtaactaacttgccatcttcaaacaggagggctggaagaagcagaccgctaacacagtacataaaaaaggagacatgaacgatgaacatcaaaaagtttgcaaaacaagcaacagtattaacctttactaccgcactgctggcaggaggcgcaactcaagcgtttgcgaaagaaacgaaccaaaagccatataaggaaacatacggcatttcccatattacacgccatgatatgctgcaaatccctgaacagcaaaaaaatgaaaaatatcaagtttctgaatttgattcgtccacaattaaaaatatctcttctgcaaaaggcctggacgtttgggacagctggccattacaaaacgctgacggcactgtcgcaaactatcacggctaccacatcgtctttgcattagccggagatcctaaaaatgcggatgacacatcgatttacatgttctatcaaaaagtcggcgaaacttctattgacagctggaaaaacgctggccgcgtctttaaagacagcgacaaattcgatgcaaatgattctatcctaaaagaccaaacacaagaatggtcaggttcagccacatttacatctgacggaaaaatccgtttattctacactgatttctccggtaaacattacggcaaacaaacactgacaactgcacaagttaacgtatcagcatcagacagctctttgaacatcaacggtgtagaggattataaatcaatctttgacggtgacggaaaaacgtatcaaaatgtacagcagttcatcgatgaaggcaactacagctcaggcgacaaccatacgctgagagatcctcactacgtagaagataaaggccacaaatacttagtatttgaagcaaacactggaactgaagatggctaccaaggcgaagaatctttatttaacaaagcatactatggcaaaagcacatcattcttccgtcaagaaagtcaaaaacttctgcaaagcgataaaaaacgcacggctgagttagcaaacggcgctctcggtatgattgagctaaacgatgattacacactgaaaaaagtgatgaaaccgctgattgcatctaacacagtaacagatgaaattgaacgcgcgaacgtctttaaaatgaacggcaaatggtacctgttcactgactcccgcggatcaaaaatgacgattgacggcattacgtctaacgatatttacatgcttggttatgtttctaattctttaactggcccatacaagccgctgaacaaaactggccttgtgttaaaaatggatcttgatcctaacgatgtaacctttacttactcacacttcgctgtacctcaagcgaaaggaaacaatgtcgtgattacaagctatatgacaaacagaggattctacgcagacaaacaatcaacgtttgcgccgagcttcctgctgaacatcaaaggcaagaaaacatctgttgtcaaagacagcatccttgaacaaggacaattaacagttaacaaataaaaacgcaaaagaaaatgccgatgggtaccgagcgaaatgaccgaccaagcgacgcccaacctgccatcacgagatttcgattccaccgccgccttctatgaaaggttgggcttcggaatcgttttccgggacgccctcgcggacgtgctcatagtccacgacgcccgtgattttgtagccctggccgacggccagcaggtaggccgacaggctcatgccggccgccgccgccttttcctcaatcgctcttcgttcgtctggaaggcagtacaccttgataggtgggctgcccttcctggttggcttggtttcatcagccatccgcttgccctcatctgttacgccggcggtagccggccagcctcgcagagcaggattcccgttgagcaccgccaggtgcgaataagggacagtgaagaaggaacacccgctcgcgggtgggcctacttcacctatcctgccccgctgacgccgttggatacaccaaggaaagtctacacgaaccctttggcaaaatcctgtatatcgtgcgaaaaaggatggatataccgaaaaaatcgctataatgaccccgaagcagggttatgcagcggaaaagcgctgcttccctgctgttttgtggaatatctaccgactggaaacaggcaaatgcaggaaattactgaactgaggggacaggcgagagacgatgccaaagagctcctgaaaatctcgataactcaaaaaatacgcccggtagtgatcttatttcattatggtgaaagttggaacctcttacgtgccgatcaacgtctcattttcgccaaaagttggcccagggcttcccggtatcaacagggacaccaggatttatttattctgcgaagtgatcttccgtcacaggtatttattcggcgcaaagtgcgtcgggtgatgctgccaacttactgatttagtgtatgatggtgtttttgaggtgctccagtggcttctgtttctatcagctcctgaaaatctcgataactcaaaaaatacgcccggtagtgatcttatttcattatggtgaaagttggaacctcttacgtgccgatcaacgtctcattttcgccaaaagttggcccagggcttcccggtatcaacagggacaccaggatttatttattctgcgaagtgatcttccgtcacaggtatttattcggcgcaaagtgcgtcgggtgatgctgccaacttactgatttagtgtatgatggtgtttttgaggtgctccagtggcttctgtttctatcagggctggatgatcctccagcgcggggatctcatgctggagttcttcgcccaccccaaaaggatctaggtgaagatcctttttgataatctcatgaccaaaatcccttaacgtgagttttcgttccactgagcgtcagaccccgtagaaaagatcaaaggatcttcttgagatcctttttttctgcgcgtaatctgctgcttgcaaacaaaaaaaccaccgctaccagcggtggtttgtttgccggatcaagagctaccaactctttttccgaaggtaactggcttcagcagagcgcagataccaaatactgtccttctagtgtagccgtagttaggccaccacttcaagaactctgtagcaccgcctacatacctcgctctgctaatcctgttaccagtggctgctgccagtggcgataagtcgtgtcttaccgggttggactcaagacgatagttaccggataaggcgcagcggtcgggctgaacggggggttcgtgcacacagcccagcttggagcgaacgacctacaccgaactgagatacctacagcgtgagcattgagaaagcgccacgcttcccgaagggagaaaggcggacaggtatccggtaagcggcagggtcggaacaggagagcgcacgagggagcttccagggggaaacgcctggtatctttatagtcctgtcgggtttcgccacctctgacttgagcgtcgatttttgtgatgctcgtcaggggggcggagcctatggaaaaacgccagcaacgcggcctttttacggttcctggccttttgctggccttttgctcacatgttctttcctgcgttatcccctgattctgtggataaccgtattaccgcctttgagtgagctgataccgctcgccgcagccgaacgaccgagcgcagcgagtcagtgagcgaggaagcggaagagcgcccaatacgcaaaccgcctctccccgcgcgttggccgattcattaatgcagctggcacgacaggtttcccgactggaaagcgggcagtgagcgcaacgcaattaatgtgagttagctcactc

SEQ ID NO: 46 - DNA, 7988 bp, synthetic construct
  source 1..7988: mol_type = other DNA
cgacaggacaagcactggttgcactaccaagagggtgccgaaaccaagtgctactgtttgtaagaaatatgccagcatcgcgtactcatgcctgcccaccacatcggtgtcatcagagcattgagtaaaggtgagctccttagggagccatcttttggggtgcggagcgcgatccggtgtctgaccacggtgccccatgcgattgttaatgccgatgctagggcgaaaagcacggcgagcagattgctttgcacttgattcagggtagttgactaaagagttgctcgcgaagtagcacctgtcacttttgtctcaaatattaaatcgaatatcaatatatggtctgtttattggaacgcgtcccagtggctgagacgcatccgctaaagccccaggaaccctgtgcagaaagaaaacactcctctggctaggtagacacagtttataaaggtagagttgagcgggtaactgtcagcacgtagatcgaaaggtgcacaaaggttgctttagttgttcaaaaatatggtggttcttctttagaatctgctgaaagaattagaaatgttgctgaaagaattgttgctactaaaaaagctggtaatgatgttgttgttgtttgttctgctatgggtgatactactgatgaattattagaattagctgctgctgttaatcctgttcctcctgctagagaaatggatatgttattaactgctggtgaaagaatttctaatgctttagttgctatggctattgaatctttaggtgctgaagctcaatcttttactggttctcaagctggtgttttaactactgaaagacatggtaatgctagaattgttgatgttactcctggtagagttagagaagctttagatgaaggtaaaatttgtattgttgctggttttcaaggtgttaataaagaaactagagatgttactactttaggtagaggtggttctgatactactgctgttgctttagctgctgctttaaatgctgatgtttgtgaaatttattctgatgttgatggtgtttatactgctgatcctagaattgttcctaatgctcaaaaattagaaaaattatcttttgaagaaatgttagaattagctgctgttggttctaaaattttagttttaagatctgttgaatatgctagagcttttaatgttcctttaagagttagatcttcttattctaatgatcctggtactttaattgctggttctatggaagatattcctgttgaagaagctgttttaactggtgttgctactgataaatctgaagctaaagttactgttttaggtatttctgataaacctggtgaagctgctaaagtttttagagctttagctgatgctgaaattaatattgatatggttttacaaaatgtttcttctgttgaagatggtactactgatattatttttacttgtcctagatctgatggtagaagagctatggaaattttaaaaaaattacaagttcaaggtaattggactaatgttttatatgatgatcaagttggtaaagtttctttagttggtgctggtatgaaatctcatcctggtgttactgctgaatttatggaagctttaagagatgttaatgttaatattgaattaatttctacttctgaaattagaatttctgttttaattagagaagatgatttagatgctgctgctagagctttacatgaacaatttcaattaggtggtgaagatgaagctgttgtttatgctggtactggtagataaagttttaaaggagtagttttacaatgaccaccatcgcagttgttggtgcaaccggccaggtcggccaggttatgcgcacccttttggaagagcgcaatttcccagctgacactgttcgtttctttgcttccccacgttccgcaggccgtaagattgaattccgtggcacggaaatcgaggtagaagacattactcaggcaaccgaggagtccctcaaggacatcgacgttgcgttgttctccgctggaggcaccgcttccaagcagtacgctccactgttcgctgctgcaggcgcgactgttgtggataactcttctgcttggcgcaaggacgacgaggttccactaatcgtctctgaggtgaacccttccgacaaggattccctggtcaagggcattattgcgaaccctaactgcaccaccatggctgcgatgccagtgctgaagccacttcacgatgccgctggtcttgtaaagcttcacgtttcctcttaccaggctgggtaccgagctcgaattcactggccgtcgttttacaacgtcgtgactgggaaaaccctggcgttacccaacttaatcgccttgcagcacatccccctttcgccagctggcgtaatagcgaagaggcccgcaccgatcgcccttcccaacagttgcgcagcctgaatggcgaatggcgcgataagctagcttcacgctgccgcaagcactcagggcgcaagggctgctaaaggaagcggaacacgtagaaagccagtccgcagaaacggtgctgaccccggatgaatgtcagctactgggctatctggacaagggaaaacgcaagcgcaaagagaaagcaggtagcttgcagtgggcttacatggcgatagctagactgggcggttttatggacagcaagcgaaccggaattgccagctggggcgccctctggtaaggttgggaagccctgcaaagtaaactggatggctttcttgccgccaaggatctgatggcgcaggggatcaagatctgatcaagagacaggatgaggatcgtttcgcatgattgaacaagatggattgcacgcaggttctccggccgcttgggtggagaggctattcggctatgactgggcacaacagacaatcggctgctctgatgccgccgtgttccggctgtcagcgcaggggcgcccggttctttttgtcaagaccgacctgtccggtgccctgaatgaactccaagacgaggcagcgcggctatcgtggctggccacgacgggcgttccttgcgcagctgtgctcgacgttgtcactgaagcgggaagggactggctgctattgggcgaagtgccggggcaggatctcctgtcatctcaccttgctcctgccgagaaagtatccatcatggctgatgcaatgcggcggctgcatacgcttgatccggctacctgcccattcgaccaccaagcgaaacatcgcatcgagcgagcacgtactcggatggaagccggtcttgtcgatcaggatgatctggacgaagagcatcaggggctcgcgccagccgaactgttcgccaggctcaaggcgcggatgcccgacggcgaggatctcgtcgtgacccatggcgatgcctgcttgccgaatatcatggtggaaaatggccgcttttctggattcatcgactgtggccggctgggtgtggcggaccgctatcaggacatagcgttggctacccgtgatattgctgaagagcttggcggcgaatgggctgaccgcttcctcgtgctttacggtatcgccgctcccgattcgcagcgcatcgccttctatcgccttcttgacgagttcttctgagcgggactctggggttcgctagaggatcgatcctttttaacccatcacatatacctgccgttcactattatttagtgaaatgagatattatgatattttctgaattgtgattaaaaaggcaactttatgcccatgcaacagaaactataaaaaatacagagaatgaaaagaaacagatagattttttagttctttaggcccgtagtctgcaaatccttttatgattttctatcaaacaaaagaggaaaatagaccagttgcaatccaaacgagagtctaatagaatgaggtcgaaaagtaaatcgcgcgggtttgttactgataaagcaggcaagacctaaaatgtgtaaagggcaaagtgtatactttggcgtcaccccttacatattttaggtctttttttattgtgcgtaactaacttgccatcttcaaacaggagggctggaagaagcagaccgctaacacagtacataaaaaaggagacatgaacgatgaacatcaaaaagtttgcaaaacaagcaacagtattaacctttactaccgcactgctggcaggaggcgcaactcaagcgtttgcgaaagaaacgaaccaaaagccatataaggaaacatacggcatttcccatattacacgccatgatatgctgcaaatccctgaacagcaaaaaaatgaaaaatatcaagtttctgaatttgattcgtccacaattaaaaatatctcttctgcaaaaggcctggacgtttgggacagctggccattacaaaacgctgacggcactgtcgcaaactatcacggctaccacatcgtctttgcattagccggagatcctaaaaatgcggatgacacatcgatttacatgttctatcaaaaagtcggcgaaacttctattgacagctggaaaaacgctggccgcgtctttaaagacagcgacaaattcgatgcaaatgattctatcctaaaagaccaaacacaagaatggtcaggttcagccacatttacatctgacggaaaaatccgtttattctacactgatttctccggtaaacattacggcaaacaaacactgacaactgcacaagttaacgtatcagcatcagacagctctttgaacatcaacggtgtagaggattataaatcaatctttgacggtgacggaaaaacgtatcaaaatgtacagcagttcatcgatgaaggcaactacagctcaggcgacaaccatacgctgagagatcctcactacgtagaagataaaggccacaaatacttagtatttgaagcaaacactggaactgaagatggctaccaaggcgaagaatctttatttaacaaagcatactatggcaaaagcacatcattcttccgtcaagaaagtcaaaaacttctgcaaagcgataaaaaacgcacggctgagttagcaaacggcgctctcggtatgattgagctaaacgatgattacacactgaaaaaagtgatgaaaccgctgattgcatctaacacagtaacagatgaaattgaacgcgcgaacgtctttaaaatgaacggcaaatggtacctgttcactgactcccgcggatcaaaaatgacgattgacggcattacgtctaacgatatttacatgcttggttatgtttctaattctttaactggcccatacaagccgctgaacaaaactggccttgtgttaaaaatggatcttgatcctaacgatgtaacctttacttactcacacttcgctgtacctcaagcgaaaggaaacaatgtcgtgattacaagctatatgacaaacagaggattctacgcagacaaacaatcaacgtttgcgccgagcttcctgctgaacatcaaaggcaagaaaacatctgttgtcaaagacagcatccttgaacaaggacaattaacagttaacaaataaaaacgcaaaagaaaatgccgatgggtaccgagcgaaatgaccgaccaagcgacgcccaacctgccatcacgagatttcgattccaccgccgccttctatgaaaggttgggcttcggaatcgttttccgggacgccctcgcggacgtgctcatagtccacgacgcccgtgattttgtagccctggccgacggccagcaggtaggccgacaggctcatgccggccgccgccgccttttcctcaatcgctcttcgttcgtctggaaggcagtacaccttgataggtgggctgcccttcctggttggcttggtttcatcagccatccgcttgccctcatctgttacgccggcggtagccggccagcctcgcagagcaggattcccgttgagcaccgccaggtgcgaataagggacagtgaagaaggaacacccgctcgcgggtgggcctacttcacctatcctgccccgctgacgccgttggatacaccaaggaaagtctacacgaaccctttggcaaaatcctgtatatcgtgcgaaaaaggatggatataccgaaaaaatcgctataatgaccccgaagcagggttatgcagcggaaaagcgctgcttccctgctgttttgtggaatatctaccgactggaaacaggcaaatgcaggaaattactgaactgaggggacaggcgagagacgatgccaaagagctcctgaaaatctcgataactcaaaaaatacgcccggtagtgatcttatttcattatggtgaaagttggaacctcttacgtgccgatcaacgtctcattttcgccaaaagttggcccagggcttcccggtatcaacagggacaccaggatttatttattctgcgaagtgatcttccgtcacaggtatttattcggcgcaaagtgcgtcgggtgatgctgccaacttactgatttagtgtatgatggtgtttttgaggtgctccagtggcttctgtttctatcagctcctgaaaatctcgataactcaaaaaatacgcccggtagtgatcttatttcattatggtgaaagttggaacctcttacgtgccgatcaacgtctcattttcgccaaaagttggcccagggcttcccggtatcaacagggacaccaggatttatttattctgcgaagtgatcttccgtcacaggtatttattcggcgcaaagtgcgtcgggtgatgctgccaacttactgatttagtgtatgatggtgtttttgaggtgctccagtggcttctgtttctatcagggctggatgatcctccagcgcggggatctcatgctggagttcttcgcccaccccaaaaggatctaggtgaagatcctttttgataatctcatgaccaaaatcccttaacgtgagttttcgttccactgagcgtcagaccccgtagaaaagatcaaaggatcttcttgagatcctttttttctgcgcgtaatctgctgcttgcaaacaaaaaaaccaccgctaccagcggtggtttgtttgccggatcaagagctaccaactctttttccgaaggtaactggcttcagcagagcgcagataccaaatactgtccttctagtgtagccgtagttaggccaccacttcaagaactctgtagcaccgcctacatacctcgctctgctaatcctgttaccagtggctgctgccagtggcgataagtcgtgtcttaccgggttggactcaagacgatagttaccggataaggcgcagcggtcgggctgaacggggggttcgtgcacacagcccagcttggagcgaacgacctacaccgaactgagatacctacagcgtgagcattgagaaagcgccacgcttcccgaagggagaaaggcggacaggtatccggtaagcggcagggtcggaacaggagagcgcacgagggagcttccagggggaaacgcctggtatctttatagtcctgtcgggtttcgccacctctgacttgagcgtcgatttttgtgatgctcgtcaggggggcggagcctatggaaaaacgccagcaacgcggcctttttacggttcctggccttttgctggccttttgctcacatgttctttcctgcgttatcccctgattctgtggataaccgtattaccgcctttgagtgagctgataccgctcgccgcagccgaacgaccgagcgcagcgagtcagtgagcgaggaagcggaagagcgcccaatacgcaaaccgcctctccccgcgcgttggccgattcattaatgcagctggcacgacaggtttcccgactggaaagcgggcagtgagcgcaacgcaattaatgtgagttagctcactcattaggcaccccaggctttacactttatgcttccggctcgtatgttgtgtggaattgtgagcggataacaatttcacacaggaaacagctatgaccatgattacgccaagcttgcatgcctgcaggtcgactctagaggatcccc

SEQ ID NO: 47 - DNA, 8060 bp, synthetic construct
  source 1..8060: mol_type = other DNA
attaggcaccccaggctttacactttatgcttccggctcgtatgttgtgtggaattgtgagcggataacaatttcacacaggaaacagctatgaccatgattacgccaagcttgcatgcctgcaggtcgactctagaggatccccgaggggaacttgatcagaggaatacaccatggagccgatgtcagaggcgactgcgggcagatccttttgaagctgtttcacaatttctttgcccagttcgcggcggatctggaaccacttttgcatgcgatcgtcgtcagagtggttcatgtgaaaaatacactcaccatctcaatggtcatggtgaaggcctgtactggctgcgacagcatggaactcagtgcaatggctgtaaggcctgcaccaacaatgattgagcgaagctccaaaatgtcctccccgggttgatattagatttcataaatatactaaaaatcttgagagtttttccgttgaaaactaaaaagctgggaaggtgaatcgaatttcggggctttaaagcaaaaatgaacagcttggtctatagtggctaggtaccctttttgttttggacacatgtagggtggccgaaacaaagtaataggacaacaacgctcgaccgcgattatttttggagaatcatgacgagcgcgtcggcgccgtcatttaatcccggcaaggggccgggtagcgctgttggtatcgcgttgttgggctttgggacggtaggcacagaggtgatgagactgatgacagagtacggcgatgagctcgcccaccgtatcggcggcccgctcgaagtgcgaggcatcgcggtcagcgacatcagcaagccacgcgagggcgtggctcctgagttgctgaccgaggatgccttcgcacttatcgagcgggaggacgtcgatatagtggtcgaggtcatcggcggaatagagtatccacgtgaggtggtcttggcggcgttgaaagccggcaagagtgtggtgaccgccaacaaggcgttggtggcagcacactctgccgagcttgccgacgccgccgaggccgccaacgtggatctctatttcgaggccgcggtcgccggagcgatcccagtggtgggaccgctccggcgatcgctggccggggatcagatacagtcggtcatgggtattgtcaatggcaccacgaattttattctggatgccatggacagtaccggtgccgactatgctgattccctagccgaggccactcggctgggctatgctgaggcagatccgacggccgacgtggaggggcacgatgccgcctccaaggccgcgattctggccagcatagcctttcacacgcgcgtgacggcggacgatgtctattgtgagggaatttctaacatatcggcagcagacattgaggcggcccagcaggctgggcacaccatcaagctgctggcgatatgtgagaagttcaccaacaaggagggcaagtccgccatcagcgcgcgtgtgcacccgactctgttaccagtctctcaccctctggcctccgtcaataagtccttcaacgcgatcttcgtggaggcggaggcggcggggcgcctcatgttctatggcaatggagcaggaggcgccccgaccgcctccgccgtcctcggagacgtggtgggcgccgcccggaacaaggttcacggggggcgcgcaccaggggagagtacgtacgcgaacctccccatcgccgacttcggcgagaccaccacccggtaccacctcgacatggatgtcgaggaccgggtgggggtcttggcggagttggcgagtctcttcagtgagcagggcatctcgttgcgcaccatccggcaggaggagcgcgacgacgatgcccggctcattgtggtgacccacagtgcgctcgagtccgacttgagccgcactgtggagctcttgaaggccaagccggtcgtcaaggctatcaacagcgttatccggctcgagcgggattaattttactgacatggcaattgaactgaacgtcggtcgtaaggttaccgtcacggtacctggatcttctgcaaacctcggacctggctttgacactttaggtttggcactgtcggtatacgacactgtcgaagtggaaattattccatctggcttggaagtggaagtttttggcgaaggccaaggcgaagtccctcttgatggctcccacctggtggttaaagctattcgtgctggcctgaaggcagctgacgctgaagttcctggattgcgagtggtgtgccacaacaacattccgcagtctcgtggtcttggctcctctgctgcagcggcggttgctggtgttgctgcagctaatggtttggcggatttcccgctgactcaagagcagattgttcagttgtcctctgcctttgaaggccacccagataatgctgcggcttctgtgctgggtggagcagtggtgtcgtggacaaatctgtctatcgacggcaagagccagcgggtaccgagctcgaattcactggccgtcgttttacaacgtcgtgactgggaaaaccctggcgttacccaacttaatcgccttgcagcacatccccctttcgccagctggcgtaatagcgaagaggcccgcaccgatcgcccttcccaacagttgcgcagcctgaatggcgaatggcgcgataagctagcttcacgctgccgcaagcactcagggcgcaagggctgctaaaggaagcggaacacgtagaaagccagtccgcagaaacggtgctgaccccggatgaatgtcagctactgggctatctggacaagggaaaacgcaagcgcaaagagaaagcaggtagcttgcagtgggcttacatggcgatagctagactgggcggttttatggacagcaagcgaaccggaattgccagctggggcgccctctggtaaggttgggaagccctgcaaagtaaactggatggctttcttgccgccaaggatctgatggcgcaggggatcaagatctgatcaagagacaggatgaggatcgtttcgcatgattgaacaagatggattgcacgcaggttctccggccgcttgggtggagaggctattcggctatgactgggcacaacagacaatcggctgctctgatgccgccgtgttccggctgtcagcgcaggggcgcccggttctttttgtcaagaccgacctgtccggtgccctgaatgaactccaagacgaggcagcgcggctatcgtggctggccacgacgggcgttccttgcgcagctgtgctcgacgttgtcactgaagcgggaagggactggctgctattgggcgaagtgccggggcaggatctcctgtcatctcaccttgctcctgccgagaaagtatccatcatggctgatgcaatgcggcggctgcatacgcttgatccggctacctgcccattcgaccaccaagcgaaacatcgcatcgagcgagcacgtactcggatggaagccggtcttgtcgatcaggatgatctggacgaagagcatcaggggctcgcgccagccgaactgttcgccaggctcaaggcgcggatgcccgacggcgaggatctcgtcgtgacccatggcgatgcctgcttgccgaatatcatggtggaaaatggccgcttttctggattcatcgactgtggccggctgggtgtggcggaccgctatcaggacatagcgttggctacccgtgatattgctgaagagcttggcggcgaatgggctgaccgcttcctcgtgctttacggtatcgccgctcccgattcgcagcgcatcgccttctatcgccttcttgacgagttcttctgagcgggactctggggttcgctagaggatcgatcctttttaacccatcacatatacctgccgttcactattatttagtgaaatgagatattatgatattttctgaattgtgattaaaaaggcaactttatgcccatgcaacagaaactataaaaaatacagagaatgaaaagaaacagatagattttttagttctttaggcccgtagtctgcaaatccttttatgattttctatcaaacaaaagaggaaaatagaccagttgcaatccaaacgagagtctaatagaatgaggtcgaaaagtaaatcgcgcgggtttgttactgataaagcaggcaagacctaaaatgtgtaaagggcaaagtgtatactttggcgtcaccccttacatattttaggtctttttttattgtgcgtaactaacttgccatcttcaaacaggagggctggaagaagcagaccgctaacacagtacataaaaaaggagacatgaacgatgaacatcaaaaagtttgcaaaacaagcaacagtattaacctttactaccgcactgctggcaggaggcgcaactcaagcgtttgcgaaagaaacgaaccaaaagccatataaggaaacatacggcatttcccatattacacgccatgatatgctgcaaatccctgaacagcaaaaaaatgaaaaatatcaagtttctgaatttgattcgtccacaattaaaaatatctcttctgcaaaaggcctggacgtttgggacagctggccattacaaaacgctgacggcactgtcgcaaactatcacggctaccacatcgtctttgcattagccggagatcctaaaaatgcggatgacacatcgatttacatgttctatcaaaaagtcggcgaaacttctattgacagctggaaaaacgctggccgcgtctttaaagacagcgacaaattcgatgcaaatgattctatcctaaaagaccaaacacaagaatggtcaggttcagccacatttacatctgacggaaaaatccgtttattctacactgatttctccggtaaacattacggcaaacaaacactgacaactgcacaagttaacgtatcagcatcagacagctctttgaacatcaacggtgtagaggattataaatcaatctttgacggtgacggaaaaacgtatcaaaatgtacagcagttcatcgatgaaggcaactacagctcaggcgacaaccatacgctgagagatcctcactacgtagaagataaaggccacaaatacttagtatttgaagcaaacactggaactgaagatggctaccaaggcgaagaatctttatttaacaaagcatactatggcaaaagcacatcattcttccgtcaagaaagtcaaaaacttctgcaaagcgataaaaaacgcacggctgagttagcaaacggcgctctcggtatgattgagctaaacgatgattacacactgaaaaaagtgatgaaaccgctgattgcatctaacacagtaacagatgaaattgaacgcgcgaacgtctttaaaatgaacggcaaatggtacctgttcactgactcccgcggatcaaaaatgacgattgacggcattacgtctaacgatatttacatgcttggttatgtttctaattctttaactggcccatacaagccgctgaacaaaactggccttgtgttaaaaatggatcttgatcctaacgatgtaacctttacttactcacacttcgctgtacctcaagcgaaaggaaacaatgtcgtgattacaagctatatgacaaacagaggattctacgcagacaaacaatcaacgtttgcgccgagcttcctgctgaacatcaaaggcaagaaaacatctgttgtcaaagacagcatccttgaacaaggacaattaacagttaacaaataaaaacgcaaaagaaaatgccgatgggtaccgagcgaaatgaccgaccaagcgacgcccaacctgccatcacgagatttcgattccaccgccgccttctatgaaaggttgggcttcggaatcgttttccgggacgccctcgcggacgtgctcatagtccacgacgcccgtgattttgtagccctggccgacggccagcaggtaggccgacaggctcatgccggccgccgccgccttttcctcaatcgctcttcgttcgtctggaaggcagtacaccttgataggtgggctgcccttcctggttggcttggtttcatcagccatccgcttgccctcatctgttacgccggcggtagccggccagcctcgcagagcaggattcccgttgagcaccgccaggtgcgaataagggacagtgaagaaggaacacccgctcgcgggtgggcctacttcacctatcctgccccgctgacgccgttggatacaccaaggaaagtctacacgaaccctttggcaaaatcctgtatatcgtgcgaaaaaggatggatataccgaaaaaatcgctataatgaccccgaagcagggttatgcagcggaaaagcgctgcttccctgctgttttgtggaatatctaccgactggaaacaggcaaatgcaggaaattactgaactgaggggacaggcgagagacgatgccaaagagctcctgaaaatctcgataactcaaaaaatacgcccggtagtgatcttatttcattatggtgaaagttggaacctcttacgtgccgatcaacgtctcattttcgccaaaagttggcccagggcttcccggtatcaacagggacaccaggatttatttattctgcgaagtgatcttccgtcacaggtatttattcggcgcaaagtgcgtcgggtgatgctgccaacttactgatttagtgtatgatggtgtttttgaggtgctccagtggcttctgtttctatcagctcctgaaaatctcgataactcaaaaaatacgcccggtagtgatcttatttcattatggtgaaagttggaacctcttacgtgccgatcaacgtctcattttcgccaaaagttggcccagggcttcccggtatcaacagggacaccaggatttatttattctgcgaagtgatcttccgtcacaggtatttattcggcgcaaagtgcgtcgggtgatgctgccaacttactgatttagtgtatgatggtgtttttgaggtgctccagtggcttctgtttctatcagggctggatgatcctccagcgcggggatctcatgctggagttcttcgcccaccccaaaaggatctaggtgaagatcctttttgataatctcatgaccaaaatcccttaacgtgagttttcgttccactgagcgtcagaccccgtagaaaagatcaaaggatcttcttgagatcctttttttctgcgcgtaatctgctgcttgcaaacaaaaaaaccaccgctaccagcggtggtttgtttgccggatcaagagctaccaactctttttccgaaggtaactggcttcagcagagcgcagataccaaatactgtccttctagtgtagccgtagttaggccaccacttcaagaactctgtagcaccgcctacatacctcgctctgctaatcctgttaccagtggctgctgccagtggcgataagtcgtgtcttaccgggttggactcaagacgatagttaccggataaggcgcagcggtcgggctgaacggggggttcgtgcacacagcccagcttggagcgaacgacctacaccgaactgagatacctacagcgtgagcattgagaaagcgccacgcttcccgaagggagaaaggcggacaggtatccggtaagcggcagggtcggaacaggagagcgcacgagggagcttccagggggaaacgcctggtatctttatagtcctgtcgggtttcgccacctctgacttgagcgtcgatttttgtgatgctcgtcaggggggcggagcctatggaaaaacgccagcaacgcggcctttttacggttcctggccttttgctggccttttgctcacatgttctttcctgcgttatcccctgattctgtggataaccgtattaccgcctttgagtgagctgataccgctcgccgcagccgaacgaccgagcgcagcgagtcagtgagcgaggaagcggaagagcgcccaatacgcaaaccgcctctccccgcgcgttggccgattcattaatgcagctggcacgacaggtttcccgactggaaagcgggcagtgagcgcaacgcaattaatgtgagttagctcactc

SEQ ID NO: 48 - DNA, 21 bp, synthetic construct
  source 1..21: mol_type = other DNA
gccacattccacccattactg

SEQ ID NO: 49 - DNA, 20 bp, synthetic construct
  source 1..20: mol_type = other DNA
ggacgaaacggttccaaagg

SEQ ID NO: 50 - DNA, 20 bp, synthetic construct
  source 1..20: mol_type = other DNA
cgtccaggagttcctctacg

SEQ ID NO: 51 - DNA, 20 bp, synthetic construct
  source 1..20: mol_type = other DNA
cgcgtcagcgtgcttataac

SEQ ID NO: 52 - DNA, 1350 bp, synthetic construct
  source 1..1350: mol_type = other DNA
atgtctgaaattgttgtctccaaatttggcggtaccagcgtagctgattttgacgccatgaaccgcagcgctgatattgtgctttctgatgccaacgtgcgtttagttgtcctctcggcttctgctggtatcactaatctgctggtcgctttagctgaaggactggaacctggcgagcgattcgaaaaactcgacgctatccgcaacatccagtttgccattctggaacgtctgcgttacccgaacgttatccgtgaagagattgaacgtctgctggagaacattactgttctggcagaagcggcggcgctggcaacgtctccggcgctgacagatgagctggtcagccacggcgagctgatgtcgaccctgctgtttgttgagatcctgcgcgaacgcgatgttcaggcacagtggtttgatgtacgtaaagtgatgcgtaccaacgaccgatttggtcgtgcagagccagatatagccgcgctggcggaactggccgcgctgcagctgctcccacgtctcaatgaaggcttagtgatcacccagggatttatcggtagcgaaaataaaggtcgtacaacgacgcttggccgtggaggcagcgattatacggcagccttgctggcggaggctttacacgcatctcgtgttgatatctggaccgacgtcccgggcatctacaccaccgatccacgcgtagtttccgcagcaaaacgcattgatgaaatcgcgtttgccgaagcggcagagatggcaaggtttggtgcaaaagtactgcatccggcaacgttgctacccgcagtacgcagcgatatcccggtctttgtcggctccagcaaagacccacgcgcaggtggtacgctggtgtgcaataaaactgaaaatccgccgctgttccgcgctctggcgcttcgtcgcaatcagactctgctcactttgcacagcctgaatatgctgcattctcgcggtttcctcgcggaagttttcggcatcctcgcgcggcataatatttcggtagacttaatcaccacgtcagaagtgagcgtggcattaacccttgataccaccggttcaacctccactggcgatacgttgctgacgcaatctctgctgatggagctttccgcactgtgtcgggtggaggtggaagaaggtctggcgctggtcgcgttgattggcaatgacctgtcaaaagcctgcggcgttggcaaagaggtattcggcgtactggaaccgttcaacattcgcatgatttgttatggcgcatccagccataacctgtgcttcctggtgcccggcgaagatgccgagcaggtggtgcaaaaactgcatagtaatttgtttgagtaa

SEQ ID NO: 53 - DNA, 1350 bp, synthetic construct
  source 1..1350: mol_type = other DNA
atgtctgaaattgttgtttctaaatttggtggtacttctgttgctgattttgatgctatgaatagatctgctgatattgttttatctgatgctaatgttagattagttgttttatctgcttctgctggtattactaatttattagttgctttagctgaaggtttagaacctggtgaaagatttgaaaaattagatgctattagaaatattcaatttgctattttagaaagattaagatatcctaatgttattagagaagaaattgaaagattattagaaaatattactgttttagctgaagctgctgctttagctacttctcctgctttaactgatgaattagtttctcatggtgaattaatgtctactttattatttgttgaaattttaagagaaagagatgttcaagctcaatggtttgatgttagaaaagttatgagaactaatgatagatttggtagagctgaacctgatattgctgctttagctgaattagctgctttacaattattacctagattaaatgaaggtttagttattactcaaggttttattggttctgaaaataaaggtagaactactactttaggtagaggtggttctgattatactgctgctttattagctgaagctttacatgcttctagagttgatatttggactgatgttcctggtatttatactactgatcctagagttgtttctgctgctaaaagaattgatgaaattgcttttgctgaagctgctgaaatggctagatttggtgctaaagttttacatcctgctactttattacctgctgttagatctgatattcctgtttttgttggttcttctaaagatcctagagctggtggtactttagtttgtaataaaactgaaaatcctcctttatttagagctttagctttaagaagaaatcaaactttattaactttacattctttaaatatgttacattctagaggttttttagctgaagtttttggtattttagctagacataatatttctgttgatttaattactacttctgaagtttctgttgctttaactttagatactactggttctacttctactggtgatactttattaactcaatctttattaatggaattatctgctttatgtagagttgaagttgaagaaggtttagctttagttgctttaattggtaatgatttatctaaagcttgtggtgttggtaaagaagtttttggtgttttagaaccttttaatattagaatgatttgttatggtgcttcttctcataatttatgttttttagttcctggtgaagatgctgaacaagttgttcaaaaattacattctaatttatttgaataa

SEQ ID NO: 54 - DNA, 2727 bp, synthetic construct
  source 1..2727: mol_type = other DNA
ccgtcttccgctcttcccttgtgccaaggctgaaaatggatcccctgacacgaggtagttatgtctgaaattgttgtctccaaatttggcggtaccagcgtagctgattttgacgccatgaaccgcagcgctgatattgtgctttctgatgccaacgtgcgtttagttgtcctctcggcttctgctggtatcactaatctgctggtcgctttagctgaaggactggaacctggcgagcgattcgaaaaactcgacgctatccgcaacatccagtttgccattctggaacgtctgcgttacccgaacgttatccgtgaagagattgaacgtctgctggagaacattactgttctggcagaagcggcggcgctggcaacgtctccggcgctgacagatgagctggtcagccacggcgagctgatgtcgaccctgctgtttgttgagatcctgcgcgaacgcgatgttcaggcacagtggtttgatgtacgtaaagtgatgcgtaccaacgaccgatttggtcgtgcagagccagatatagccgcgctggcggaactggccgcgctgcagctgctcccacgtctcaatgaaggcttagtgatcacccagggatttatcggtagcgaaaataaaggtcgtacaacgacgcttggccgtggaggcagcgattatacggcagccttgctggcggaggctttacacgcatctcgtgttgatatctggaccgacgtcccgggcatctacaccaccgatccacgcgtagtttccgcagcaaaacgcattgatgaaatcgcgtttgccgaagcggcagagatggcaaggtttggtgcaaaagtactgcatccggcaacgttgctacccgcagtacgcagcgatatcccggtctttgtcggctccagcaaagacccacgcgcaggtggtacgctggtgtgcaataaaactgaaaatccgccgctgttccgcgctctggcgcttcgtcgcaatcagactctgctcactttgcacagcctgaatatgctgcattctcgcggtttcctcgcggaagttttcggcatcctcgcgcggcataatatttcggtagacttaatcaccacgtcagaagtgagcgtggcattaacccttgataccaccggttcaacctccactggcgatacgttgctgacgcaatctctgctgatggagctttccgcactgtgtcgggtggaggtggaagaaggtctggcgctggtcgcgttgattggcaatgacctgtcaaaagcctgcggcgttggcaaagaggtattcggcgtactggaaccgttcaacattcgcatgatttgttatggcgcatccagccataacctgtgcttcctggtgcccggcgaagatgccgagcaggtggtgcaaaaactgcatagtaatttgtttgagtaagaagttcctatactttctagagaataggaacttcggaataggaacttcaagatccccttattagaagaactcgtcaagaaggcgatagaaggcgatgcgctgcgaatcgggagcggcgataccgtaaagcacgaggaagcggtcagcccattcgccgccaagctcttcagcaatatcacgggtagccaacgctatgtcctgatagcggtccgccacacccagccggccacagtcgatgaatccagaaaagcggccattttccaccatgatattcggcaagcaggcatcgccatgggtcacgacgagatcctcgccgtcgggcatgcgcgccttgagcctggcgaacagttcggctggcgcgagcccctgatgctcttcgtccagatcatcctgatcgacaagaccggcttccatccgagtacgtgctcgctcgatgcgatgtttcgcttggtggtcgaatgggcaggtagccggatcaagcgtatgcagccgccgcattgcatcagccatgatggatactttctcggcaggagcaaggtgagatgacaggagatcctgccccggcacttcgcccaatagcagccagtcccttcccgcttcagtgacaacgtcgagcacagctgcgcaaggaacgcccgtcgtggccagccacgatagccgcgctgcctcgtcctgcagttcattcagggcaccggacaggtcggtcttgacaaaaagaaccgggcgcccctgcgctgacagccggaacacggcggcatcagagcagccgattgtctgttgtgcccagtcatagccgaatagcctctccacccaagcggccggagaacctgcgtgcaatccatcttgttcaatcatgcgaaacgatcctcatcctgtctcttgatcagatcttgatcccctgcgccatcagatccttggcggcaagaaagccatccagtttactttgcagggcttcccaaccttaccagagggcgccccagctggcaattccggttcgcttgctgtccataaaaccgcccagtctagctatcgccatgtaagcccactgcaagctacctgctttctctttgcgcttgcgttttcccttgtccagatagcccagtagctgacattcatccggggtcagcaccgtttctgcggactggctttctacgtgttccgcttcctttagcagcccttgcgccctgagtgcttgcggcagcgtgagcttcaaaagcgctctgaagttcctatactttctagagaataggaacttcgatactgtatggcctggaagctatatttcgggccgtattgattttcttgtcactatgctca

SEQ ID NO: 55 - DNA, 2727 bp, synthetic construct
  source 1..2727: mol_type = other DNA
ccgtcttccgctcttcccttgtgccaaggctgaaaatggatcccctgacacgaggtagttatgtctgaaattgttgtttctaaatttggtggtacttctgttgctgattttgatgctatgaatagatctgctgatattgttttatctgatgctaatgttagattagttgttttatctgcttctgctggtattactaatttattagttgctttagctgaaggtttagaacctggtgaaagatttgaaaaattagatgctattagaaatattcaatttgctattttagaaagattaagatatcctaatgttattagagaagaaattgaaagattattagaaaatattactgttttagctgaagctgctgctttagctacttctcctgctttaactgatgaattagtttctcatggtgaattaatgtctactttattatttgttgaaattttaagagaaagagatgttcaagctcaatggtttgatgttagaaaagttatgagaactaatgatagatttggtagagctgaacctgatattgctgctttagctgaattagctgctttacaattattacctagattaaatgaaggtttagttattactcaaggttttattggttctgaaaataaaggtagaactactactttaggtagaggtggttctgattatactgctgctttattagctgaagctttacatgcttctagagttgatatttggactgatgttcctggtatttatactactgatcctagagttgtttctgctgctaaaagaattgatgaaattgcttttgctgaagctgctgaaatggctagatttggtgctaaagttttacatcctgctactttattacctgctgttagatctgatattcctgtttttgttggttcttctaaagatcctagagctggtggtactttagtttgtaataaaactgaaaatcctcctttatttagagctttagctttaagaagaaatcaaactttattaactttacattctttaaatatgttacattctagaggttttttagctgaagtttttggtattttagctagacataatatttctgttgatttaattactacttctgaagtttctgttgctttaactttagatactactggttctacttctactggtgatactttattaactcaatctttattaatggaattatctgctttatgtagagttgaagttgaagaaggtttagctttagttgctttaattggtaatgatttatctaaagcttgtggtgttggtaaagaagtttttggtgttttagaaccttttaatattagaatgatttgttatggtgcttcttctcataatttatgttttttagttcctggtgaagatgctgaacaagttgttcaaaaattacattctaatttatttgaataagaagttcctatactttctagagaataggaacttcggaataggaacttcaagatccccttattagaagaactcgtcaagaaggcgatagaaggcgatgcgctgcgaatcgggagcggcgataccgtaaagcacgaggaagcggtcagcccattcgccgccaagctcttcagcaatatcacgggtagccaacgctatgtcctgatagcggtccgccacacccagccggccacagtcgatgaatccagaaaagcggccattttccaccatgatattcggcaagcaggcatcgccatgggtcacgacgagatcctcgccgtcgggcatgcgcgccttgagcctggcgaacagttcggctggcgcgagcccctgatgctcttcgtccagatcatcctgatcgacaagaccggcttccatccgagtacgtgctcgctcgatgcgatgtttcgcttggtggtcgaatgggcaggtagccggatcaagcgtatgcagccgccgcattgcatcagccatgatggatactttctcggcaggagcaaggtgagatgacaggagatcctgccccggcacttcgcccaatagcagccagtcccttcccgcttcagtgacaacgtcgagcacagctgcgcaaggaacgcccgtcgtggccagccacgatagccgcgctgcctcgtcctgcagttcattcagggcaccggacaggtcggtcttgacaaaaagaaccgggcgcccctgcgctgacagccggaacacggcggcatcagagcagccgattgtctgttgtgcccagtcatagccgaatagcctctccacccaagcggccggagaacctgcgtgcaatccatcttgttcaatcatgcgaaacgatcctcatcctgtctcttgatcagatcttgatcccctgcgccatcagatccttggcggcaagaaagccatccagtttactttgcagggcttcccaaccttaccagagggcgccccagctggcaattccggttcgcttgctgtccataaaaccgcccagtctagctatcgccatgtaagcccactgcaagctacctgctttctctttgcgcttgcgttttcccttgtccagatagcccagtagctgacattcatccggggtcagcaccgtttctgcggactggctttctacgtgttccgcttcctttagcagcccttgcgccctgagtgcttgcggcagcgtgagcttcaaaagcgctctgaagttcctatactttctagagaataggaacttcgatactgtatggcctggaagctatatttcgggccgtattgattttcttgtcactatgctca

SEQ ID NO: 56 - DNA, 6329 bp, synthetic construct
  source 1..6329: mol_type = other DNA
catcgatttattatgacaacttgacggctacatcattcactttttcttcacaaccggcacggaactcgctcgggctggccccggtgcattttttaaatacccgcgagaaatagagttgatcgtcaaaaccaacattgcgaccgacggtggcgataggcatccgggtggtgctcaaaagcagcttcgcctggctgatacgttggtcctcgcgccagcttaagacgctaatccctaactgctggcggaaaagatgtgacagacgcgacggcgacaagcaaacatgctgtgcgacgctggcgatatcaaaattgctgtctgccaggtgatcgctgatgtactgacaagcctcgcgtacccgattatccatcggtggatggagcgactcgttaatcgcttccatgcgccgcagtaacaattgctcaagcagatttatcgccagcagctccgaatagcgcccttccccttgcccggcgttaatgatttgcccaaacaggtcgctgaaatgcggctggtgcgcttcatccgggcgaaagaaccccgtattggcaaatattgacggccagttaagccattcatgccagtaggcgcgcggacgaaagtaaacccactggtgataccattcgcgagcctccggatgacgaccgtagtgatgaatctctcctggcgggaacagcaaaatatcacccggtcggcaaacaaattctcgtccctgatttttcaccaccccctgaccgcgaatggtgagattgagaatataacctttcattcccagcggtcggtcgataaaaaaatcgagataaccgttggcctcaatcggcgttaaacccgccaccagatgggcattaaacgagtatcccggcagcaggggatcattttgcgcttcagccatacttttcatactcccgccattcagagaagaaaccaattgtccatattgcatcagacattgccgtcactgcgtcttttactggctcttctcgctaaccaaaccggtaaccccgcttattaaaagcattctgtaacaaagcgggaccaaagccatgacaaaaacgcgtaacaaaagtgtctataatcacggcagaaaagtccacattgattatttgcacggcgtcacactttgctatgccatagcatttttatccataagattagcggatcctacctgacgctttttatcgcaactctctactgtttctccatacccgtttttttgggaattcgagctctaaggaggttataaaaaatggatattaatactgaaactgagatcaagcaaaagcattcactaaccccctttcctgttttcctaatcagcccggcatttcgcgggcgatattttcacagctatttcaggagttcagccatgaacgcttattacattcaggatcgtcttgaggctcagagctgggcgcgtcactaccagcagctcgcccgtgaagagaaagaggcagaactggcagacgacatggaaaaaggcctgccccagcacctgtttgaatcgctatgcatcgatcatttgcaacgccacggggccagcaaaaaatccattacccgtgcgtttgatgacgatgttgagtttcaggagcgcatggcagaacacatccggtacatggttgaaaccattgctcaccaccaggttgatattgattcagaggtataaaacgaatgagtactgcactcgcaacgctggctgggaagctggctgaacgtgtcggcatggattctgtcgacccacaggaactgatcaccactcttcgccagacggcatttaaaggtgatgccagcgatgcgcagttcatcgcattactgatcgttgccaaccagtacggccttaatccgtggacgaaagaaatttacgcctttcctgataagcagaatggcatcgttccggtggtgggcgttgatggctggtcccgcatcatcaatgaaaaccagcagtttgatggcatggactttgagcaggacaatgaatcctgtacatgccggatttaccgcaaggaccgtaatcatccgatctgcgttaccgaatggatggatgaatgccgccgcgaaccattcaaaactcgcgaaggcagagaaatcacggggccgtggcagtcgcatcccaaacggatgttacgtcataaagccatgattcagtgtgcccgtctggccttcggatttgctggtatctatgacaaggatgaagccgagcgcattgtcgaaaatactgcatacactgcagaacgtcagccggaacgcgacatcactccggttaacgatgaaaccatgcaggagattaacactctgctgatcgccctggataaaacatgggatgacgacttattgccgctctgttcccagatatttcgccgcgacattcgtgcatcgtcagaactgacacaggccgaagcagtaaaagctcttggattcctgaaacagaaagccgcagagcagaaggtggcagcatgacaccggacattatcctgcagcgtaccgggatcgatgtgagagctgtcgaacagggggatgatgcgtggcacaaattacggctcggcgtcatcaccgcttcagaagttcacaacgtgatagcaaaaccccgctccggaaagaagtggcctgacatgaaaatgtcctacttccacaccctgcttgctgaggtttgcaccggtgtggctccggaagttaacgctaaagcactggcctggggaaaacagtacgagaacgacgccagaaccctgtttgaattcacttccggcgtgaatgttactgaatccccgatcatctatcgcgacgaaagtatgcgtaccgcctgctctcccgatggtttatgcagtgacggcaacggccttgaactgaaatgcccgtttacctcccgggatttcatgaagttccggctcggtggtttcgaggccataaagtcagcttacatggcccaggtgcagtacagcatgtgggtgacgcgaaaaaatgcctggtactttgccaactatgacccgcgtatgaagcgtgaaggcctgcattatgtcgtgattgagcgggatgaaaagtacatggcgagttttgacgagatcgtgccggagttcatcgaaaaaatggacgaggcactggctgaaattggttttgtatttggggagcaatggcgatgacgcatcctcacgataatatccgggtaggcgcaatcactttcgtctactccgttacaaagcgaggctgggtatttcccggcctttctgttatccgaaatccactgaaagcacagcggctggctgaggagataaataataaacgaggggctgtatgcacaaagcatcttctgttgagttaagaacgagtatcgagatggcacatagccttgctcaaattggaatcaggtttgtgccaataccagtagaaacagacgaagaatccatgggtatggacagttttccctttgatatgtaacggtgaacagttgttctacttttgtttgttagtcttgatgcttcactgatagatacaagagccataagaacctcagatccttccgtatttagccagtatgttctctagtgtggttcgttgtttttgcgtgagccatgagaacgaaccattgagatcatacttactttgcatgtcactcaaaaattttgcctcaaaactggtgagctgaatttttgcagttaaagcatcgtgtagtgtttttcttagtccgttacgtaggtaggaatctgatgtaatggttgttggtattttgtcaccattcatttttatctggttgttctcaagttcggttacgagatccatttgtctatctagttcaacttggaaaatcaacgtatcagtcgggcggcctcgcttatcaaccaccaatttcatattgctgtaagtgtttaaatctttacttattggtttcaaaacccattggttaagccttttaaactcatggtagttattttcaagcattaacatgaacttaaattcatcaaggctaatctctatatttgccttgtgagttttcttttgtgttagttcttttaataaccactcataaatcctcatagagtatttgttttcaaaagacttaacatgttccagattatattttatgaatttttttaactggaaaagataaggcaatatctcttcactaaaaactaattctaatttttcgcttgagaacttggcatagtttgtccactggaaaatctcaaagcctttaaccaaaggattcctgatttccacagttctcgtcatcagctctctggttgctttagctaatacaccataagcattttccctactgatgttcatcatctgagcgtattggttataagtgaacgataccgtccgttctttccttgtagggttttcaatcgtggggttgagtagtgccacacagcataaaattagcttggtttcatgctccgttaagtcatagcgactaatcgctagttcatttgctttgaaaacaactaattcagacatacatctcaattggtctaggtgattttaatcactataccaattgagatgggctagtcaatgataattactagtccttttcctttgagttgtgggtatctgtaaattctgctagacctttgctggaaaacttgtaaattctgctagaccctctgtaaattccgctagacctttgtgtgttttttttgtttatattcaagtggttataatttatagaataaagaaagaataaaaaaagataaaaagaatagatcccagccctgtgtataactcactactttagtcagttccgcagtattacaaaaggatgtcgcaaacgctgtttgctcctctacaaaacagaccttaaaaccctaaaggcttaagtagcaccctcgcaagctcggttgcggccgcaatcgggcaaatcgctgaatattccttttgtctccgaccatcaggcacctgagtcgctgtctttttcgtgacattcagttcgctgcgctcacggctctggcagtgaatgggggtaaatggcactacaggcgccttttatggattcatgcaaggaaactacccataatacaagaaaagcccgtcacgggcttctcagggcgttttatggcgggtctgctatgtggtgctatctgactttttgctgttcagcagttcctgccctctgattttccagtctgaccacttcggattatcccgtgacaggtcattcagactggctaatgcacccagtaaggcagcggtatcatcaacggggtctgacgctcagtggaacgaaaactcacgttaagggattttggtcatgagattatcaaaaaggatcttcacctagatccttttaaattaaaaatgaagttttaaatcaatctaaagtatatatgagtaaacttggtctgacagttaccaatgcttaatcagtgaggcacctatctcagcgatctgtctatttcgttcatccatagttgcctgactccccgtcgtgtagataactacgatacgggagggcttaccatctggccccagtgctgcaatgataccgcgagacccacgctcaccggctccagatttatcagcaataaaccagccagccggaagggccgagcgcagaagtggtcctgcaactttatccgcctccatccagtctattaattgttgccgggaagctagagtaagtagttcgccagttaatagtttgcgcaacgttgttgccattgctacaggcatcgtggtgtcacgctcgtcgtttggtatggcttcattcagctccggttcccaacgatcaaggcgagttacatgatcccccatgttgtgcaaaaaagcggttagctccttcggtcctccgatcgttgtcagaagtaagttggccgcagtgttatcactcatggttatggcagcactgcataattctcttactgtcatgccatccgtaagatgcttttctgtgactggtgagtactcaaccaagtcattctgagaatagtgtatgcggcgaccgagttgctcttgcccggcgtcaatacgggataataccgcgccacatagcagaactttaaaagtgctcatcattggaaaacgttcttcggggcgaaaactctcaaggatcttaccgctgttgagatccagttcgatgtaacccactcgtgcacccaactgatcttcagcatcttttactttcaccagcgtttctgggtgagcaaaaacaggaaggcaaaatgccgcaaaaaagggaataagggcgacacggaaatgttgaatactcatactcttcctttttcaatattattgaagcatttatcagggttattgtctcatgagcggatacatatttgaatgtatttagaaaaataaacaaataggggttccgcgcacatttccccgaaaagtgccacctg

SEQ ID NO: 57 - DNA, 20 bp, synthetic construct
  source 1..20: mol_type = other DNA
gttgtcaccagaagcgttcg

SEQ ID NO: 58 - DNA, 21 bp, synthetic construct
  source 1..21: mol_type = other DNA
tcgataattaattagagatgc

SEQ ID NO: 59 - DNA, 9332 bp, synthetic construct
  source 1..9332: mol_type = other DNA
gagacacaacgtggctttgttgaataaatcgaacttttgctgagttgaaggatcagatcacgcatcttcccgacaacgcagaccgttccgtggcaaagcaaaagttcaaaatcaccaactggtccacctacaacaaagctctcatcaaccgtggctccctcactttctggctggatgatggggcgattcaggcctggtatgagtcagcaacaccttcttcacgaggcagacctcagcgccacaggtgcggttgctggcgctaaccgtttttatcaggctctgggaggcagaataaatgatcatatcgtcaattattacctccacggggagagcctgagcaaactggcctcaggcatttgagaagcacacggtcacactgcttccggtagtcaataaaccggtaaaccagcaatagacataagcggctatttaacgaccctgccctgaaccgacgaccgggtcgaatttgctttcgaatttctgccattcatccgcttattatcacttattcaggcgtagcaaccaggcgtttaagggcaccaataactgccttaaaaaaattacgccccgccctgccactcatcgcagtactgttgtaattcattaagcattctgccgacatggaagccatcacaaacggcatgatgaacctgaatcgccagcggcatcagcaccttgtcgccttgcgtataatatttgcccatggtgaaaacgggggcgaagaagttgtccatattggccacgtttaaatcaaaactggtgaaactcacccagggattggctgagacgaaaaacatattctcaataaaccctttagggaaataggccaggttttcaccgtaacacgccacatcttgcgaatatatgtgtagaaactgccggaaatcgtcgtggtattcactccagagcgatgaaaacgtttcagtttgctcatggaaaacggtgtaacaagggtgaacactatcccatatcaccagctcaccgtctttcattgccatacggaattccggatgagcattcatcaggcgggcaagaatgtgaataaaggccggataaaacttgtgcttatttttctttacggtctttaaaaaggccgtaatatccagctgaacggtctggttataggtacattgagcaactgactgaaatgcctcaaaatgttctttacgatgccattgggatatatcaacggtggtatatccagtgatttttttctccattttagcttccttagctcctgaaaatctcgataactcaaaaaatacgcccggtagtgatcttatttcattatggtgaaagttggaacctcttacgtgccgatcaacgtctcattttcgccaaaagttggcccagggcttcccggtatcaacagggacaccaggatttatttattctgcgaagtgatcttccgtcacaggtatttattcggcgcaaagtgcgtcgggtgatgctgccaacttactgatttagtgtatgatggtgtttttgaggtgctccagtggcttctgtttctatcagctgtccctcctgttcagctactgacggggtggtgcgtaacggcaaaagcaccgccggacatcagcgcttgtttcggcgtgggtatggtggcaggccccgtggccgggggactgttgggcgcctgtagtgccatttacccccattcactgccagagccgtgagcgcagcgaactgaatgtcacgaaaaagacagcgactcaggtgcctgatggtcggagacaaaaggaatattcagcgatttgcccgagcttgcgagggtgctacttaagcctttagggttttaaggtctgttttgtagaggagcaaacagcgtttgcgacatccttttgtaatactgcggaactgactaaagtagtgagttatacacagggctgggatctattctttttatctttttttattctttctttattctataaattataaccacttgaatataaacaaaaaaaacacacaaaggtctagcggaatttacagagggtctagcagaatttacaagttttccagcaaaggtctagcagaatttacagatacccacaactcaaaggaaaaggactagtaattatcattgactagcccatctcaattggtatagtgattaaaatcacctagaccaattgagatgtatgtctgaattagttgttttcaaagcaaatgaactagcgattagtcgctatgacttaacggagcatgaaaccaagctaattttatgctgtgtggcactactcaaccccacgattgaaaaccctacaaggaaagaacggacggtatcgttcacttataaccaatacgttcagatgatgaacatcagtagggaaaatgcttatggtgtattagctaaagcaaccagagagctgatgacgagaactgtggaaatcaggaatcctttggttaaaggctttgagattttccagtggacaaactatgccaagttctcaagcgaaaaattagaattagtttttagtgaagagatattgccttatcttttccagttaaaaaaattcataaaatataatctggaacatgttaagtcttttgaaaacaaatactctatgaggatttatgagtggttattaaaagaactaacacaaaagaaaactcacaaggcaaatatagagattagccttgatgaatttaagttcatgttaatgcttgaaaataactaccatgagtttaaaaggcttaaccaatgggttttgaaaccaataagtaaagatttaaacacttacagcaatatgaaattggtggttgataagcgaggccgcccgactgatacgttgattttccaagttgaactagatagacaaatggatctcgtaaccgaacttgagaacaaccagataaaaatgaatggtgacaaaataccaacaaccattacatcagattcctacctacataacggactaagaaaaacactacacgatgctttaactgcaaaaattcagctcaccagttttgaggcaaaatttttgagtgacatgcaaagtaagtatgatctcaatggttcgttctcatggctcacgcaaaaacaacgaaccacactagagaacatactggctaaatacggaaggatctgaggttcttatggctcttgtatctatcagtgaagcatcaagactaacaaacaaaagtagaacaactgttcaccgttacatatcaaagggaaaactgtccatatgcacagatgaaaacggtgtaaaaaagatagatacatcagagcttttacgagtttttggtgcatttaaagctgttcaccatgaacagatcgacaatgtaacagatgaacagcatgtaacacctaatagaacaggtgaaaccagtaaaacaaagcaactagaacatgaaattgaacacctgagacaacttgttacagctcaacagtcacacatagacagcctgaaacaggcgatgctgcttatcgaatcaaagctgccgacaacacgggagccagtgacgcctcccgtggggaaaaaatcatggcaattctggaagaaatagcgcctgtttcgtttcaggcaggttatcagggagtgtcagcgtcctgcggttctccggggcgttcgggtcatgcagcccgtaatggtgatttaccagcgtctgccaggcatcaattctaggcctgtctgcgcggtcgtagtacggctggaggcgttttccggtctgtagctccatgttcggaatgacaaaattcagctcaagccgtcccttgtcctggtgctccacccacaggatgctgtactgatttttttcgagaccgggcatcagtacacgctcaaagctcgccatcactttttcacgtcctcccggcggcagctccttctccgcgaacgacagaacaccggacgtgtatttcttcgcaaatggcgtggcatcgatgagttcccggacttcttccggattaccctgaagcaccgttgcgccttcgcggttacgctccctccccagcaggtaatcaaccggaccactgccaccaccttttcccctggcatgaaatttaactatcatcccgcgccccctgttccctgacagccagacgcagccggcgcagctcatccccgatggccatcagtgcggccaccacctgaacccggtcaccggaagaccactgcccgctgttcaccttacgggctgtctgattcaggttatttccgatggcggccagctgacgcagtaacggcggtgccagtgtcggcagttttccggaacgggcaaccggctcccccaggcagacccgccgcatccataccgccagttgtttaccctcacagcgttcaagtaaccgggcatgttcatcatcagtaacccgtattgtgagcatcctctcgcgtttcatcggtatcattaccccatgaacagaaatcccccttacacggaggcatcagtgactaaacggggtctgacgctcagtggaacgaaaactcacgttaagggattttggtcatgagattatcaaaaaggatcttcacctagatccttttaaattaaaaatgaagttttaaatcaatctaaagtatatatgagtaaacttggtctgacagttaccaatgcttaatcagtgaggcacctatctcagcgatctgtctatttcgttcatccatagttgcctgactccccgtcgtgtagataactacgatacgggagggcttaccatctggccccagtgctgcaatgataccgcgagacccacgctcaccggctccagatttatcagcaataaaccagccagccggaagggccgagcgcagaagtggtcctgcaactttatccgcctccatccagtctattaattgttgccgggaagctagagtaagtagttcgccagttaatagtttgcgcaacgttgttgccattgctgcaggcatcgtggtgtcacgctcgtcgtttggtatggcttcattcagctccggttcccaacgatcaaggcgagttacatgatcccccatgttgtgcaaaaaagcggttagctccttcggtcctccgatcgttgtcagaagtaagttggccgcagtgttatcactcatggttatggcagcactgcataattctcttactgtcatgccatccgtaagatgcttttctgtgactggtgagtactcaaccaagtcattctgagaatagtgtatgcggcgaccgagttgctcttgcccggcgtcaacacgggataataccgcgccacatagcagaactttaaaagtgctcatcattggaaaacgttcttcggggcgaaaactctcaaggatcttaccgctgttgagatccagttcgatgtaacccactcgtgcacccaactgatcttcagcatcttttactttcaccagcgtttctgggtgagcaaaaacaggaaggcaaaatgccgcaaaaaagggaataagggcgacacggaaatgttgaatactcatactcttcctttttcaatattattgaagcatttatcagggttattgtctcatgagcggatacatatttgaatgtatttagaaaaataaacaaataggggttccgcgcacatttccccgaaaagtgccacctgacgtctaagaaaccattattatcatgacattaacctataaaaataggcgtatcacgaggccctttcgtcttcaagaattttataaaccgtggagcgggcaatactgagctgatgagcaatttccgttgcaccagtgcccttctgatgaagcgtcagcacgacgttcctgtccacggtacgcctgcggccaaatttgattcctttcagctttgcttcctgtcggccctcattcgtgcgctctaggatcctctacgccggacgcatcgtggccggcatcaccggcgctgaggtctgcctcgtgaagaaggtgttgctgactcataccaggcctgaatcgccccatcatccagccagaaagtgagggagccacggttgatgagagctttgttgtaggtggaccagttggtgattttgaacttttgctttgccacggaacggtctgcgttgtcgggaagatgcgtgatctgatccttcaactcagcaaaagttcgatttattcaacaaagccgccgtcccgtcaagtcagcgtaatgctctgccagtgttacaaccaattaaccaattctgattagaaaaactcatcgagcatcaaatgaaactgcaatttattcatatcaggattatcaataccatatttttgaaaaagccgtttctgtaatgaaggagaaaactcaccgaggcagttccataggatggcaagatcctggtatcggtctgcgattccgactcgtccaacatcaatacaacctattaatttcccctcgtcaaaaataaggttatcaagtgagaaatcaccatgagtgacgactgaatccggtgagaatggcagaataggaacttcggaataggaacttcaaagcgtttccgaaaacgagcgcttccgaaaatgcaacgcgagctgcgcacatacagctcactgttcacgtcgcacctatatctgcgtgttgcctgtatatatatatacatgagaagaacggcatagtgcgtgtttatgcttaaatgcgtacttatatgcgtctatttatgtaggatgaaaggtagtctagtacctcctgtgatattatcccattccatgcggggtatcgtatgcttccttcagcactaccctttagctgttctatatgctgccactcctcaattggattagtctcatccttcaatgctatcatttcctttgatattggatcatatgcatagtaccgagaaactagtgcgaagtagtgatcaggtattgctgttatctgatgagtatacgttgtcctggccacggcagaagcacgcttatcgctccaatttcccacaacattagtcaactccgttaggcccttcattgaaagaaatgaggtcatcaaatgtcttccaatgtgagattttgggccattttttatagcaaagattgaataaggcgcatttttcttcaaagctttattgtacgatctgactaagttatcttttaataattggtattcctgtttattgcttgaagaattgccggtcctatttactcgttttaggactggttcagaattcctcaaaaattcatccaaatatacaagtggatcgatcctaccccttgcgctaaagaagtatatgtgcctactaacgcttgtctttgtctctgtcactaaacactggattattactcccagatacttattttggactaatttaaatgatttcggatcaacgttcttaatatcgctgaatcttccacaattgatgaaagtagctaggaagaggaattggtataaagtttttgtttttgtaaatctcgaagtatactcaaacgaatttagtattttctcagtgatctcccagatgctttcaccctcacttagaagtgctttaagcatttttttactgtggctatttcccttatctgcttcttccgatgattcgaactgtaattgcaaactacttacaatatcagtgatatcagattgatgtttttgtccatagtaaggaataattgtaaattcccaagcaggaatcaatttctttaatgaggcttccagaattgttgctttttgcgtcttgtatttaaactggagtgatttattgacaatatcgaaactcagcgaattgcttatgatagtattatagctcatgaatgtggctctcttgattgctgttccgttatgtgtaatcatccaacataaataggttagttcagcagcacataatgctattttctcacctgaaggtctttcaaacctttccacaaactgacgaacaagcaccttaggtggtgttttacataatatatcaaattgtggcatacaacctccttagtacatgcaaccattatcaccgccagaggtaaaatagtcaacacgcacggtgttagatatttatcccttgcggtgatagatttaacgtatgagcacaaaaaagaaaccattaacacaagagcagcttgaggacgcacgtcgccttaaagcaatttatgaaaaaaagaaaaatgaacttggcttatcccaggaatctgtcgcagacaagatggggatggggcagtcaggcgttggtgctttatttaatggcatcaatgcattaaatgcttataacgccgcattgcttacaaaaattctcaaagttagcgttgaagaatttagcccttcaatcgccagagaaatctacgagatgtatgaagcggttagtatgcagccgtcacttagaagtgagtatgagtaccctgttttttctcatgttcaggcagggatgttctcacctaagcttagaacctttaccaaaggtgatgcggagagatgggtaagcacaaccaaaaaagccagtgattctgcattctggcttgaggttgaaggtaattccatgaccgcaccaacaggctccaagccaagctttcctgacggaatgttaattctcgttgaccctgagcaggctgttgagccaggtgatttctgcatagccagacttgggggtgatgagtttaccttcaagaaactgatcagggatagcggtcaggtgtttttacaaccactaaacccacagtacccaatgatcccatgcaatgagagttgttccgttgtggggaaagttatcgctagtcagtggcctgaagagacgtttggctgatcggcaaggtgttctggtcggcgcatagctgataacaattgagcaagaatctgcatttctttccagacttgttcaacaggccagccattacgctcgtcatcaaaatcactcgcatcaaccaaaccgttattcattcgtgattgcgcctgagcgagacgaaatacgcgatcgctgttaaaaggacaattacaaacaggaatcgaatgcaaccggcgcaggaacactgccagcgcatcaacaatattttcacctgaatcaggatattcttctaatacctggaatgctgttttcccggggatcgcagtggtgagtaaccatgcatcatcaggagtacggataaaatgcttgatggtcggaagaggcataaattccgtcagccagtttagtctgaccatctcatctgtaacatcattggcaacgctacctttgccatgtttcagaaacaactctggcgcatcgggcttcccatacaatcgatagattgtcgcacctgattgcccgacattatcgcgagcccatttatacccatataaatcagcatccatgttggaatttaatcgcggcctcgagcaagacgtttcccgttgaatatggctcataacaccccttgtattactgtttatgtaagcagacagttttattgttcatgatgatatatttttatcttgtgcaatgtaacatcagagatttt

SEQ ID NO: 60 - DNA, 1013 bp, synthetic construct
  source 1..1013: mol_type = other DNA
taatacgactcactatagggtaccacgtagaccgtacggcagtaataaccagctgaccgcatacccgagtaatggcttccaaggtgtacgaccccgagcaacgcaaacgcatgatcactgggcctcagtggtgggctcgctgcaagcaaatgaacgtgctggactccttcatcaactactatgattccgagaagcacgccgagaacgccgtgatttttctgcatggtaacgctgcctccagctacctgtggaggcacgtcgtgcctcacatcgagcccgtggctagatgcatcatccctgatctgatcggaatgggtaagtccggcaagagcgggaatggctcatatcgcctcctggatcactacaagtacctcaccgcttggttcgagctgctgaaccttccaaagaaaatcatctttgtgggccacgactggggggcttgtctggcctttcactactcctacgagcaccaagacaagatcaaggccatcgtccatgctgagagtgtcgtggacgtgatcgagtcctgggacgagtggcctgacatcgaggaggatatcgccctgatcaagagcgaagagggcgagaaaatggtgcttgagaataacttcttcgtcgagaccatgctcccaagcaagatcatgcggaaactggagcctgaggagttcgctgcctacctggagccattcaaggagaagggcgaggttagacggcctaccctctcctggcctcgcgagatccctctcgttaagggaggcaagcccgacgtcgtccagattgtccgcaactacaacgcctaccttcgggccagcgacgatctgcctaagatgttcatcgagtccgaccctgggttcttttccaacgctattgtcgagggagctaagaagttccctaacaccgagttcgtgaaggtgaagggcctccacttcagccaggaggacgctccagatgaaatgggtaagtacatcaagagcttcgtggagcgcgtgctgaagaacgagcagtaatacgta

SEQ ID NO: 61 - DNA, 1013 bp, synthetic construct
  source 1..1013: mol_type = other DNA
taatacgactcactatagggtaccacgtagaccgtacggcagtaataaccagctgaccgcatacccgagtaatggcgtccaaggtttacgaccctgagcagcggaagcgcatgatcacgggcccacagtggtgggcccgttgcaagcagatgaacgttctcgacagcttcatcaactattacgatagtgagaagcatgcagagaacgccgtcatcttcttgcacgggaatgcagcgagcagctatctatggcggcacgttgtgccgcacatagagcctgttgctcgctgcataatcccggaccttatagggatggggaagagcggtaagagcggcaacggctcttaccgccttctcgatcactataagtacttgacagcatggttcgagctcctcaatctgcccaagaagatcatcttcgttgggcacgattggggagcttgtctcgccttccattactcttacgagcaccaggacaagatcaaggccatcgtccacgcggagagcgtggtcgatgtgatcgagtcctgggatgagtggcccgatatcgaggaggatatcgcactcatcaagagtgaggaaggcgagaagatggtcctggagaataatttcttcgtggagaccatgctgccaagtaagatcatgcgcaagctcgagccggaggagtttgcggcgtacctcgagcccttcaaggagaagggcgaggtacgccgcccgactctctcctggcctcgagagatcccgctggtcaagggtggtaagccggacgtcgtgcagatagtgcgtaactacaacgcctatctgcgggcaagtgacgacttgcccaagatgttcattgagagcgaccccggcttcttctcgaacgccattgttgagggagctaagaagttccccaacacggagttcgtgaaggtgaaggggttgcatttcagtcaggaggacgcgcccgacgaaatgggcaagtacatcaagtccttcgtcgagcgcgtcctcaagaatgagcagtaatacgta

SEQ ID NO: 62 - DNA, 6080 bp, synthetic construct
  source 1..6080: mol_type = other DNA
gtagtactcagctgtaatacgactcactatagggtaccacgtagaccgtacggcagtaataaccagctgaccgcatacccgagtaatggcttccaaggtgtacgaccccgagcaacgcaaacgcatgatcactgggcctcagtggtgggctcgctgcaagcaaatgaacgtgctggactccttcatcaactactatgattccgagaagcacgccgagaacgccgtgatttttctgcatggtaacgctgcctccagctacctgtggaggcacgtcgtgcctcacatcgagcccgtggctagatgcatcatccctgatctgatcggaatgggtaagtccggcaagagcgggaatggctcatatcgcctcctggatcactacaagtacctcaccgcttggttcgagctgctgaaccttccaaagaaaatcatctttgtgggccacgactggggggcttgtctggcctttcactactcctacgagcaccaagacaagatcaaggccatcgtccatgctgagagtgtcgtggacgtgatcgagtcctgggacgagtggcctgacatcgaggaggatatcgccctgatcaagagcgaagagggcgagaaaatggtgcttgagaataacttcttcgtcgagaccatgctcccaagcaagatcatgcggaaactggagcctgaggagttcgctgcctacctggagccattcaaggagaagggcgaggttagacggcctaccctctcctggcctcgcgagatccctctcgttaagggaggcaagcccgacgtcgtccagattgtccgcaactacaacgcctaccttcgggccagcgacgatctgcctaagatgttcatcgagtccgaccctgggttcttttccaacgctattgtcgagggagctaagaagttccctaacaccgagttcgtgaaggtgaagggcctccacttcagccaggaggacgctccagatgaaatgggtaagtacatcaagagcttcgtggagcgcgtgctgaagaacgagcagtaatacgtagatatcatccaatggatctgtcgacggccgtcgttttacagccaagcttggctgttttggcggatgagagaagattttcagcctgatacagattaaatcagaacgcagaagcggtctgataaaacagaatttgcctggcggcagtagcgcggtggtcccacctgaccccatgccgaactcagaagtgaaacgccgtagcgccgatggtagtgtggggtctccccatgcgagagtagggaactgccaggcatcaaataaaacgaaaggctcagtcgaaagactgggcctttcgttttatctgttgtttgtcggtgaacgctctcctgagtaggacaaatccgccgggagcggatttgaacgttgcgaagcaacggcccggagggtggcgggcaggacgcccgccataaactgccaggcatcaaattaagcagaaggccatcctgacggatggcctttttgcgtttctacaaactcttttggtcgactctagagttccactgagcgtcagaccccgtagaaaagatcaaaggatcttcttgagatcctttttttctgcgcgtaatctgctgcttgcaaacaaaaaaaccaccgctaccagcggtggtttgtttgccggatcaagagctaccaactctttttccgaaggtaactggcttcagcagagcgcagataccaaatactgtccttctagtgtagccgtagttaggccaccacttcaagaactctgtagcaccgcctacatacctcgctctgctaatcctgttaccagtggctgctgccagtggcgataagtcgtgtcttaccgggttggactcaagacgatagttaccggataaggcgcagcggtcgggctgaacggggggttcgtgcacacagcccagcttggagcgaacgacctacaccgaactgagatacctacagcgtgagctatgagaaagcgccacgcttcccgaagggagaaaggcggacaggtatccggtaagcggcagggtcggaacaggagagcgcacgagggagcttccagggggaaacgcctggtatctttatagtcctgtcgggtttcgccacctctgacttgagcgtcgatttttgtgatgctcgtcaggggggcggagcctatggaaaaacgccagcaacgcggcctttttacggttcctggccttttgctggccttttgctcacatgttctttcctgcgttatcccctgattctgtggataaccgtattaccgcctttgagtgagctgataccgctcgccgcagccgaacgaccgagcgcagcgagtcagtgagcgaggaagcggaagatctagaagtactgctgactcataccaggcctgaatcgccccatcatccagccagaaagtgagggagccacggttgatgagagctttgttgtaggtggaccagttggtgattttgaacttttgctttgccacggaacggtctgcgttgtcgggaagatgcgtgatctgatccttcaactcagcaaaagttcgatttattcaacaaagccacgttgtgtctcaaaatctctgatgttacattgcacaagataaaaatatatcatcatgaacaataaaactgtctgcttacataaacagtaatacaaggggtgttatgagccatattcaacgggaaacgtcttgctcaaggccgcgattaaattccaacatggatgctgatttatatgggtataaatgggctcgcgataatgtcgggcaatcaggtgcgacaatctatcgattgtatgggaagcccgatgcgccagagttgtttctgaaacatggcaaaggtagcgttgccaatgatgttacagatgagatggtcagactaaactggctgacggaatttatgcctcttccgaccatcaagcattttatccgtactcctgatgatgcatggttactcaccactgcgatccccggaaaaacagcattccaggtattagaagaatatcctgattcaggtgaaaatattgttgatgcgctggcagtgttcctgcgccggttgcattcgattcctgtttgtaattgtccttttaacagcgatcgcgtatttcgtctcgctcaggcgcaatcacgaatgaataacggtttggttgatgcgagtgattttgatgacgagcgtaatggctggcctgttgaacaagtctggaaagaaatgcataagcttttgccattctcaccggattcagtcgtcactcatggtgatttctcacttgataaccttatttttgacgaggggaaattaataggttgtattgatgttggacgagtcggaatcgcagaccgataccaggatcttgccatcctatggaactgcctcggtgagttttctccttcattacagaaacggctttttcaaaaatatggtattgataatcctgatatgaataaattgcagtttcatttgatgctcgatgagtttttctaaggctagccccgggactagtgatctttgggagcagtccttgtgcgcttacgaggtgagccggtggggaaccgttatctgcctatggtgtgagcccccctagagagcttcaagagcaatcagcccgacctagaaaggaggccaagagagagacccctacggggggaaccgttttctgcctacgagatggcacatttactgggaagctttacggcgtcctcgtggaagttcaatgcccgcagacttaagtgctctattcacggtctgacgtgacacgctaaattcagacatagcttcattgattgtcggccacgagccagtctctccctcaacagtcataaaccaacctgcaatggtcaagcgattttctttagctttcctagcttgtcgttgactggacttagctagtttttctcgctgtgctcgggcgtactcactgtttgggtctttccagcgttctgcggcctttttaccgccacgtcttcccatagtggccagagcttttcgccctcggctgctctgcgtctctgtctgacgagcagggacgactggctggcctttagcgacgtagccgcgcacacgtcgcgccatcgtctggcggtcacgcatcggcggcagatcaggctcacggccgtctgctccgaccgcctgagcgacggtgtaggcacgctcgtaggcgtcgatgatcttggtgtcttttaggcgctcaccagccgcttttaactggtatcccacagtcaaagcgtggcgaaaagccgtctcatcacgggcggcacgccctggagcagtccagaggacacggacgccgtcgatcagctctccagacgcttcagcggcgctcggcaggcttgcttcaagcgtggcaagtgcttttgcttccgcagtggcttttcttgccgcttcgatacgtgcccgtccgctagaaaactcctgctcatagcgttttttaggtttttctgtgcctgagatcatgcgagcaacctccataagatcagctaggcgatccacgcgattgtgctgggcatgccagcggtacgcggtgggatcgtcggagacgtgcagtggccaccggctcagcctatgtgaaaaagcctggtcagcgccgaaaacgcgggtcatttcctcggtcgttgcagccagcaggcgcatattcgggctgctcatgcctgctgcggcatacaccggatcaatgagccagatgagctggcatttcccgctcagtggattcacgccgatccaagctggcgctttttccaggcgtgcccagcgctccaaaatcgcgtagacctcggggtttacgtgctcgattttcccgccggcctggtggctcggcacatcaatgtccaggacaagcacggctgcgtgctgcgcgtgcgtcagagcaacatactggcaccgggcaagcgattttgaaccaactcggtataacttcggctgtgtttctcccgtgtccgggtctttgatccaagcgctggcgaagtcgcgggtcttgctgccctggaaattttctctgcccaggtgagcgaggaattcgcggcggtcttcgctcgtccagccacgtgatcgcagcgcgagctcgggatgggtgtcgaacagatcagcggaaaatttccaggccggtgtgtcaatgtctcgtgaatccgctagagtcatttttgagcgctttctcccaggtttggactgggggttagccgacgccctgtgagttaccgctcacggggcgttcaacatttttcaggtattcgtgcagcttatcgcttcttgccgcctgtgcgctttttcgacgcgcgacgctgctgccgattcggtgcaggtggtggcggcgctgacacgtcctgggcggccacggccacacgaaacgcggcatttacgatgtttgtcatgcctgcgggcaccgcgccacgatcgcggataattctcgctgccgcttccagctctgtgacgaccatggccaaaatttcgctcgggggacgcacttccagcgccatttgcgacctagccgcctccagctcctcggcgtggcgtttgttggcgcgctcgcggctggctgcggcacgacacgcatctgagcaatattttgcgcgccgtcctcgcgggtcaggccggggaggaatcaggccaccgcagtaggcgcaactgattcgatcctccactactgtgcgtcctcctggcgctgccgagcacgcagctcgtcagccagctcctcaagatccgccacgagagtttctaggtcgctcgcggcactggcccagtctcgtgatgctggcgcgtccgtcgtatcgagagctcggaaaaatccgatcaccgtttttaaatcgacggcagcatcgagcgcgtcggactccagcgcgacatcagagagatccatagctgatgattcgggccaattttggtacttcgtcgtgaaggtcatgacaccattataacgaacgttcgttaaagtttttggcggaaaatcacgcggcacgaaaattttcacgaagcgggactttgcgcagctcaggggtgctaaaaattttgtatcgcacttgatttttccgaaagacagattatctgcaaacggtgtgtcgtatttctggcttggtttttaaaaaatctggaatcgaaaatttgcggggcga

SEQ ID NO: 63 - DNA, 6080 bp, synthetic construct
  source 1..6080: mol_type = other DNA
gtagtactcagctgtaatacgactcactatagggtaccacgtagaccgtacggcagtaataaccagctgaccgcatacccgagtaatggcgtccaaggtttacgaccctgagcagcggaagcgcatgatcacgggcccacagtggtgggcccgttgcaagcagatgaacgttctcgacagcttcatcaactattacgatagtgagaagcatgcagagaacgccgtcatcttcttgcacgggaatgcagcgagcagctatctatggcggcacgttgtgccgcacatagagcctgttgctcgctgcataatcccggaccttatagggatggggaagagcggtaagagcggcaacggctcttaccgccttctcgatcactataagtacttgacagcatggttcgagctcctcaatctgcccaagaagatcatcttcgttgggcacgattggggagcttgtctcgccttccattactcttacgagcaccaggacaagatcaaggccatcgtccacgcggagagcgtggtcgatgtgatcgagtcctgggatgagtggcccgatatcgaggaggatatcgcactcatcaagagtgaggaaggcgagaagatggtcctggagaataatttcttcgtggagaccatgctgccaagtaagatcatgcgcaagctcgagccggaggagtttgcggcgtacctcgagcccttcaaggagaagggcgaggtacgccgcccgactctctcctggcctcgagagatcccgctggtcaagggtggtaagccggacgtcgtgcagatagtgcgtaactacaacgcctatctgcgggcaagtgacgacttgcccaagatgttcattgagagcgaccccggcttcttctcgaacgccattgttgagggagctaagaagttccccaacacggagttcgtgaaggtgaaggggttgcatttcagtcaggaggacgcgcccgacgaaatgggcaagtacatcaagtccttcgtcgagcgcgtcctcaagaatgagcagtaatacgtagatatcatccaatggatctgtcgacggccgtcgttttacagccaagcttggctgttttggcggatgagagaagattttcagcctgatacagattaaatcagaacgcagaagcggtctgataaaacagaatttgcctggcggcagtagcgcggtggtcccacctgaccccatgccgaactcagaagtgaaacgccgtagcgccgatggtagtgtggggtctccccatgcgagagtagggaactgccaggcatcaaataaaacgaaaggctcagtcgaaagactgggcctttcgttttatctgttgtttgtcggtgaacgctctcctgagtaggacaaatccgccgggagcggatttgaacgttgcgaagcaacggcccggagggtggcgggcaggacgcccgccataaactgccaggcatcaaattaagcagaaggccatcctgacggatggcctttttgcgtttctacaaactcttttggtcgactctagagttccactgagcgtcagaccccgtagaaaagatcaaaggatcttcttgagatcctttttttctgcgcgtaatctgctgcttgcaaacaaaaaaaccaccgctaccagcggtggtttgtttgccggatcaagagctaccaactctttttccgaaggtaactggcttcagcagagcgcagataccaaatactgtccttctagtgtagccgtagttaggccaccacttcaagaactctgtagcaccgcctacatacctcgctctgctaatcctgttaccagtggctgctgccagtggcgataagtcgtgtcttaccgggttggactcaagacgatagttaccggataaggcgcagcggtcgggctgaacggggggttcgtgcacacagcccagcttggagcgaacgacctacaccgaactgagatacctacagcgtgagctatgagaaagcgccacgcttcccgaagggagaaaggcggacaggtatccggtaagcggcagggtcggaacaggagagcgcacgagggagcttccagggggaaacgcctggtatctttatagtcctgtcgggtttcgccacctctgacttgagcgtcgatttttgtgatgctcgtcaggggggcggagcctatggaaaaacgccagcaacgcggcctttttacggttcctggccttttgctggccttttgctcacatgttctttcctgcgttatcccctgattctgtggataaccgtattaccgcctttgagtgagctgataccgctcgccgcagccgaacgaccgagcgcagcgagtcagtgagcgaggaagcggaagatctagaagtactgctgactcataccaggcctgaatcgccccatcatccagccagaaagtgagggagccacggttgatgagagctttgttgtaggtggaccagttggtgattttgaacttttgctttgccacggaacggtctgcgttgtcgggaagatgcgtgatctgatccttcaactcagcaaaagttcgatttattcaacaaagccacgttgtgtctcaaaatctctgatgttacattgcacaagataaaaatatatcatcatgaacaataaaactgtctgcttacataaacagtaatacaaggggtgttatgagccatattcaacgggaaacgtcttgctcaaggccgcgattaaattccaacatggatgctgatttatatgggtataaatgggctcgcgataatgtcgggcaatcaggtgcgacaatctatcgattgtatgggaagcccgatgcgccagagttgtttctgaaacatggcaaaggtagcgttgccaatgatgttacagatgagatggtcagactaaactggctgacggaatttatgcctcttccgaccatcaagcattttatccgtactcctgatgatgcatggttactcaccactgcgatccccggaaaaacagcattccaggtattagaagaatatcctgattcaggtgaaaatattgttgatgcgctggcagtgttcctgcgccggttgcattcgattcctgtttgtaattgtccttttaacagcgatcgcgtatttcgtctcgctcaggcgcaatcacgaatgaataacggtttggttgatgcgagtgattttgatgacgagcgtaatggctggcctgttgaacaagtctggaaagaaatgcataagcttttgccattctcaccggattcagtcgtcactcatggtgatttctcacttgataaccttatttttgacgaggggaaattaataggttgtattgatgttggacgagtcggaatcgcagaccgataccaggatcttgccatcctatggaactgcctcggtgagttttctccttcattacagaaacggctttttcaaaaatatggtattgataatcctgatatgaataaattgcagtttcatttgatgctcgatgagtttttctaaggctagccccgggactagtgatctttgggagcagtccttgtgcgcttacgaggtgagccggtggggaaccgttatctgcctatggtgtgagcccccctagagagcttcaagagcaatcagcccgacctagaaaggaggccaagagagagacccctacggggggaaccgttttctgcctacgagatggcacatttactgggaagctttacggcgtcctcgtggaagttcaatgcccgcagacttaagtgctctattcacggtctgacgtgacacgctaaattcagacatagcttcattgattgtcggccacgagccagtctctccctcaacagtcataaaccaacctgcaatggtcaagcgattttctttagctttcctagcttgtcgttgactggacttagctagtttttctcgctgtgctcgggcgtactcactgtttgggtctttccagcgttctgcggcctttttaccgccacgtcttcccatagtggccagagcttttcgccctcggctgctctgcgtctctgtctgacgagcagggacgactggctggcctttagcgacgtagccgcgcacacgtcgcgccatcgtctggcggtcacgcatcggcggcagatcaggctcacggccgtctgctccgaccgcctgagcgacggtgtaggcacgctcgtaggcgtcgatgatcttggtgtcttttaggcgctcaccagccgcttttaactggtatcccacagtcaaagcgtggcgaaaagccgtctcatcacgggcggcacgccctggagcagtccagaggacacggacgccgtcgatcagctctccagacgcttcagcggcgctcggcaggcttgcttcaagcgtggcaagtgcttttgcttccgcagtggcttttcttgccgcttcgatacgtgcccgtccgctagaaaactcctgctcatagcgttttttaggtttttctgtgcctgagatcatgcgagcaacctccataagatcagctaggcgatccacgcgattgtgctgggcatgccagcggtacgcggtgggatcgtcggagacgtgcagtggccaccggctcagcctatgtgaaaaagcctggtcagcgccgaaaacgcgggtcatttcctcggtcgttgcagccagcaggcgcatattcgggctgctcatgcctgctgcggcatacaccggatcaatgagccagatgagctggcatttcccgctcagtggattcacgccgatccaagctggcgctttttccaggcgtgcccagcgctccaaaatcgcgtagacctcggggtttacgtgctcgattttcccgccggcctggtggctcggcacatcaatgtccaggacaagcacggctgcgtgctgcgcgtgcgtcagagcaacatactggcaccgggcaagcgattttgaaccaactcggtataacttcggctgtgtttctcccgtgtccgggtctttgatccaagcgctggcgaagtcgcgggtcttgctgccctggaaattttctctgcccaggtgagcgaggaattcgcggcggtcttcgctcgtccagccacgtgatcgcagcgcgagctcgggatgggtgtcgaacagatcagcggaaaatttccaggccggtgtgtcaatgtctcgtgaatccgctagagtcatttttgagcgctttctcccaggtttggactgggggttagccgacgccctgtgagttaccgctcacggggcgttcaacatttttcaggtattcgtgcagcttatcgcttcttgccgcctgtgcgctttttcgacgcgcgacgctgctgccgattcggtgcaggtggtggcggcgctgacacgtcctgggcggccacggccacacgaaacgcggcatttacgatgtttgtcatgcctgcgggcaccgcgccacgatcgcggataattctcgctgccgcttccagctctgtgacgaccatggccaaaatttcgctcgggggacgcacttccagcgccatttgcgacctagccgcctccagctcctcggcgtggcgtttgttggcgcgctcgcggctggctgcggcacgacacgcatctgagcaatattttgcgcgccgtcctcgcgggtcaggccggggaggaatcaggccaccgcagtaggcgcaactgattcgatcctccactactgtgcgtcctcctggcgctgccgagcacgcagctcgtcagccagctcctcaagatccgccacgagagtttctaggtcgctcgcggcactggcccagtctcgtgatgctggcgcgtccgtcgtatcgagagctcggaaaaatccgatcaccgtttttaaatcgacggcagcatcgagcgcgtcggactccagcgcgacatcagagagatccatagctgatgattcgggccaattttggtacttcgtcgtgaaggtcatgacaccattataacgaacgttcgttaaagtttttggcggaaaatcacgcggcacgaaaattttcacgaagcgggactttgcgcagctcaggggtgctaaaaattttgtatcgcacttgatttttccgaaagacagattatctgcaaacggtgtgtcgtatttctggcttggtttttaaaaaatctggaatcgaaaatttgcggggcga

SEQ ID NO: 64 - DNA, 1615 bp, synthetic construct
  source 1..1615: mol_type = other DNA
ggatcccccgctgacgaacaaggatctcgcctgcggaaacctgctgaccaccgaaacgcttgacgccaaggcgcttagcctcggaatcacgaccgttgctggagctagatgcacccttcttgtgtgccatgtggtaattccctccttctaaaggaaaaactcatagaaagcccgagggcttacttgattccggttaccttcagaacggtcaggggctgacggtgtccctggcgcttcttgtatccggtcttgttcttgtacttcaggatcttgatcttcgggcccttggtgtgctcgacgatctcggtgttgacgctcacagaagcgagcttgtcagcggcggtggttacatcggcgccatcgacgagcagaaccggggtgagagccacggatgcacccggctcaccctcgatcttctcgaccttaacgaggtcaccttcggcaaccttgtactgctttccgccggtcttgacgatcgcgtacatagagggctaccccttatctgattctcggctcaggtactcggatgatgagtccctgattggacttacgttttacaattgcgttttagacatgcggagccaaaatgacctcacgtcattcacacattcgccgtgaaatgggcaaatgggcattactgacattgcctaaaacagcgactgtccaaggttacccctaaaggcggcttcaacacaaaccgcccttataccctagcttcgtggatttggcacagcgacactcctattttcttatctccacgattgagcaatgcacccgggcgctggtagggacaagatctcctaccgccgccgcgcaggtacatgcgccaatctaaaactgtatggtctaaattttccgacccgcaaatatattcgccaggcctgctgccattcttccataagtcttaggtcaagcttgcatttattggctagtgtcggaaatcatgggagatttagcaaagcacatgggcagtgaaccaccagcatggtggaagtttttaccgatgattgtcctcgctggagccactcgagttacctatgaagtagaaccttggctggcgatcccattattcattttggcttttgcatcgatattgatcccattcccgatctctaagacaaaaggactccgtgatatcgatgcctggaaaatccacaccacgcaaggcgataaaaagcgtgccatccgccaactgatcattccggctacggctttggccatcgacatcattgggctgccgacattatttaatgcccctccccttgcttccgctgcactttttggcggtgtttacggcgcttccctagcttgggctgcgtacagagctgatcagcttccacgcattcgaacgaaggaacgcctcgcagaactttcacaaaatgcatctctggatgatgtgcgctcagatgacttagatgttctagagcagccggaatcccgtgaattagtgcgctgtctgcttgcccacggtgcgatggatggcactcgggtgatggccagacaggtcgcgcgagtactggataccgaggtagacgaagtacatcaggtagcacgctcactagaacagcatggtttggttagtcgctccaccatcatgggtaccgagctcgaattc

SEQ ID NO: 65 - DNA, 7310 bp, synthetic construct
  source 1..7310: mol_type = other DNA
attaggcaccccaggctttacactttatgcttccggctcgtatgttgtgtggaattgtgagcggataacaatttcacacaggaaacagctatgaccatgattacgccaagcttgcatgcctgcaggtcgactctagaggatcccccgctgacgaacaaggatctcgcctgcggaaacctgctgaccaccgaaacgcttgacgccaaggcgcttagcctcggaatcacgaccgttgctggagctagatgcacccttcttgtgtgccatgtggtaattccctccttctaaaggaaaaactcatagaaagcccgagggcttacttgattccggttaccttcagaacggtcaggggctgacggtgtccctggcgcttcttgtatccggtcttgttcttgtacttcaggatcttgatcttcgggcccttggtgtgctcgacgatctcggtgttgacgctcacagaagcgagcttgtcagcggcggtggttacatcggcgccatcgacgagcagaaccggggtgagagccacggatgcacccggctcaccctcgatcttctcgaccttaacgaggtcaccttcggcaaccttgtactgctttccgccggtcttgacgatcgcgtacatagagggctaccccttatctgattctcggctcaggtactcggatgatgagtccctgattggacttacgttttacaattgcgttttagacatgcggagccaaaatgacctcacgtcattcacacattcgccgtgaaatgggcaaatgggcattactgacattgcctaaaacagcgactgtccaaggttacccctaaaggcggcttcaacacaaaccgcccttataccctagcttcgtggatttggcacagcgacactcctattttcttatctccacgattgagcaatgcacccgggcgctggtagggacaagatctcctaccgccgccgcgcaggtacatgcgccaatctaaaactgtatggtctaaattttccgacccgcaaatatattcgccaggcctgctgccattcttccataagtcttaggtcaagcttgcatttattggctagtgtcggaaatcatgggagatttagcaaagcacatgggcagtgaaccaccagcatggtggaagtttttaccgatgattgtcctcgctggagccactcgagttacctatgaagtagaaccttggctggcgatcccattattcattttggcttttgcatcgatattgatcccattcccgatctctaagacaaaaggactccgtgatatcgatgcctggaaaatccacaccacgcaaggcgataaaaagcgtgccatccgccaactgatcattccggctacggctttggccatcgacatcattgggctgccgacattatttaatgcccctccccttgcttccgctgcactttttggcggtgtttacggcgcttccctagcttgggctgcgtacagagctgatcagcttccacgcattcgaacgaaggaacgcctcgcagaactttcacaaaatgcatctctggatgatgtgcgctcagatgacttagatgttctagagcagccggaatcccgtgaattagtgcgctgtctgcttgcccacggtgcgatggatggcactcgggtgatggccagacaggtcgcgcgagtactggataccgaggtagacgaagtacatcaggtagcacgctcactagaacagcatggtttggttagtcgctccaccatcatgggtaccgagctcgaattcactggccgtcgttttacaacgtcgtgactgggaaaaccctggcgttacccaacttaatcgccttgcagcacatccccctttcgccagctggcgtaatagcgaagaggcccgcaccgatcgcccttcccaacagttgcgcagcctgaatggcgaatggcgcgataagctagcttcacgctgccgcaagcactcagggcgcaagggctgctaaaggaagcggaacacgtagaaagccagtccgcagaaacggtgctgaccccggatgaatgtcagctactgggctatctggacaagggaaaacgcaagcgcaaagagaaagcaggtagcttgcagtgggcttacatggcgatagctagactgggcggttttatggacagcaagcgaaccggaattgccagctggggcgccctctggtaaggttgggaagccctgcaaagtaaactggatggctttcttgccgccaaggatctgatggcgcaggggatcaagatctgatcaagagacaggatgaggatcgtttcgcatgattgaacaagatggattgcacgcaggttctccggccgcttgggtggagaggctattcggctatgactgggcacaacagacaatcggctgctctgatgccgccgtgttccggctgtcagcgcaggggcgcccggttctttttgtcaagaccgacctgtccggtgccctgaatgaactccaagacgaggcagcgcggctatcgtggctggccacgacgggcgttccttgcgcagctgtgctcgacgttgtcactgaagcgggaagggactggctgctattgggcgaagtgccggggcaggatctcctgtcatctcaccttgctcctgccgagaaagtatccatcatggctgatgcaatgcggcggctgcatacgcttgatccggctacctgcccattcgaccaccaagcgaaacatcgcatcgagcgagcacgtactcggatggaagccggtcttgtcgatcaggatgatctggacgaagagcatcaggggctcgcgccagccgaactgttcgccaggctcaaggcgcggatgcccgacggcgaggatctcgtcgtgacccatggcgatgcctgcttgccgaatatcatggtggaaaatggccgcttttctggattcatcgactgtggccggctgggtgtggcggaccgctatcaggacatagcgttggctacccgtgatattgctgaagagcttggcggcgaatgggctgaccgcttcctcgtgctttacggtatcgccgctcccgattcgcagcgcatcgccttctatcgccttcttgacgagttcttctgagcgggactctggggttcgctagaggatcgatcctttttaacccatcacatatacctgccgttcactattatttagtgaaatgagatattatgatattttctgaattgtgattaaaaaggcaactttatgcccatgcaacagaaactataaaaaatacagagaatgaaaagaaacagatagattttttagttctttaggcccgtagtctgcaaatccttttatgattttctatcaaacaaaagaggaaaatagaccagttgcaatccaaacgagagtctaatagaatgaggtcgaaaagtaaatcgcgcgggtttgttactgataaagcaggcaagacctaaaatgtgtaaagggcaaagtgtatactttggcgtcaccccttacatattttaggtctttttttattgtgcgtaactaacttgccatcttcaaacaggagggctggaagaagcagaccgctaacacagtacataaaaaaggagacatgaacgatgaacatcaaaaagtttgcaaaacaagcaacagtattaacctttactaccgcactgctggcaggaggcgcaactcaagcgtttgcgaaagaaacgaaccaaaagccatataaggaaacatacggcatttcccatattacacgccatgatatgctgcaaatccctgaacagcaaaaaaatgaaaaatatcaagtttctgaatttgattcgtccacaattaaaaatatctcttctgcaaaaggcctggacgtttgggacagctggccattacaaaacgctgacggcactgtcgcaaactatcacggctaccacatcgtctttgcattagccggagatcctaaaaatgcggatgacacatcgatttacatgttctatcaaaaagtcggcgaaacttctattgacagctggaaaaacgctggccgcgtctttaaagacagcgacaaattcgatgcaaatgattctatcctaaaagaccaaacacaagaatggtcaggttcagccacatttacatctgacggaaaaatccgtttattctacactgatttctccggtaaacattacggcaaacaaacactgacaactgcacaagttaacgtatcagcatcagacagctctttgaacatcaacggtgtagaggattataaatcaatctttgacggtgacggaaaaacgtatcaaaatgtacagcagttcatcgatgaaggcaactacagctcaggcgacaaccatacgctgagagatcctcactacgtagaagataaaggccacaaatacttagtatttgaagcaaacactggaactgaagatggctaccaaggcgaagaatctttatttaacaaagcatactatggcaaaagcacatcattcttccgtcaagaaagtcaaaaacttctgcaaagcgataaaaaacgcacggctgagttagcaaacggcgctctcggtatgattgagctaaacgatgattacacactgaaaaaagtgatgaaaccgctgattgcatctaacacagtaacagatgaaattgaacgcgcgaacgtctttaaaatgaacggcaaatggtacctgttcactgactcccgcggatcaaaaatgacgattgacggcattacgtctaacgatatttacatgcttggttatgtttctaattctttaactggcccatacaagccgctgaacaaaactggccttgtgttaaaaatggatcttgatcctaacgatgtaacctttacttactcacacttcgctgtacctcaagcgaaaggaaacaatgtcgtgattacaagctatatgacaaacagaggattctacgcagacaaacaatcaacgtttgcgccgagcttcctgctgaacatcaaaggcaagaaaacatctgttgtcaaagacagcatccttgaacaaggacaattaacagttaacaaataaaaacgcaaaagaaaatgccgatgggtaccgagcgaaatgaccgaccaagcgacgcccaacctgccatcacgagatttcgattccaccgccgccttctatgaaaggttgggcttcggaatcgttttccgggacgccctcgcggacgtgctcatagtccacgacgcccgtgattttgtagccctggccgacggccagcaggtaggccgacaggctcatgccggccgccgccgccttttcctcaatcgctcttcgttcgtctggaaggcagtacaccttgataggtgggctgcccttcctggttggcttggtttcatcagccatccgcttgccctcatctgttacgccggcggtagccggccagcctcgcagagcaggattcccgttgagcaccgccaggtgcgaataagggacagtgaagaaggaacacccgctcgcgggtgggcctacttcacctatcctgccccgctgacgccgttggatacaccaaggaaagtctacacgaaccctttggcaaaatcctgtatatcgtgcgaaaaaggatggatataccgaaaaaatcgctataatgaccccgaagcagggttatgcagcggaaaagcgctgcttccctgctgttttgtggaatatctaccgactggaaacaggcaaatgcaggaaattactgaactgaggggacaggcgagagacgatgccaaagagctcctgaaaatctcgataactcaaaaaatacgcccggtagtgatcttatttcattatggtgaaagttggaacctcttacgtgccgatcaacgtctcattttcgccaaaagttggcccagggcttcccggtatcaacagggacaccaggatttatttattctgcgaagtgatcttccgtcacaggtatttattcggcgcaaagtgcgtcgggtgatgctgccaacttactgatttagtgtatgatggtgtttttgaggtgctccagtggcttctgtttctatcagctcctgaaaatctcgataactcaaaaaatacgcccggtagtgatcttatttcattatggtgaaagttggaacctcttacgtgccgatcaacgtctcattttcgccaaaagttggcccagggcttcccggtatcaacagggacaccaggatttatttattctgcgaagtgatcttccgtcacaggtatttattcggcgcaaagtgcgtcgggtgatgctgccaacttactgatttagtgtatgatggtgtttttgaggtgctccagtggcttctgtttctatcagggctggatgatcctccagcgcggggatctcatgctggagttcttcgcccaccccaaaaggatctaggtgaagatcctttttgataatctcatgaccaaaatcccttaacgtgagttttcgttccactgagcgtcagaccccgtagaaaagatcaaaggatcttcttgagatcctttttttctgcgcgtaatctgctgcttgcaaacaaaaaaaccaccgctaccagcggtggtttgtttgccggatcaagagctaccaactctttttccgaaggtaactggcttcagcagagcgcagataccaaatactgtccttctagtgtagccgtagttaggccaccacttcaagaactctgtagcaccgcctacatacctcgctctgctaatcctgttaccagtggctgctgccagtggcgataagtcgtgtcttaccgggttggactcaagacgatagttaccggataaggcgcagcggtcgggctgaacggggggttcgtgcacacagcccagcttggagcgaacgacctacaccgaactgagatacctacagcgtgagcattgagaaagcgccacgcttcccgaagggagaaaggcggacaggtatccggtaagcggcagggtcggaacaggagagcgcacgagggagcttccagggggaaacgcctggtatctttatagtcctgtcgggtttcgccacctctgacttgagcgtcgatttttgtgatgctcgtcaggggggcggagcctatggaaaaacgccagcaacgcggcctttttacggttcctggccttttgctggccttttgctcacatgttctttcctgcgttatcccctgattctgtggataaccgtattaccgcctttgagtgagctgataccgctcgccgcagccgaacgaccgagcgcagcgagtcagtgagcgaggaagcggaagagcgcccaatacgcaaaccgcctctccccgcgcgttggccgattcattaatgcagctggcacgacaggtttcccgactggaaagcgggcagtgagcgcaacgcaattaatgtgagttagctcactc

SEQ ID NO: 66 - DNA, 20 bp, synthetic construct
  source 1..20: mol_type = other DNA
caagtgccttgatggctgag

SEQ ID NO: 67 - DNA, 20 bp, synthetic construct
  source 1..20: mol_type = other DNA
ccagtcttcagtgcgaagag

SEQ ID NO: 68 - DNA, 4169 bp, synthetic construct
  source 1..4169: mol_type = other DNA
tcaagccttcgtcactggtcccgccaccaaacgtttcggcgagaagcaggccattatcgccggcatggcggccgacgcgcggggagaggcggtttgcgtattgggcgccagggtggtttttcttttcaccagtgagacgggcaacagctgattgcccttcaccgcctggccctgagagagttgcagcaagcggtccacgctggtttgccccagcaggcgaaaatcctgtttgatggtggttaacggcgggatataacatgagctgtcttcggtatcgtcgtatcccactaccgagatatccgcaccaacgcgcagcccggactcggtaatggcgcgcattgcgcccagcgccatctgatcgttggcaaccagcatcgcagtgggaacgatgccctcattcagcatttgcatggtttgttgaaaaccggacatggcactccagtcgccttcccgttccgctatcggctgaatttgattgcgagtgagatatttatgccagccagccagacgcagacgcgccgagacagaacttaatgggcccgctaacagcgcgatttgctggtgacccaatgcgaccagatgctccacgcccagtcgcgtaccgtcttcatgggagaaaataatactgttgatgggtgtctggtcagagacatcaagaaataacgccggaacattagtgcaggcagcttccacagcaatggcatcctggtcatccagcggatagttaatgatcagcccactgacgcgttgcgcgagaagattgtgcaccgccgctttacaggcttcgacgccgcttcgttctaccatcgacaccaccacgctggcacccagttgatcggcgcgagatttaatcgccgcgacaatttgcgacggcgcgtgcagggccagactggaggtggcaacgccaatcagcaacgactgtttgcccgccagttgttgtgccacgcggttgggaatgtaattcagctccgccatcgccgcttccactttttcccgcgttttcgcagaaacgtggctggcctggttcaccacgcgggaaacggtctgataagagacaccggcatactctgcgacatcgtataacgttactggtttcacattcaccaccctgaattgactctcttccgggcgctatcatgccataccgcgaaaggttttgcaccattcgatggtgtcaacgtaaatgcatgccgcttcgccttcgcgcgcgaattgcaagctgatccgggcttatcgactgcacggtgcaccaatgcttctggcgtcaggcagccatcggaagctgtggtatggctgtgcaggtcgtaaatcactgcataattcgtgtcgctcaaggcgcactcccgttctggataatgttttttgcgccgacatcataacggttctggcaaatattctgaaatgagctgttgacaattaatcatcggctcgtataatgtgtggaattgtgagcggataacaatttcacacaggaaacagggatctgatccggatttactaactggaagaggcactaaatgaacacgattaacatcgctaagaacgacttctctgacatcgaactggctgctatcccgttcaacactctggctgaccattacggtgagcgtttagctcgcgaacagttggcccttgagcatgagtcttacgagatgggtgaagcacgcttccgcaagatgtttgagcgtcaacttaaagctggtgaggttgcggataacgctgccgccaagcctctcatcactaccctactccctaagatgattgcacgcatcaacgactggtttgaggaagtgaaagctaagcgcggcaagcgcccgacagccttccagttcctgcaagaaatcaagccggaagccgtagcgtacatcaccattaagaccactctggcttgcctaaccagtgctgacaatacaaccgttcaggctgtagcaagcgcaatcggtcgggccattgaggacgaggctcgcttcggtcgtatccgtgaccttgaagctaagcacttcaagaaaaacgttgaggaacaactcaacaagcgcgtagggcacgtctacaagaaagcatttatgcaagttgtcgaggctgacatgctctctaagggtctactcggtggcgaggcgtggtcttcgtggcataaggaagactctattcatgtaggagtacgctgcatcgagatgctcattgagtcaaccggaatggttagcttacaccgccaaaatgctggcgtagtaggtcaagactctgagactatcgaactcgcacctgaatacgctgaggctatcgcaacccgtgcaggtgcgctggctggcatctctccgatgttccaaccttgcgtagttcctcctaagccgtggactggcattactggtggtggctattgggctaacggtcgtcgtcctctggcgctggtgcgtactcacagtaagaaagcactgatgcgctacgaagacgtttacatgcctgaggtgtacaaagcgattaacattgcgcaaaacaccgcatggaaaatcaacaagaaagtcctagcggtcgccaacgtaatcaccaagtggaagcattgtccggtcgaggacatccctgcgattgagcgtgaagaactcccgatgaaaccggaagacatcgacatgaatcctgaggctctcaccgcgtggaaacgtgctgccgctgctgtgtaccgcaaggacaaggctcgcaagtctcgccgtatcagccttgagttcatgcttgagcaagccaataagtttgctaaccataaggccatctggttcccttacaacatggactggcgcggtcgtgtttacgctgtgtcaatgttcaacccgcaaggtaacgatatgaccaaaggactgcttacgctggcgaaaggtaaaccaatcggtaaggaaggttactactggctgaaaatccacggtgcaaactgtgcgggtgtcgataaggttccgttccctgagcgcatcaagttcattgaggaaaaccacgagaacatcatggcttgcgctaagtctccactggagaacacttggtgggctgagcaagattctccgttctgcttccttgcgttctgctttgagtacgctggggtacagcaccacggcctgagctataactgctcccttccgctggcgtttgacgggtcttgctctggcatccagcacttctccgcgatgctccgagatgaggtaggtggtcgcgcggttaacttgcttcctagtgaaaccgttcaggacatctacgggattgttgctaagaaagtcaacgagattctacaagcagacgcaatcaatgggaccgataacgaagtagttaccgtgaccgatgagaacactggtgaaatctctgagaaagtcaagctgggcactaaggcactggctggtcaatggctggcttacggtgttactcgcagtgtgactaagcgttcagtcatgacgctggcttacgggtccaaagagttcggcttccgtcaacaagtgctggaagataccattcagccagctattgattccggcaagggtctgatgttcactcagccgaatcaggctgctggatacatggctaagctgatttgggaatctgtgagcgtgacggtggtagctgcggttgaagcaatgaactggcttaagtctgctgctaagctgctggctgctgaggtcaaagataagaagactggagagattcttcgcaagcgttgcgctgtgcattgggtaactcctgatggtttccctgtgtggcaggaatacaagaagcctattcagacgcgcttgaacctgatgttcctcggtcagttccgcttacagcctaccattaacaccaacaaagatagcgagattgatgcacacaaacaggagtctggtatcgctcctaactttgtacacagccaagacggtagccaccttcgtaagactgtagtgtgggcacacgagaagtacggaatcgaatcttttgcactgattcacgactccttcggtaccattccggctgacgctgcgaacctgttcaaagcagtgcgcgaaactatggttgacacatatgagtcttgtgatgtactggctgatttctacgaccagttcgctgaccagttgcacgagtctcaattggacaaaatgccagcacttccggctaaaggtaacttgaacctccgtgacatcttagagtcggacttcgcgttcgcgtaa

SEQ ID NO: 69 - DNA, 9272 bp, synthetic construct
  source 1..9272: mol_type = other DNA
gaagctgtcaaacatggcctgtcgcttgcggtattcggaatcttgcacgccctcgctcaagccttcgtcactggtcccgccaccaaacgtttcggcgagaagcaggccattatcgccggcatggcggccgacgcgcggggagaggcggtttgcgtattgggcgccagggtggtttttcttttcaccagtgagacgggcaacagctgattgcccttcaccgcctggccctgagagagttgcagcaagcggtccacgctggtttgccccagcaggcgaaaatcctgtttgatggtggttaacggcgggatataacatgagctgtcttcggtatcgtcgtatcccactaccgagatatccgcaccaacgcgcagcccggactcggtaatggcgcgcattgcgcccagcgccatctgatcgttggcaaccagcatcgcagtgggaacgatgccctcattcagcatttgcatggtttgttgaaaaccggacatggcactccagtcgccttcccgttccgctatcggctgaatttgattgcgagtgagatatttatgccagccagccagacgcagacgcgccgagacagaacttaatgggcccgctaacagcgcgatttgctggtgacccaatgcgaccagatgctccacgcccagtcgcgtaccgtcttcatgggagaaaataatactgttgatgggtgtctggtcagagacatcaagaaataacgccggaacattagtgcaggcagcttccacagcaatggcatcctggtcatccagcggatagttaatgatcagcccactgacgcgttgcgcgagaagattgtgcaccgccgctttacaggcttcgacgccgcttcgttctaccatcgacaccaccacgctggcacccagttgatcggcgcgagatttaatcgccgcgacaatttgcgacggcgcgtgcagggccagactggaggtggcaacgccaatcagcaacgactgtttgcccgccagttgttgtgccacgcggttgggaatgtaattcagctccgccatcgccgcttccactttttcccgcgttttcgcagaaacgtggctggcctggttcaccacgcgggaaacggtctgataagagacaccggcatactctgcgacatcgtataacgttactggtttcacattcaccaccctgaattgactctcttccgggcgctatcatgccataccgcgaaaggttttgcaccattcgatggtgtcaacgtaaatgcatgccgcttcgccttcgcgcgcgaattgcaagctgatccgggcttatcgactgcacggtgcaccaatgcttctggcgtcaggcagccatcggaagctgtggtatggctgtgcaggtcgtaaatcactgcataattcgtgtcgctcaaggcgcactcccgttctggataatgttttttgcgccgacatcataacggttctggcaaatattctgaaatgagctgttgacaattaatcatcggctcgtataatgtgtggaattgtgagcggataacaatttcacacaggaaacagggatctgatccggatttactaactggaagaggcactaaatgaacacgattaacatcgctaagaacgacttctctgacatcgaactggctgctatcccgttcaacactctggctgaccattacggtgagcgtttagctcgcgaacagttggcccttgagcatgagtcttacgagatgggtgaagcacgcttccgcaagatgtttgagcgtcaacttaaagctggtgaggttgcggataacgctgccgccaagcctctcatcactaccctactccctaagatgattgcacgcatcaacgactggtttgaggaagtgaaagctaagcgcggcaagcgcccgacagccttccagttcctgcaagaaatcaagccggaagccgtagcgtacatcaccattaagaccactctggcttgcctaaccagtgctgacaatacaaccgttcaggctgtagcaagcgcaatcggtcgggccattgaggacgaggctcgcttcggtcgtatccgtgaccttgaagctaagcacttcaagaaaaacgttgaggaacaactcaacaagcgcgtagggcacgtctacaagaaagcatttatgcaagttgtcgaggctgacatgctctctaagggtctactcggtggcgaggcgtggtcttcgtggcataaggaagactctattcatgtaggagtacgctgcatcgagatgctcattgagtcaaccggaatggttagcttacaccgccaaaatgctggcgtagtaggtcaagactctgagactatcgaactcgcacctgaatacgctgaggctatcgcaacccgtgcaggtgcgctggctggcatctctccgatgttccaaccttgcgtagttcctcctaagccgtggactggcattactggtggtggctattgggctaacggtcgtcgtcctctggcgctggtgcgtactcacagtaagaaagcactgatgcgctacgaagacgtttacatgcctgaggtgtacaaagcgattaacattgcgcaaaacaccgcatggaaaatcaacaagaaagtcctagcggtcgccaacgtaatcaccaagtggaagcattgtccggtcgaggacatccctgcgattgagcgtgaagaactcccgatgaaaccggaagacatcgacatgaatcctgaggctctcaccgcgtggaaacgtgctgccgctgctgtgtaccgcaaggacaaggctcgcaagtctcgccgtatcagccttgagttcatgcttgagcaagccaataagtttgctaaccataaggccatctggttcccttacaacatggactggcgcggtcgtgtttacgctgtgtcaatgttcaacccgcaaggtaacgatatgaccaaaggactgcttacgctggcgaaaggtaaaccaatcggtaaggaaggttactactggctgaaaatccacggtgcaaactgtgcgggtgtcgataaggttccgttccctgagcgcatcaagttcattgaggaaaaccacgagaacatcatggcttgcgctaagtctccactggagaacacttggtgggctgagcaagattctccgttctgcttccttgcgttctgctttgagtacgctggggtacagcaccacggcctgagctataactgctcccttccgctggcgtttgacgggtcttgctctggcatccagcacttctccgcgatgctccgagatgaggtaggtggtcgcgcggttaacttgcttcctagtgaaaccgttcaggacatctacgggattgttgctaagaaagtcaacgagattctacaagcagacgcaatcaatgggaccgataacgaagtagttaccgtgaccgatgagaacactggtgaaatctctgagaaagtcaagctgggcactaaggcactggctggtcaatggctggcttacggtgttactcgcagtgtgactaagcgttcagtcatgacgctggcttacgggtccaaagagttcggcttccgtcaacaagtgctggaagataccattcagccagctattgattccggcaagggtctgatgttcactcagccgaatcaggctgctggatacatggctaagctgatttgggaatctgtgagcgtgacggtggtagctgcggttgaagcaatgaactggcttaagtctgctgctaagctgctggctgctgaggtcaaagataagaagactggagagattcttcgcaagcgttgcgctgtgcattgggtaactcctgatggtttccctgtgtggcaggaatacaagaagcctattcagacgcgcttgaacctgatgttcctcggtcagttccgcttacagcctaccattaacaccaacaaagatagcgagattgatgcacacaaacaggagtctggtatcgctcctaactttgtacacagccaagacggtagccaccttcgtaagactgtagtgtgggcacacgagaagtacggaatcgaatcttttgcactgattcacgactccttcggtaccattccggctgacgctgcgaacctgttcaaagcagtgcgcgaaactatggttgacacatatgagtcttgtgatgtactggctgatttctacgaccagttcgctgaccagttgcacgagtctcaattggacaaaatgccagcacttccggctaaaggtaacttgaacctccgtgacatcttagagtcggacttcgcgttcgcgtaacatatggatatctgtcgacggccgtcgttttacagccaagcttggctgttttggcggatgagagaagattttcagcctgatacagattaaatcagaacgcagaagcggtctgataaaacagaatttgcctggcggcagtagcgcggtggtcccacctgaccccatgccgaactcagaagtgaaacgccgtagcgccgatggtagtgtggggtctccccatgcgagagtagggaactgccaggcatcaaataaaacgaaaggctcagtcgaaagactgggcctttcgttttatctgttgtttgtcggtgaacgctctcctgagtaggacaaatccgccgggagcggatttgaacgttgcgaagcaacggcccggagggtggcgggcaggacgcccgccataaactgccaggcatcaaattaagcagaaggccatcctgacggatggcctttttgcgtttctacaaactcttttggtcgactctagagttccactgagcgtcagaccccgtagaaaagatcaaaggatcttcttgagatcctttttttctgcgcgtaatctgctgcttgcaaacaaaaaaaccaccgctaccagcggtggtttgtttgccggatcaagagctaccaactctttttccgaaggtaactggcttcagcagagcgcagataccaaatactgtccttctagtgtagccgtagttaggccaccacttcaagaactctgtagcaccgcctacatacctcgctctgctaatcctgttaccagtggctgctgccagtggcgataagtcgtgtcttaccgggttggactcaagacgatagttaccggataaggcgcagcggtcgggctgaacggggggttcgtgcacacagcccagcttggagcgaacgacctacaccgaactgagatacctacagcgtgagctatgagaaagcgccacgcttcccgaagggagaaaggcggacaggtatccggtaagcggcagggtcggaacaggagagcgcacgagggagcttccagggggaaacgcctggtatctttatagtcctgtcgggtttcgccacctctgacttgagcgtcgatttttgtgatgctcgtcaggggggcggagcctatggaaaaacgccagcaacgcggcctttttacggttcctggccttttgctggccttttgctcacatgttctttcctgcgttatcccctgattctgtggataaccgtattaccgcctttgagtgagctgataccgctcgccgcagccgaacgaccgagcgcagcgagtcagtgagcgaggaagcggaagatctagaagtactgctgactcataccaggcctgaatcgccccatcatccagccagaaagtgagggagccacggttgatgagagctttgttgtaggtggaccagttggtgattttgaacttttgctttgccacggaacggtctgcgttgtcgggaagatgcgtgatctgatccttcaactcagcaaaagttcgatttattcaacaaagccacgttgtgtctcaaaatctctgatgttacattgcacaagataaaaatatatcatcatgaacaataaaactgtctgcttacataaacagtaatacaaggggtgttatgagccatattcaacgggaaacgtcttgctcaaggccgcgattaaattccaacatggatgctgatttatatgggtataaatgggctcgcgataatgtcgggcaatcaggtgcgacaatctatcgattgtatgggaagcccgatgcgccagagttgtttctgaaacatggcaaaggtagcgttgccaatgatgttacagatgagatggtcagactaaactggctgacggaatttatgcctcttccgaccatcaagcattttatccgtactcctgatgatgcatggttactcaccactgcgatccccggaaaaacagcattccaggtattagaagaatatcctgattcaggtgaaaatattgttgatgcgctggcagtgttcctgcgccggttgcattcgattcctgtttgtaattgtccttttaacagcgatcgcgtatttcgtctcgctcaggcgcaatcacgaatgaataacggtttggttgatgcgagtgattttgatgacgagcgtaatggctggcctgttgaacaagtctggaaagaaatgcataagcttttgccattctcaccggattcagtcgtcactcatggtgatttctcacttgataaccttatttttgacgaggggaaattaataggttgtattgatgttggacgagtcggaatcgcagaccgataccaggatcttgccatcctatggaactgcctcggtgagttttctccttcattacagaaacggctttttcaaaaatatggtattgataatcctgatatgaataaattgcagtttcatttgatgctcgatgagtttttctaaggctagccccgggactagtgatctttgggagcagtccttgtgcgcttacgaggtgagccggtggggaaccgttatctgcctatggtgtgagcccccctagagagcttcaagagcaatcagcccgacctagaaaggaggccaagagagagacccctacggggggaaccgttttctgcctacgagatggcacatttactgggaagctttacggcgtcctcgtggaagttcaatgcccgcagacttaagtgctctattcacggtctgacgtgacacgctaaattcagacatagcttcattgattgtcggccacgagccagtctctccctcaacagtcataaaccaacctgcaatggtcaagcgatttcctttagctttcctagcttgtcgttgactggacttagctagtttttctcgctgtgctcgggcgtactcactgtttgggtctttccagcgttctgcggcctttttaccgccacgtcttcccatagtggccagagcttttcgccctcggctgctctgcgtctctgtctgacgagcagggacgactggctggcctttagcgacgtagccgcgcacacgtcgcgccatcgtctggcggtcacgcatcggcggcagatcaggctcacggccgtctgctccgaccgcctgagcgacggtgtaggcacgctcgtaggcgtcgatgatcttggtgtcttttaggcgctcaccagccgcttttaactggtatcccacagtcaaagcgtggcgaaaagccgtctcatcacgggcggcacgccctggagcagtccagaggacacggacgccgtcgatcagctctccagacgcttcagcggcgctcggcaggcttgcttcaagcgtggcaagtgcttttgcttccgcagtggcttttcttgccgcttcgatacgtgcccgtccgctagaaaactcctgctcatagcgttttttaggtttttctgtgcctgagatcatgcgagcaacctccataagatcagctaggcgatccacgcgattgtgctgggcatgccagcggtacgcggtgggatcgtcggagacgtgcagtggccaccggctcagcctatgtgaaaaagcctggtcagcgccgaaaacgcgggtcatttcctcggtcgttgcagccagcaggcgcatattcgggctgctcatgcctgctgcggcatacaccggatcaatgagccagatgagctggcatttcccgctcagtggattcacgccgatccaagctggcgctttttccaggcgtgcccagcgctccaaaatcgcgtagacctcggggtttacgtgctcgattttcccgccggcctggtggctcggcacatcaatgtccaggacaagcacggctgcgtgctgcgcgtgcgtcagagcaacatactggcaccgggcaagcgattttgaaccaactcggtataacttcggctgtgtttctcccgtgtccgggtctttgatccaagcgctggcgaagtcgcgggtcttgctgccctggaaattttctctgcccaggtgagcgaggaattcgcggcggtcttcgctcgtccagccacgtgatcgcagcgcgagctcgggatgggtgtcgaacagatcagcggaaaatttccaggccggtgtgtcaatgtctcgtgaatccgctagagtcatttttgagcgctttctcccaggtttggactgggggttagccgacgccctgtgagttaccgctcacggggcgttcaacatttttcaggtattcgtgcagcttatcgcttcttgccgcctgtgcgctttttcgacgcgcgacgctgctgccgattcggtgcaggtggtggcggcgctgacacgtcctgggcggccacggccacacgaaacgcggcatttacgatgtttgtcatgcctgcgggcaccgcgccacgatcgcggataattctcgctgccgcttccagctctgtgacgaccatggccaaaatttcgctcgggggacgcacttccagcgccatttgcgacctagccgcctccagctcctcggcgtggcgtttgttggcgcgctcgcggctggctgcggcacgacacgcatctgagcaatattttgcgcgccgtcctcgcgggtcaggccggggaggaatcaggccaccgcagtaggcgcaactgattcgatcctccactactgtgcgtcctcctggcgctgccgagcacgcagctcgtcagccagctcctcaagatccgccacgagagtttctaggtcgctcgcggcactggcccagtctcgtgatgctggcgcgtccgtcgtatcgagagctcggaaaaatccgatcaccgtttttaaatcgacggcagcatcgagcgcgtcggactccagcgcgacatcagagagatccatagctgatgattcgggccaattttggtacttcgtcgtgaaggtcatgacaccattataacgaacgttcgttaaagtttttggcggaaaatcacgcggcacgaaaattttcacgaagcgggactttgcgcagctcaggggtgctaaaaattttgtatcgcacttgatttttccgaaagacagattatctgcaaacggtgtgtcgtatttctggcttggtttttaaaaaatctggaatcgaaaatttgcggggcga